European Patent Application EP 4 711 464 A1, published March 18, 2026. Title: 一种预防和治疗动物传染性腹膜炎的药物组合物. Applicant: 北京伟杰信生物科技有限公司. The sequence listing filed with the application follows.

SEQUENCE LISTING (76 sequences)

SEQ ID NO: 1 - DNA, 68 bp, synthetic construct
  source 1..68: mol_type = other DNA
ggatagctaccagcttacacttgcttctgacacaactgtgttcgctatcaaccacacaaacagacacc

SEQ ID NO: 2 - skipped

SEQ ID NO: 3 - DNA, 126 bp, synthetic construct
  source 1..126: mol_type = other DNA
gctccctttcttgctttccagggaaagtcccttggtccccagaccctaatacctggacatgtctaaatcatgaaattctttgaacatctggctcctgcctaataaagaatatttattttcattgca

SEQ ID NO: 4 - DNA, 63 bp, synthetic construct
  source 1..63: mol_type = other DNA
ggcagcggcgaaggccgcggcagcctgctgacctgcggcgatgtggaagaaaacccgggcccg

SEQ ID NO: 5 - DNA, 66 bp, synthetic construct
  source 1..66: mol_type = other DNA
ggcagcggcgcgaccaactttagcctgctgaaacaggcgggcgatgtggaagaaaacccgggcccg

SEQ ID NO: 6 - DNA, 100 bp, synthetic construct
  source 1..100: mol_type = other DNA
aaaaaaaaaaaaaaaaaaaaaaaaaaaaaaaaaaaaaaaaaaaaaaaaaaaaaaaaaaaaaaaaaaaaaaaaaaaaaaaaaaaaaaaaaaaaaaaaaaaa

SEQ ID NO: 7 - DNA, 789 bp, Feline Coronavirus
  source 1..789: mol_type = genomic DNA
atgaagtacattttgttaatactcgcgtgcattattgcatgcgtttatggagaacgctactgtgccatgcaaaatacaggctcgcagtgcattaatggcacagattcatcatgtagcacctgttttgaacgtggtggtcttatttggcatctggctaactggaacttcagctggtctgtaatattgattgtttttataacagtgttaaaatatggaagaccgcaattcagctggctcgtttatggcattaaaatgctgatcatgtggctattatggcctattgttctagcgcttacgatttttaatgcatactctgagtaccaagtttccagatatgtaatgttcggctttagtgttgcaggtgcagttgtaacgtttgcactatggatgatgtattttgtgagatctattcagctgtatagacggaccaaatcatggtggtcttttaatcctgaaaccaatgcgattctttgtgtcaatgcattgggtagaagctatgtactccctcttgatggcactcctacaggtgttactcttaccctactttcaggaaatctatacgctgaaggttttaaaatggctggtggtcttaccatcgagcatttgcctaaatatgtcatgattgctacgcctagtagaaccatcgtttacacattagttggaaaacaactaaaggcaactactgccactggatgggcttactatgtaaaatctaaagctggtgattactcaacagaagcacgtactgataatttgagtgaacatgaaaaattattacatatggtgtaa

SEQ ID NO: 8 - DNA, 1131 bp, Feline Coronavirus
  source 1..1131: mol_type = genomic DNA
atggccacacagggacaacgcgtcaactggggagatgaaccttccaaaagacgtggtcgttctaactctcgtggtcggaagaataacactatacctctttcattcttcaatcccatccaactcgaaccaggatcaaaattttggagcgtatgtccgagagattttgttcccaagggaataggtaacaaggatcaacaaattggttattggaatagacaagagcgttaccgcattgtcaaaggtcagcgtaaggaacttcctgagaggtggtttttctacttcttaggcacaggacctcaagctgatgctaaatttaaagacaagattgatggagtcttctgggttgcaaaggatggtgccatgaataaaccaacaacacttggcactcgtggtaccaacaatgaatccaaaccactgaaatttgatggtaagataccaccgcaatttcagcttgaagtgaaccgatctaggaacaactcaagaagtggttctcagtctagatctgtctctagaaacaggtctcaatccagaggaagacaacaatccaataatcagaataatgttgaggatacaattgtagctgtgcttcagaaattaggtgttactgaaaagcaaaggtcacgttctaaatctagagatcgtggtgactctaaacctagagacacaacacctaataatgccaacaaacacacctggaagaagactgcaggtaaaggtgatgtgacaaatttctatggtgctagaagtgcttcagctaactttggtgatagtgatctcgttgccaacggtaacgctgccaaatcctaccctcagatagctgaatgcgttccatcagtgtctagcatgctcttcggtagtcaatggtctgctgaagatgatggtgatcaagtgaaagtcacgctcactcatacctattacctgccaaaagatgatgccaaaaccagccaattcctagaacagattgacgcttacaagcggccatctcaagtggctaaagatcagaggcaaagaaaatctcgttctaagtctgctgagaagaagcctgaggaattgtctgtaactcttgtagaggcatatacggatgtgtttgatgacacacaggttgagatgattgatgaggttacgaactaa

SEQ ID NO: 9 - DNA, 4359 bp, Feline Coronavirus
  source 1..4359: mol_type = genomic DNA
atgattgtgctcgtaacttgcctcttgttgttatgttcataccacacagttttgagtacaacaaataatgaatgcatacaagttaacgtaacacaattggctggcaatgaaaaccttatcagagattttctgtttagtaactttaaagaagaaggaagtgtagttgttggtggttattaccctacagaggtgtggtacaactgctctagaacagctcgaactactgcctttcagtattttaataatatacatgccttttattttgttatggaagccatggaaaatagcactggtaatgcacgtggtaaaccattattatttcatgtgcatggtgagcctgttagtgttattatatcggcttatagggatgatgtgcaacaaaggccccttttaaaacatgggttagtgtgcataactaaaaatcgccatattaactatgaacaattcacctccaaccagtggaattccacatgtacgggtgctgacagaaaaattcctttctctgtcatacccacggacaatggaacaaaaatctatggtcttgagtggaatgatgactttgttacagcttatattagtggtcgttcttatcacttgaacatcaatactaattggtttaacaatgtcacacttttgtattcacgctcaagcactgctacctgggaatacagtgctgcatatgcttaccaaggtgtttctaacttcacttattacaagttaaataacaccaatggtctaaaaacctatgaattatgtgaagattatgaacattgcactggctatgctaccaatgtatttgctccgacatcaggtggttacatacctgatggatttagttttaacaattggttcttgcttacaaatagttccacttttgttagtggcaggtttgtaacaaatcaaccattattgattaattgcttgtggccagtgcccagttttggtgtagcagcacaagaattttgttttgaaggtgcacagtttagccaatgtaatggtgtgtctttaaataacacagtggatgttattagattcaaccttaatttcactgcagatgtacaatctggtatgggtgctacagtattttcactgaatacaacaggtggtgtcattcttgaaatttcatgttatagtgacacagtgagtgagtctagttcttacagttatggtgaaatcccgttcggcataactgacggaccacgatactgttatgtactttacaatggcacagctcttaaatatttaggaacattaccacccagtgtaaaggaaattgctattagtaagtggggccatttttatattaatggttacaatttctttagcacatttcctattggttgtatatcttttaatttaaccactggtgttagtggagctttttggacaattgcttacacatcgtatactgaagcattagtacaagttgaaaacacagctattaaaaatgtgacgtattgtaacagtcacattaataacattaaatgttctcaacttactgctaatttgaataatggattttatcctgttgcttcaagtgaagtaggtttcgttaataagagtgttgtgttattacctagctttttcacatacaccgctgtcaatataaccattgatcttggtatgaagcttagtggttatggtcaacccatagcctcgacactaagtaacatcacactaccaatgcaggataacaatactgatgtgtactgtattcgttctaaccaattctcagtttatgttcattccacttgcaaaagttctttatgggacaatatttttaatcaagactgcacggatgttttagaggctacagctgttataaaaactggtacttgtcctttctcatttgataaattgaacaattacttgacttttaacaagttctgtttgtcgttgagtcctgttggtgctaattgcaagtttgatgttgctgcacgtacaagaaccaatgagcaggttgttagaagtctatatgtaatatatgaagaaggagacaacatagtgggtgtaccgtctgataatagcggtctgcacgatttgtctgtgctacacctagactcctgtacagattacaatatatatggtagaactggtgttggtattattagacgaactaacagtacgctacttagtggcttatattacacatcactatcaggtgatttgttaggctttaaaaatgttagtgatggtgtcatttattctgtgacgccatgtgatgtaagcgcacaagcggctgttattgatggtgccatagttggagctatgacttccattaacagtgaactgttaggtctaacacattggacaacgacacctaatttttattactactctatatataattacacaagtgagaggactcgtgacactgcaattgacagtaacgatgttgattgtgaacctgtcataacctattctaatataggtgtttgtaaaaatggtgctttggtttttattaacgtcacacattctgacggagacgtgcaaccaattagcactggtaatgtcacgatacctacaaattttaccatatctgtgcaagttgaatacatgcaggtttacactacaccagtatcaatagattgtgcaagatacgtttgtaatggtaaccctagatgtaacaaattgttaacacaatatgtgtctgcatgtcaaactattgaacaagcacttgcaatgggtgccagacttgaaaacatggaggttgattccatgttgtttgtctcggaaaatgcccttaaattggcatctgttgaggcgttcaatagtacagaaaatttagattctatttacaaagaatggcctagcataggtggttcttggctaggaggtctaaaagatatactaccgtcccataatagcaaacgtaagtatggttctgctatagaagatttgctttttgataaagttgtaacatctggtttaggtacagttgatgaagattataaacgttgtactggtggttacgacatagcagacttggtgtgtgctcaatattacaatggcatcatggttctaccaggtgtagctaatgctgacaagatgactatgtacacagcatcacttgcaggtggtataacattaggtgcacttggtggtggcgccgtggctataccttttgcagtagcagtacaggctagacttaattatgttgctctacaaactgatgtattgaataaaaaccaacagatcctggctaatgccttcaatcaagctattggtaacattacacaggcttttggtaaggttaatgatgctatacatcaaacatcacaaggtcttgccactgttgctaaagcgttggcaaaagtgcaagatgttgtcaacacacaagggcaagctttaagtcaccttacagtacaattgcaaaataattttcaagccattagtagttctattagtgatatttataacaggcttgacgaactgagtgctgatgcacaagttgataggctgattacaggtagacttacagcacttaatgcatttgtgtctcagactctaaccagacaagcagaggttagggctagtagacaacttgccaaagacaaggttaatgaatgtgttaggtctcagtctcagagattcggattctgtggtaatggtacacatttgttttcactagcaaatgcagcaccaaatggcatgattttctttcatacagtactattaccaacagcttatgaaactgtaacagcttggtcaggtatttgtgcttcagatggcgatcgcactttcggacttgtcgttaaagatgtgcagttgacgttgtttcgtaatctagatgacaagttctatttgacccccagaactatgtatcagcctagagttgcaactagttctgattttgttcaaattgaagggtgtgatgtgttgtttgtcaacgcgactgtaattgatttgcctagtattatacctgactatattgacattaatcaaactgttcaagacatattagaaaattacagaccaaactggactgtacctgaatttacacttgatattttcaacgcaacctatttaaatctgactggtgaaattgatgacttagagtttaggtcagaaaagctacataacactacagtagaacttgccattctcattgataacattaataatacattagtcaatcttgaatggctcaatagaattgaaacttatgtaaaatggccttggtatgtgtggctactgataggtttagtagtagtattttgcataccattactgctattttgctgttttagcacaggttgttgtggatgcataggttgtttaggaagttgttgtcactctatatgtagtagaagacaatttgaaaattatgaaccaattgaaaaagtgcatgtccactaa

SEQ ID NO: 10 - DNA, 2337 bp, Feline Coronavirus
  source 1..2337: mol_type = genomic DNA
atgattgtgctcgtaacttgcctcttgttgttatgttcataccacacagttttgagtacaacaaataatgaatgcatacaagttaacgtaacacaattggctggcaatgaaaaccttatcagagattttctgtttagtaactttaaagaagaaggaagtgtagttgttggtggttattaccctacagaggtgtggtacaactgctctagaacagctcgaactactgcctttcagtattttaataatatacatgccttttattttgttatggaagccatggaaaatagcactggtaatgcacgtggtaaaccattattatttcatgtgcatggtgagcctgttagtgttattatatcggcttatagggatgatgtgcaacaaaggccccttttaaaacatgggttagtgtgcataactaaaaatcgccatattaactatgaacaattcacctccaaccagtggaattccacatgtacgggtgctgacagaaaaattcctttctctgtcatacccacggacaatggaacaaaaatctatggtcttgagtggaatgatgactttgttacagcttatattagtggtcgttcttatcacttgaacatcaatactaattggtttaacaatgtcacacttttgtattcacgctcaagcactgctacctgggaatacagtgctgcatatgcttaccaaggtgtttctaacttcacttattacaagttaaataacaccaatggtctaaaaacctatgaattatgtgaagattatgaacattgcactggctatgctaccaatgtatttgctccgacatcaggtggttacatacctgatggatttagttttaacaattggttcttgcttacaaatagttccacttttgttagtggcaggtttgtaacaaatcaaccattattgattaattgcttgtggccagtgcccagttttggtgtagcagcacaagaattttgttttgaaggtgcacagtttagccaatgtaatggtgtgtctttaaataacacagtggatgttattagattcaaccttaatttcactgcagatgtacaatctggtatgggtgctacagtattttcactgaatacaacaggtggtgtcattcttgaaatttcatgttatagtgacacagtgagtgagtctagttcttacagttatggtgaaatcccgttcggcataactgacggaccacgatactgttatgtactttacaatggcacagctcttaaatatttaggaacattaccacccagtgtaaaggaaattgctattagtaagtggggccatttttatattaatggttacaatttctttagcacatttcctattggttgtatatcttttaatttaaccactggtgttagtggagctttttggacaattgcttacacatcgtatactgaagcattagtacaagttgaaaacacagctattaaaaatgtgacgtattgtaacagtcacattaataacattaaatgttctcaacttactgctaatttgaataatggattttatcctgttgcttcaagtgaagtaggtttcgttaataagagtgttgtgttattacctagctttttcacatacaccgctgtcaatataaccattgatcttggtatgaagcttagtggttatggtcaacccatagcctcgacactaagtaacatcacactaccaatgcaggataacaatactgatgtgtactgtattcgttctaaccaattctcagtttatgttcattccacttgcaaaagttctttatgggacaatatttttaatcaagactgcacggatgttttagaggctacagctgttataaaaactggtacttgtcctttctcatttgataaattgaacaattacttgacttttaacaagttctgtttgtcgttgagtcctgttggtgctaattgcaagtttgatgttgctgcacgtacaagaaccaatgagcaggttgttagaagtctatatgtaatatatgaagaaggagacaacatagtgggtgtaccgtctgataatagcggtctgcacgatttgtctgtgctacacctagactcctgtacagattacaatatatatggtagaactggtgttggtattattagacgaactaacagtacgctacttagtggcttatattacacatcactatcaggtgatttgttaggctttaaaaatgttagtgatggtgtcatttattctgtgacgccatgtgatgtaagcgcacaagcggctgttattgatggtgccatagttggagctatgacttccattaacagtgaactgttaggtctaacacattggacaacgacacctaatttttattactac

SEQ ID NO: 11 - DNA, 2023 bp, Feline Coronavirus
  source 1..2023: mol_type = genomic DNA
atgtatatataattacacaagtgagaggactcgtgacactgcaattgacagtaacgatgttgattgtgaacctgtcataacctattctaatataggtgtttgtaaaaatggtgctttggtttttattaacgtcacacattctgacggagacgtgcaaccaattagcactggtaatgtcacgatacctacaaattttaccatatctgtgcaagttgaatacatgcaggtttacactacaccagtatcaatagattgtgcaagatacgtttgtaatggtaaccctagatgtaacaaattgttaacacaatatgtgtctgcatgtcaaactattgaacaagcacttgcaatgggtgccagacttgaaaacatggaggttgattccatgttgtttgtctcggaaaatgcccttaaattggcatctgttgaggcgttcaatagtacagaaaatttagattctatttacaaagaatggcctagcataggtggttcttggctaggaggtctaaaagatatactaccgtcccataatagcaaacgtaagtatggttctgctatagaagatttgctttttgataaagttgtaacatctggtttaggtacagttgatgaagattataaacgttgtactggtggttacgacatagcagacttggtgtgtgctcaatattacaatggcatcatggttctaccaggtgtagctaatgctgacaagatgactatgtacacagcatcacttgcaggtggtataacattaggtgcacttggtggtggcgccgtggctataccttttgcagtagcagtacaggctagacttaattatgttgctctacaaactgatgtattgaataaaaaccaacagatcctggctaatgccttcaatcaagctattggtaacattacacaggcttttggtaaggttaatgatgctatacatcaaacatcacaaggtcttgccactgttgctaaagcgttggcaaaagtgcaagatgttgtcaacacacaagggcaagctttaagtcaccttacagtacaattgcaaaataattttcaagccattagtagttctattagtgatatttataacaggcttgacgaactgagtgctgatgcacaagttgataggctgattacaggtagacttacagcacttaatgcatttgtgtctcagactctaaccagacaagcagaggttagggctagtagacaacttgccaaagacaaggttaatgaatgtgttaggtctcagtctcagagattcggattctgtggtaatggtacacatttgttttcactagcaaatgcagcaccaaatggcatgattttctttcatacagtactattaccaacagcttatgaaactgtaacagcttggtcaggtatttgtgcttcagatggcgatcgcactttcggacttgtcgttaaagatgtgcagttgacgttgtttcgtaatctagatgacaagttctatttgacccccagaactatgtatcagcctagagttgcaactagttctgattttgttcaaattgaagggtgtgatgtgttgtttgtcaacgcgactgtaattgatttgcctagtattatacctgactatattgacattaatcaaactgttcaagacatattagaaaattacagaccaaactggactgtacctgaatttacacttgatattttcaacgcaacctatttaaatctgactggtgaaattgatgacttagagtttaggtcagaaaagctacataacactacagtagaacttgccattctcattgataacattaataatacattagtcaatcttgaatggctcaatagaattgaaacttatgtaaaatggccttggtatgtgtggctactgataggtttagtagtagtattttgcataccattactgctattttgctgttttagcacaggttgttgtggatgcataggttgtttaggaagttgttgtcactctatatgtagtagaagacaatttgaaaattatgaaccaattgaaaaagtgcatgtccactaa

SEQ ID NO: 12 - DNA, 1980 bp, synthetic construct
  source 1..1980: mol_type = other DNA
atgaagtacattttgttaatactcgcgtgcattattgcatgcgtttatggagaacgctactgtgccatgcaaaatacaggctcgcagtgcattaatggcacagattcatcatgtagcacctgttttgaacgtggtggtcttatttggcatctggctaactggaacttcagctggtctgtaatattgattgtttttataacagtgttaaaatatggaagaccgcaattcagctggctcgtttatggcattaaaatgctgatcatgtggctattatggcctattgttctagcgcttacgatttttaatgcatactctgagtaccaagtttccagatatgtaatgttcggctttagtgttgcaggtgcagttgtaacgtttgcactatggatgatgtattttgtgagatctattcagctgtatagacggaccaaatcatggtggtcttttaatcctgaaaccaatgcgattctttgtgtcaatgcattgggtagaagctatgtactccctcttgatggcactcctacaggtgttactcttaccctactttcaggaaatctatacgctgaaggttttaaaatggctggtggtcttaccatcgagcatttgcctaaatatgtcatgattgctacgcctagtagaaccatcgtttacacattagttggaaaacaactaaaggcaactactgccactggatgggcttactatgtaaaatctaaagctggtgattactcaacagaagcacgtactgataatttgagtgaacatgaaaaattattacatatggtgggcagcggcgaaggccgcggcagcctgctgacctgcggcgatgtggaagaaaacccgggcccgatggccacacagggacaacgcgtcaactggggagatgaaccttccaaaagacgtggtcgttctaactctcgtggtcggaagaataacactatacctctttcattcttcaatcccatccaactcgaaccaggatcaaaattttggagcgtatgtccgagagattttgttcccaagggaataggtaacaaggatcaacaaattggttattggaatagacaagagcgttaccgcattgtcaaaggtcagcgtaaggaacttcctgagaggtggtttttctacttcttaggcacaggacctcaagctgatgctaaatttaaagacaagattgatggagtcttctgggttgcaaaggatggtgccatgaataaaccaacaacacttggcactcgtggtaccaacaatgaatccaaaccactgaaatttgatggtaagataccaccgcaatttcagcttgaagtgaaccgatctaggaacaactcaagaagtggttctcagtctagatctgtctctagaaacaggtctcaatccagaggaagacaacaatccaataatcagaataatgttgaggatacaattgtagctgtgcttcagaaattaggtgttactgaaaagcaaaggtcacgttctaaatctagagatcgtggtgactctaaacctagagacacaacacctaataatgccaacaaacacacctggaagaagactgcaggtaaaggtgatgtgacaaatttctatggtgctagaagtgcttcagctaactttggtgatagtgatctcgttgccaacggtaacgctgccaaatcctaccctcagatagctgaatgcgttccatcagtgtctagcatgctcttcggtagtcaatggtctgctgaagatgatggtgatcaagtgaaagtcacgctcactcatacctattacctgccaaaagatgatgccaaaaccagccaattcctagaacagattgacgcttacaagcggccatctcaagtggctaaagatcagaggcaaagaaaatctcgttctaagtctgctgagaagaagcctgaggaattgtctgtaactcttgtagaggcatatacggatgtgtttgatgacacacaggttgagatgattgatgaggttacgaactaa

SEQ ID NO: 13 - DNA, 1980 bp, synthetic construct
  source 1..1980: mol_type = other DNA
atggccacacagggacaacgcgtcaactggggagatgaaccttccaaaagacgtggtcgttctaactctcgtggtcggaagaataacactatacctctttcattcttcaatcccatccaactcgaaccaggatcaaaattttggagcgtatgtccgagagattttgttcccaagggaataggtaacaaggatcaacaaattggttattggaatagacaagagcgttaccgcattgtcaaaggtcagcgtaaggaacttcctgagaggtggtttttctacttcttaggcacaggacctcaagctgatgctaaatttaaagacaagattgatggagtcttctgggttgcaaaggatggtgccatgaataaaccaacaacacttggcactcgtggtaccaacaatgaatccaaaccactgaaatttgatggtaagataccaccgcaatttcagcttgaagtgaaccgatctaggaacaactcaagaagtggttctcagtctagatctgtctctagaaacaggtctcaatccagaggaagacaacaatccaataatcagaataatgttgaggatacaattgtagctgtgcttcagaaattaggtgttactgaaaagcaaaggtcacgttctaaatctagagatcgtggtgactctaaacctagagacacaacacctaataatgccaacaaacacacctggaagaagactgcaggtaaaggtgatgtgacaaatttctatggtgctagaagtgcttcagctaactttggtgatagtgatctcgttgccaacggtaacgctgccaaatcctaccctcagatagctgaatgcgttccatcagtgtctagcatgctcttcggtagtcaatggtctgctgaagatgatggtgatcaagtgaaagtcacgctcactcatacctattacctgccaaaagatgatgccaaaaccagccaattcctagaacagattgacgcttacaagcggccatctcaagtggctaaagatcagaggcaaagaaaatctcgttctaagtctgctgagaagaagcctgaggaattgtctgtaactcttgtagaggcatatacggatgtgtttgatgacacacaggttgagatgattgatgaggttacgaacggcagcggcgaaggccgcggcagcctgctgacctgcggcgatgtggaagaaaacccgggcccgatgaagtacattttgttaatactcgcgtgcattattgcatgcgtttatggagaacgctactgtgccatgcaaaatacaggctcgcagtgcattaatggcacagattcatcatgtagcacctgttttgaacgtggtggtcttatttggcatctggctaactggaacttcagctggtctgtaatattgattgtttttataacagtgttaaaatatggaagaccgcaattcagctggctcgtttatggcattaaaatgctgatcatgtggctattatggcctattgttctagcgcttacgatttttaatgcatactctgagtaccaagtttccagatatgtaatgttcggctttagtgttgcaggtgcagttgtaacgtttgcactatggatgatgtattttgtgagatctattcagctgtatagacggaccaaatcatggtggtcttttaatcctgaaaccaatgcgattctttgtgtcaatgcattgggtagaagctatgtactccctcttgatggcactcctacaggtgttactcttaccctactttcaggaaatctatacgctgaaggttttaaaatggctggtggtcttaccatcgagcatttgcctaaatatgtcatgattgctacgcctagtagaaccatcgtttacacattagttggaaaacaactaaaggcaactactgccactggatgggcttactatgtaaaatctaaagctggtgattactcaacagaagcacgtactgataatttgagtgaacatgaaaaattattacatatggtgtaa

SEQ ID NO: 14 - DNA, 1983 bp, synthetic construct
  source 1..1983: mol_type = other DNA
atgaagtacattttgttaatactcgcgtgcattattgcatgcgtttatggagaacgctactgtgccatgcaaaatacaggctcgcagtgcattaatggcacagattcatcatgtagcacctgttttgaacgtggtggtcttatttggcatctggctaactggaacttcagctggtctgtaatattgattgtttttataacagtgttaaaatatggaagaccgcaattcagctggctcgtttatggcattaaaatgctgatcatgtggctattatggcctattgttctagcgcttacgatttttaatgcatactctgagtaccaagtttccagatatgtaatgttcggctttagtgttgcaggtgcagttgtaacgtttgcactatggatgatgtattttgtgagatctattcagctgtatagacggaccaaatcatggtggtcttttaatcctgaaaccaatgcgattctttgtgtcaatgcattgggtagaagctatgtactccctcttgatggcactcctacaggtgttactcttaccctactttcaggaaatctatacgctgaaggttttaaaatggctggtggtcttaccatcgagcatttgcctaaatatgtcatgattgctacgcctagtagaaccatcgtttacacattagttggaaaacaactaaaggcaactactgccactggatgggcttactatgtaaaatctaaagctggtgattactcaacagaagcacgtactgataatttgagtgaacatgaaaaattattacatatggtgggcagcggcgcgaccaactttagcctgctgaaacaggcgggcgatgtggaagaaaacccgggcccgatggccacacagggacaacgcgtcaactggggagatgaaccttccaaaagacgtggtcgttctaactctcgtggtcggaagaataacactatacctctttcattcttcaatcccatccaactcgaaccaggatcaaaattttggagcgtatgtccgagagattttgttcccaagggaataggtaacaaggatcaacaaattggttattggaatagacaagagcgttaccgcattgtcaaaggtcagcgtaaggaacttcctgagaggtggtttttctacttcttaggcacaggacctcaagctgatgctaaatttaaagacaagattgatggagtcttctgggttgcaaaggatggtgccatgaataaaccaacaacacttggcactcgtggtaccaacaatgaatccaaaccactgaaatttgatggtaagataccaccgcaatttcagcttgaagtgaaccgatctaggaacaactcaagaagtggttctcagtctagatctgtctctagaaacaggtctcaatccagaggaagacaacaatccaataatcagaataatgttgaggatacaattgtagctgtgcttcagaaattaggtgttactgaaaagcaaaggtcacgttctaaatctagagatcgtggtgactctaaacctagagacacaacacctaataatgccaacaaacacacctggaagaagactgcaggtaaaggtgatgtgacaaatttctatggtgctagaagtgcttcagctaactttggtgatagtgatctcgttgccaacggtaacgctgccaaatcctaccctcagatagctgaatgcgttccatcagtgtctagcatgctcttcggtagtcaatggtctgctgaagatgatggtgatcaagtgaaagtcacgctcactcatacctattacctgccaaaagatgatgccaaaaccagccaattcctagaacagattgacgcttacaagcggccatctcaagtggctaaagatcagaggcaaagaaaatctcgttctaagtctgctgagaagaagcctgaggaattgtctgtaactcttgtagaggcatatacggatgtgtttgatgacacacaggttgagatgattgatgaggttacgaactaa

SEQ ID NO: 15 - DNA, 1983 bp, synthetic construct
  source 1..1983: mol_type = other DNA
atggccacacagggacaacgcgtcaactggggagatgaaccttccaaaagacgtggtcgttctaactctcgtggtcggaagaataacactatacctctttcattcttcaatcccatccaactcgaaccaggatcaaaattttggagcgtatgtccgagagattttgttcccaagggaataggtaacaaggatcaacaaattggttattggaatagacaagagcgttaccgcattgtcaaaggtcagcgtaaggaacttcctgagaggtggtttttctacttcttaggcacaggacctcaagctgatgctaaatttaaagacaagattgatggagtcttctgggttgcaaaggatggtgccatgaataaaccaacaacacttggcactcgtggtaccaacaatgaatccaaaccactgaaatttgatggtaagataccaccgcaatttcagcttgaagtgaaccgatctaggaacaactcaagaagtggttctcagtctagatctgtctctagaaacaggtctcaatccagaggaagacaacaatccaataatcagaataatgttgaggatacaattgtagctgtgcttcagaaattaggtgttactgaaaagcaaaggtcacgttctaaatctagagatcgtggtgactctaaacctagagacacaacacctaataatgccaacaaacacacctggaagaagactgcaggtaaaggtgatgtgacaaatttctatggtgctagaagtgcttcagctaactttggtgatagtgatctcgttgccaacggtaacgctgccaaatcctaccctcagatagctgaatgcgttccatcagtgtctagcatgctcttcggtagtcaatggtctgctgaagatgatggtgatcaagtgaaagtcacgctcactcatacctattacctgccaaaagatgatgccaaaaccagccaattcctagaacagattgacgcttacaagcggccatctcaagtggctaaagatcagaggcaaagaaaatctcgttctaagtctgctgagaagaagcctgaggaattgtctgtaactcttgtagaggcatatacggatgtgtttgatgacacacaggttgagatgattgatgaggttacgaacggcagcggcgcgaccaactttagcctgctgaaacaggcgggcgatgtggaagaaaacccgggcccgatgaagtacattttgttaatactcgcgtgcattattgcatgcgtttatggagaacgctactgtgccatgcaaaatacaggctcgcagtgcattaatggcacagattcatcatgtagcacctgttttgaacgtggtggtcttatttggcatctggctaactggaacttcagctggtctgtaatattgattgtttttataacagtgttaaaatatggaagaccgcaattcagctggctcgtttatggcattaaaatgctgatcatgtggctattatggcctattgttctagcgcttacgatttttaatgcatactctgagtaccaagtttccagatatgtaatgttcggctttagtgttgcaggtgcagttgtaacgtttgcactatggatgatgtattttgtgagatctattcagctgtatagacggaccaaatcatggtggtcttttaatcctgaaaccaatgcgattctttgtgtcaatgcattgggtagaagctatgtactccctcttgatggcactcctacaggtgttactcttaccctactttcaggaaatctatacgctgaaggttttaaaatggctggtggtcttaccatcgagcatttgcctaaatatgtcatgattgctacgcctagtagaaccatcgtttacacattagttggaaaacaactaaaggcaactactgccactggatgggcttactatgtaaaatctaaagctggtgattactcaacagaagcacgtactgataatttgagtgaacatgaaaaattattacatatggtgtaa

SEQ ID NO: 16 - DNA, 6399 bp, synthetic construct
  source 1..6399: mol_type = other DNA
atggccacacagggacaacgcgtcaactggggagatgaaccttccaaaagacgtggtcgttctaactctcgtggtcggaagaataacactatacctctttcattcttcaatcccatccaactcgaaccaggatcaaaattttggagcgtatgtccgagagattttgttcccaagggaataggtaacaaggatcaacaaattggttattggaatagacaagagcgttaccgcattgtcaaaggtcagcgtaaggaacttcctgagaggtggtttttctacttcttaggcacaggacctcaagctgatgctaaatttaaagacaagattgatggagtcttctgggttgcaaaggatggtgccatgaataaaccaacaacacttggcactcgtggtaccaacaatgaatccaaaccactgaaatttgatggtaagataccaccgcaatttcagcttgaagtgaaccgatctaggaacaactcaagaagtggttctcagtctagatctgtctctagaaacaggtctcaatccagaggaagacaacaatccaataatcagaataatgttgaggatacaattgtagctgtgcttcagaaattaggtgttactgaaaagcaaaggtcacgttctaaatctagagatcgtggtgactctaaacctagagacacaacacctaataatgccaacaaacacacctggaagaagactgcaggtaaaggtgatgtgacaaatttctatggtgctagaagtgcttcagctaactttggtgatagtgatctcgttgccaacggtaacgctgccaaatcctaccctcagatagctgaatgcgttccatcagtgtctagcatgctcttcggtagtcaatggtctgctgaagatgatggtgatcaagtgaaagtcacgctcactcatacctattacctgccaaaagatgatgccaaaaccagccaattcctagaacagattgacgcttacaagcggccatctcaagtggctaaagatcagaggcaaagaaaatctcgttctaagtctgctgagaagaagcctgaggaattgtctgtaactcttgtagaggcatatacggatgtgtttgatgacacacaggttgagatgattgatgaggttacgaacggcagcggcgaaggccgcggcagcctgctgacctgcggcgatgtggaagaaaacccgggcccgatgaagtacattttgttaatactcgcgtgcattattgcatgcgtttatggagaacgctactgtgccatgcaaaatacaggctcgcagtgcattaatggcacagattcatcatgtagcacctgttttgaacgtggtggtcttatttggcatctggctaactggaacttcagctggtctgtaatattgattgtttttataacagtgttaaaatatggaagaccgcaattcagctggctcgtttatggcattaaaatgctgatcatgtggctattatggcctattgttctagcgcttacgatttttaatgcatactctgagtaccaagtttccagatatgtaatgttcggctttagtgttgcaggtgcagttgtaacgtttgcactatggatgatgtattttgtgagatctattcagctgtatagacggaccaaatcatggtggtcttttaatcctgaaaccaatgcgattctttgtgtcaatgcattgggtagaagctatgtactccctcttgatggcactcctacaggtgttactcttaccctactttcaggaaatctatacgctgaaggttttaaaatggctggtggtcttaccatcgagcatttgcctaaatatgtcatgattgctacgcctagtagaaccatcgtttacacattagttggaaaacaactaaaggcaactactgccactggatgggcttactatgtaaaatctaaagctggtgattactcaacagaagcacgtactgataatttgagtgaacatgaaaaattattacatatggtgggcagcggcgaaggccgcggcagcctgctgacctgcggcgatgtggaagaaaacccgggcccgatgattgtgctcgtaacttgcctcttgttgttatgttcataccacacagttttgagtacaacaaataatgaatgcatacaagttaacgtaacacaattggctggcaatgaaaaccttatcagagattttctgtttagtaactttaaagaagaaggaagtgtagttgttggtggttattaccctacagaggtgtggtacaactgctctagaacagctcgaactactgcctttcagtattttaataatatacatgccttttattttgttatggaagccatggaaaatagcactggtaatgcacgtggtaaaccattattatttcatgtgcatggtgagcctgttagtgttattatatcggcttatagggatgatgtgcaacaaaggccccttttaaaacatgggttagtgtgcataactaaaaatcgccatattaactatgaacaattcacctccaaccagtggaattccacatgtacgggtgctgacagaaaaattcctttctctgtcatacccacggacaatggaacaaaaatctatggtcttgagtggaatgatgactttgttacagcttatattagtggtcgttcttatcacttgaacatcaatactaattggtttaacaatgtcacacttttgtattcacgctcaagcactgctacctgggaatacagtgctgcatatgcttaccaaggtgtttctaacttcacttattacaagttaaataacaccaatggtctaaaaacctatgaattatgtgaagattatgaacattgcactggctatgctaccaatgtatttgctccgacatcaggtggttacatacctgatggatttagttttaacaattggttcttgcttacaaatagttccacttttgttagtggcaggtttgtaacaaatcaaccattattgattaattgcttgtggccagtgcccagttttggtgtagcagcacaagaattttgttttgaaggtgcacagtttagccaatgtaatggtgtgtctttaaataacacagtggatgttattagattcaaccttaatttcactgcagatgtacaatctggtatgggtgctacagtattttcactgaatacaacaggtggtgtcattcttgaaatttcatgttatagtgacacagtgagtgagtctagttcttacagttatggtgaaatcccgttcggcataactgacggaccacgatactgttatgtactttacaatggcacagctcttaaatatttaggaacattaccacccagtgtaaaggaaattgctattagtaagtggggccatttttatattaatggttacaatttctttagcacatttcctattggttgtatatcttttaatttaaccactggtgttagtggagctttttggacaattgcttacacatcgtatactgaagcattagtacaagttgaaaacacagctattaaaaatgtgacgtattgtaacagtcacattaataacattaaatgttctcaacttactgctaatttgaataatggattttatcctgttgcttcaagtgaagtaggtttcgttaataagagtgttgtgttattacctagctttttcacatacaccgctgtcaatataaccattgatcttggtatgaagcttagtggttatggtcaacccatagcctcgacactaagtaacatcacactaccaatgcaggataacaatactgatgtgtactgtattcgttctaaccaattctcagtttatgttcattccacttgcaaaagttctttatgggacaatatttttaatcaagactgcacggatgttttagaggctacagctgttataaaaactggtacttgtcctttctcatttgataaattgaacaattacttgacttttaacaagttctgtttgtcgttgagtcctgttggtgctaattgcaagtttgatgttgctgcacgtacaagaaccaatgagcaggttgttagaagtctatatgtaatatatgaagaaggagacaacatagtgggtgtaccgtctgataatagcggtctgcacgatttgtctgtgctacacctagactcctgtacagattacaatatatatggtagaactggtgttggtattattagacgaactaacagtacgctacttagtggcttatattacacatcactatcaggtgatttgttaggctttaaaaatgttagtgatggtgtcatttattctgtgacgccatgtgatgtaagcgcacaagcggctgttattgatggtgccatagttggagctatgacttccattaacagtgaactgttaggtctaacacattggacaacgacacctaatttttattactactctatatataattacacaagtgagaggactcgtgacactgcaattgacagtaacgatgttgattgtgaacctgtcataacctattctaatataggtgtttgtaaaaatggtgctttggtttttattaacgtcacacattctgacggagacgtgcaaccaattagcactggtaatgtcacgatacctacaaattttaccatatctgtgcaagttgaatacatgcaggtttacactacaccagtatcaatagattgtgcaagatacgtttgtaatggtaaccctagatgtaacaaattgttaacacaatatgtgtctgcatgtcaaactattgaacaagcacttgcaatgggtgccagacttgaaaacatggaggttgattccatgttgtttgtctcggaaaatgcccttaaattggcatctgttgaggcgttcaatagtacagaaaatttagattctatttacaaagaatggcctagcataggtggttcttggctaggaggtctaaaagatatactaccgtcccataatagcaaacgtaagtatggttctgctatagaagatttgctttttgataaagttgtaacatctggtttaggtacagttgatgaagattataaacgttgtactggtggttacgacatagcagacttggtgtgtgctcaatattacaatggcatcatggttctaccaggtgtagctaatgctgacaagatgactatgtacacagcatcacttgcaggtggtataacattaggtgcacttggtggtggcgccgtggctataccttttgcagtagcagtacaggctagacttaattatgttgctctacaaactgatgtattgaataaaaaccaacagatcctggctaatgccttcaatcaagctattggtaacattacacaggcttttggtaaggttaatgatgctatacatcaaacatcacaaggtcttgccactgttgctaaagcgttggcaaaagtgcaagatgttgtcaacacacaagggcaagctttaagtcaccttacagtacaattgcaaaataattttcaagccattagtagttctattagtgatatttataacaggcttgacgaactgagtgctgatgcacaagttgataggctgattacaggtagacttacagcacttaatgcatttgtgtctcagactctaaccagacaagcagaggttagggctagtagacaacttgccaaagacaaggttaatgaatgtgttaggtctcagtctcagagattcggattctgtggtaatggtacacatttgttttcactagcaaatgcagcaccaaatggcatgattttctttcatacagtactattaccaacagcttatgaaactgtaacagcttggtcaggtatttgtgcttcagatggcgatcgcactttcggacttgtcgttaaagatgtgcagttgacgttgtttcgtaatctagatgacaagttctatttgacccccagaactatgtatcagcctagagttgcaactagttctgattttgttcaaattgaagggtgtgatgtgttgtttgtcaacgcgactgtaattgatttgcctagtattatacctgactatattgacattaatcaaactgttcaagacatattagaaaattacagaccaaactggactgtacctgaatttacacttgatattttcaacgcaacctatttaaatctgactggtgaaattgatgacttagagtttaggtcagaaaagctacataacactacagtagaacttgccattctcattgataacattaataatacattagtcaatcttgaatggctcaatagaattgaaacttatgtaaaatggccttggtatgtgtggctactgataggtttagtagtagtattttgcataccattactgctattttgctgttttagcacaggttgttgtggatgcataggttgtttaggaagttgttgtcactctatatgtagtagaagacaatttgaaaattatgaaccaattgaaaaagtgcatgtccactaa

SEQ ID NO: 17 - DNA, 6402 bp, synthetic construct
  source 1..6402: mol_type = other DNA
atggccacacagggacaacgcgtcaactggggagatgaaccttccaaaagacgtggtcgttctaactctcgtggtcggaagaataacactatacctctttcattcttcaatcccatccaactcgaaccaggatcaaaattttggagcgtatgtccgagagattttgttcccaagggaataggtaacaaggatcaacaaattggttattggaatagacaagagcgttaccgcattgtcaaaggtcagcgtaaggaacttcctgagaggtggtttttctacttcttaggcacaggacctcaagctgatgctaaatttaaagacaagattgatggagtcttctgggttgcaaaggatggtgccatgaataaaccaacaacacttggcactcgtggtaccaacaatgaatccaaaccactgaaatttgatggtaagataccaccgcaatttcagcttgaagtgaaccgatctaggaacaactcaagaagtggttctcagtctagatctgtctctagaaacaggtctcaatccagaggaagacaacaatccaataatcagaataatgttgaggatacaattgtagctgtgcttcagaaattaggtgttactgaaaagcaaaggtcacgttctaaatctagagatcgtggtgactctaaacctagagacacaacacctaataatgccaacaaacacacctggaagaagactgcaggtaaaggtgatgtgacaaatttctatggtgctagaagtgcttcagctaactttggtgatagtgatctcgttgccaacggtaacgctgccaaatcctaccctcagatagctgaatgcgttccatcagtgtctagcatgctcttcggtagtcaatggtctgctgaagatgatggtgatcaagtgaaagtcacgctcactcatacctattacctgccaaaagatgatgccaaaaccagccaattcctagaacagattgacgcttacaagcggccatctcaagtggctaaagatcagaggcaaagaaaatctcgttctaagtctgctgagaagaagcctgaggaattgtctgtaactcttgtagaggcatatacggatgtgtttgatgacacacaggttgagatgattgatgaggttacgaacggcagcggcgaaggccgcggcagcctgctgacctgcggcgatgtggaagaaaacccgggcccgatgattgtgctcgtaacttgcctcttgttgttatgttcataccacacagttttgagtacaacaaataatgaatgcatacaagttaacgtaacacaattggctggcaatgaaaaccttatcagagattttctgtttagtaactttaaagaagaaggaagtgtagttgttggtggttattaccctacagaggtgtggtacaactgctctagaacagctcgaactactgcctttcagtattttaataatatacatgccttttattttgttatggaagccatggaaaatagcactggtaatgcacgtggtaaaccattattatttcatgtgcatggtgagcctgttagtgttattatatcggcttatagggatgatgtgcaacaaaggccccttttaaaacatgggttagtgtgcataactaaaaatcgccatattaactatgaacaattcacctccaaccagtggaattccacatgtacgggtgctgacagaaaaattcctttctctgtcatacccacggacaatggaacaaaaatctatggtcttgagtggaatgatgactttgttacagcttatattagtggtcgttcttatcacttgaacatcaatactaattggtttaacaatgtcacacttttgtattcacgctcaagcactgctacctgggaatacagtgctgcatatgcttaccaaggtgtttctaacttcacttattacaagttaaataacaccaatggtctaaaaacctatgaattatgtgaagattatgaacattgcactggctatgctaccaatgtatttgctccgacatcaggtggttacatacctgatggatttagttttaacaattggttcttgcttacaaatagttccacttttgttagtggcaggtttgtaacaaatcaaccattattgattaattgcttgtggccagtgcccagttttggtgtagcagcacaagaattttgttttgaaggtgcacagtttagccaatgtaatggtgtgtctttaaataacacagtggatgttattagattcaaccttaatttcactgcagatgtacaatctggtatgggtgctacagtattttcactgaatacaacaggtggtgtcattcttgaaatttcatgttatagtgacacagtgagtgagtctagttcttacagttatggtgaaatcccgttcggcataactgacggaccacgatactgttatgtactttacaatggcacagctcttaaatatttaggaacattaccacccagtgtaaaggaaattgctattagtaagtggggccatttttatattaatggttacaatttctttagcacatttcctattggttgtatatcttttaatttaaccactggtgttagtggagctttttggacaattgcttacacatcgtatactgaagcattagtacaagttgaaaacacagctattaaaaatgtgacgtattgtaacagtcacattaataacattaaatgttctcaacttactgctaatttgaataatggattttatcctgttgcttcaagtgaagtaggtttcgttaataagagtgttgtgttattacctagctttttcacatacaccgctgtcaatataaccattgatcttggtatgaagcttagtggttatggtcaacccatagcctcgacactaagtaacatcacactaccaatgcaggataacaatactgatgtgtactgtattcgttctaaccaattctcagtttatgttcattccacttgcaaaagttctttatgggacaatatttttaatcaagactgcacggatgttttagaggctacagctgttataaaaactggtacttgtcctttctcatttgataaattgaacaattacttgacttttaacaagttctgtttgtcgttgagtcctgttggtgctaattgcaagtttgatgttgctgcacgtacaagaaccaatgagcaggttgttagaagtctatatgtaatatatgaagaaggagacaacatagtgggtgtaccgtctgataatagcggtctgcacgatttgtctgtgctacacctagactcctgtacagattacaatatatatggtagaactggtgttggtattattagacgaactaacagtacgctacttagtggcttatattacacatcactatcaggtgatttgttaggctttaaaaatgttagtgatggtgtcatttattctgtgacgccatgtgatgtaagcgcacaagcggctgttattgatggtgccatagttggagctatgacttccattaacagtgaactgttaggtctaacacattggacaacgacacctaatttttattactactctatatataattacacaagtgagaggactcgtgacactgcaattgacagtaacgatgttgattgtgaacctgtcataacctattctaatataggtgtttgtaaaaatggtgctttggtttttattaacgtcacacattctgacggagacgtgcaaccaattagcactggtaatgtcacgatacctacaaattttaccatatctgtgcaagttgaatacatgcaggtttacactacaccagtatcaatagattgtgcaagatacgtttgtaatggtaaccctagatgtaacaaattgttaacacaatatgtgtctgcatgtcaaactattgaacaagcacttgcaatgggtgccagacttgaaaacatggaggttgattccatgttgtttgtctcggaaaatgcccttaaattggcatctgttgaggcgttcaatagtacagaaaatttagattctatttacaaagaatggcctagcataggtggttcttggctaggaggtctaaaagatatactaccgtcccataatagcaaacgtaagtatggttctgctatagaagatttgctttttgataaagttgtaacatctggtttaggtacagttgatgaagattataaacgttgtactggtggttacgacatagcagacttggtgtgtgctcaatattacaatggcatcatggttctaccaggtgtagctaatgctgacaagatgactatgtacacagcatcacttgcaggtggtataacattaggtgcacttggtggtggcgccgtggctataccttttgcagtagcagtacaggctagacttaattatgttgctctacaaactgatgtattgaataaaaaccaacagatcctggctaatgccttcaatcaagctattggtaacattacacaggcttttggtaaggttaatgatgctatacatcaaacatcacaaggtcttgccactgttgctaaagcgttggcaaaagtgcaagatgttgtcaacacacaagggcaagctttaagtcaccttacagtacaattgcaaaataattttcaagccattagtagttctattagtgatatttataacaggcttgacgaactgagtgctgatgcacaagttgataggctgattacaggtagacttacagcacttaatgcatttgtgtctcagactctaaccagacaagcagaggttagggctagtagacaacttgccaaagacaaggttaatgaatgtgttaggtctcagtctcagagattcggattctgtggtaatggtacacatttgttttcactagcaaatgcagcaccaaatggcatgattttctttcatacagtactattaccaacagcttatgaaactgtaacagcttggtcaggtatttgtgcttcagatggcgatcgcactttcggacttgtcgttaaagatgtgcagttgacgttgtttcgtaatctagatgacaagttctatttgacccccagaactatgtatcagcctagagttgcaactagttctgattttgttcaaattgaagggtgtgatgtgttgtttgtcaacgcgactgtaattgatttgcctagtattatacctgactatattgacattaatcaaactgttcaagacatattagaaaattacagaccaaactggactgtacctgaatttacacttgatattttcaacgcaacctatttaaatctgactggtgaaattgatgacttagagtttaggtcagaaaagctacataacactacagtagaacttgccattctcattgataacattaataatacattagtcaatcttgaatggctcaatagaattgaaacttatgtaaaatggccttggtatgtgtggctactgataggtttagtagtagtattttgcataccattactgctattttgctgttttagcacaggttgttgtggatgcataggttgtttaggaagttgttgtcactctatatgtagtagaagacaatttgaaaattatgaaccaattgaaaaagtgcatgtccactaaggcagcggcgaaggccgcggcagcctgctgacctgcggcgatgtggaagaaaacccgggcccgatgaagtacattttgttaatactcgcgtgcattattgcatgcgtttatggagaacgctactgtgccatgcaaaatacaggctcgcagtgcattaatggcacagattcatcatgtagcacctgttttgaacgtggtggtcttatttggcatctggctaactggaacttcagctggtctgtaatattgattgtttttataacagtgttaaaatatggaagaccgcaattcagctggctcgtttatggcattaaaatgctgatcatgtggctattatggcctattgttctagcgcttacgatttttaatgcatactctgagtaccaagtttccagatatgtaatgttcggctttagtgttgcaggtgcagttgtaacgtttgcactatggatgatgtattttgtgagatctattcagctgtatagacggaccaaatcatggtggtcttttaatcctgaaaccaatgcgattctttgtgtcaatgcattgggtagaagctatgtactccctcttgatggcactcctacaggtgttactcttaccctactttcaggaaatctatacgctgaaggttttaaaatggctggtggtcttaccatcgagcatttgcctaaatatgtcatgattgctacgcctagtagaaccatcgtttacacattagttggaaaacaactaaaggcaactactgccactggatgggcttactatgtaaaatctaaagctggtgattactcaacagaagcacgtactgataatttgagtgaacatgaaaaattattacatatggtgtaa

SEQ ID NO: 18 - DNA, 4065 bp, synthetic construct
  source 1..4065: mol_type = other DNA
atggccacacagggacaacgcgtcaactggggagatgaaccttccaaaagacgtggtcgttctaactctcgtggtcggaagaataacactatacctctttcattcttcaatcccatccaactcgaaccaggatcaaaattttggagcgtatgtccgagagattttgttcccaagggaataggtaacaaggatcaacaaattggttattggaatagacaagagcgttaccgcattgtcaaaggtcagcgtaaggaacttcctgagaggtggtttttctacttcttaggcacaggacctcaagctgatgctaaatttaaagacaagattgatggagtcttctgggttgcaaaggatggtgccatgaataaaccaacaacacttggcactcgtggtaccaacaatgaatccaaaccactgaaatttgatggtaagataccaccgcaatttcagcttgaagtgaaccgatctaggaacaactcaagaagtggttctcagtctagatctgtctctagaaacaggtctcaatccagaggaagacaacaatccaataatcagaataatgttgaggatacaattgtagctgtgcttcagaaattaggtgttactgaaaagcaaaggtcacgttctaaatctagagatcgtggtgactctaaacctagagacacaacacctaataatgccaacaaacacacctggaagaagactgcaggtaaaggtgatgtgacaaatttctatggtgctagaagtgcttcagctaactttggtgatagtgatctcgttgccaacggtaacgctgccaaatcctaccctcagatagctgaatgcgttccatcagtgtctagcatgctcttcggtagtcaatggtctgctgaagatgatggtgatcaagtgaaagtcacgctcactcatacctattacctgccaaaagatgatgccaaaaccagccaattcctagaacagattgacgcttacaagcggccatctcaagtggctaaagatcagaggcaaagaaaatctcgttctaagtctgctgagaagaagcctgaggaattgtctgtaactcttgtagaggcatatacggatgtgtttgatgacacacaggttgagatgattgatgaggttacgaacggcagcggcgaaggccgcggcagcctgctgacctgcggcgatgtggaagaaaacccgggcccgatgaagtacattttgttaatactcgcgtgcattattgcatgcgtttatggagaacgctactgtgccatgcaaaatacaggctcgcagtgcattaatggcacagattcatcatgtagcacctgttttgaacgtggtggtcttatttggcatctggctaactggaacttcagctggtctgtaatattgattgtttttataacagtgttaaaatatggaagaccgcaattcagctggctcgtttatggcattaaaatgctgatcatgtggctattatggcctattgttctagcgcttacgatttttaatgcatactctgagtaccaagtttccagatatgtaatgttcggctttagtgttgcaggtgcagttgtaacgtttgcactatggatgatgtattttgtgagatctattcagctgtatagacggaccaaatcatggtggtcttttaatcctgaaaccaatgcgattctttgtgtcaatgcattgggtagaagctatgtactccctcttgatggcactcctacaggtgttactcttaccctactttcaggaaatctatacgctgaaggttttaaaatggctggtggtcttaccatcgagcatttgcctaaatatgtcatgattgctacgcctagtagaaccatcgtttacacattagttggaaaacaactaaaggcaactactgccactggatgggcttactatgtaaaatctaaagctggtgattactcaacagaagcacgtactgataatttgagtgaacatgaaaaattattacatatggtgggcagcggcgaaggccgcggcagcctgctgacctgcggcgatgtggaagaaaacccgggcccgatgtctatatataattacacaagtgagaggactcgtgacactgcaattgacagtaacgatgttgattgtgaacctgtcataacctattctaatataggtgtttgtaaaaatggtgctttggtttttattaacgtcacacattctgacggagacgtgcaaccaattagcactggtaatgtcacgatacctacaaattttaccatatctgtgcaagttgaatacatgcaggtttacactacaccagtatcaatagattgtgcaagatacgtttgtaatggtaaccctagatgtaacaaattgttaacacaatatgtgtctgcatgtcaaactattgaacaagcacttgcaatgggtgccagacttgaaaacatggaggttgattccatgttgtttgtctcggaaaatgcccttaaattggcatctgttgaggcgttcaatagtacagaaaatttagattctatttacaaagaatggcctagcataggtggttcttggctaggaggtctaaaagatatactaccgtcccataatagcaaacgtaagtatggttctgctatagaagatttgctttttgataaagttgtaacatctggtttaggtacagttgatgaagattataaacgttgtactggtggttacgacatagcagacttggtgtgtgctcaatattacaatggcatcatggttctaccaggtgtagctaatgctgacaagatgactatgtacacagcatcacttgcaggtggtataacattaggtgcacttggtggtggcgccgtggctataccttttgcagtagcagtacaggctagacttaattatgttgctctacaaactgatgtattgaataaaaaccaacagatcctggctaatgccttcaatcaagctattggtaacattacacaggcttttggtaaggttaatgatgctatacatcaaacatcacaaggtcttgccactgttgctaaagcgttggcaaaagtgcaagatgttgtcaacacacaagggcaagctttaagtcaccttacagtacaattgcaaaataattttcaagccattagtagttctattagtgatatttataacaggcttgacgaactgagtgctgatgcacaagttgataggctgattacaggtagacttacagcacttaatgcatttgtgtctcagactctaaccagacaagcagaggttagggctagtagacaacttgccaaagacaaggttaatgaatgtgttaggtctcagtctcagagattcggattctgtggtaatggtacacatttgttttcactagcaaatgcagcaccaaatggcatgattttctttcatacagtactattaccaacagcttatgaaactgtaacagcttggtcaggtatttgtgcttcagatggcgatcgcactttcggacttgtcgttaaagatgtgcagttgacgttgtttcgtaatctagatgacaagttctatttgacccccagaactatgtatcagcctagagttgcaactagttctgattttgttcaaattgaagggtgtgatgtgttgtttgtcaacgcgactgtaattgatttgcctagtattatacctgactatattgacattaatcaaactgttcaagacatattagaaaattacagaccaaactggactgtacctgaatttacacttgatattttcaacgcaacctatttaaatctgactggtgaaattgatgacttagagtttaggtcagaaaagctacataacactacagtagaacttgccattctcattgataacattaataatacattagtcaatcttgaatggctcaatagaattgaaacttatgtaaaatggccttggtatgtgtggctactgataggtttagtagtagtattttgcataccattactgctattttgctgttttagcacaggttgttgtggatgcataggttgtttaggaagttgttgtcactctatatgtagtagaagacaatttgaaaattatgaaccaattgaaaaagtgcatgtccactaa

SEQ ID NO: 19 - DNA, 4065 bp, synthetic construct
  source 1..4065: mol_type = other DNA
atggccacacagggacaacgcgtcaactggggagatgaaccttccaaaagacgtggtcgttctaactctcgtggtcggaagaataacactatacctctttcattcttcaatcccatccaactcgaaccaggatcaaaattttggagcgtatgtccgagagattttgttcccaagggaataggtaacaaggatcaacaaattggttattggaatagacaagagcgttaccgcattgtcaaaggtcagcgtaaggaacttcctgagaggtggtttttctacttcttaggcacaggacctcaagctgatgctaaatttaaagacaagattgatggagtcttctgggttgcaaaggatggtgccatgaataaaccaacaacacttggcactcgtggtaccaacaatgaatccaaaccactgaaatttgatggtaagataccaccgcaatttcagcttgaagtgaaccgatctaggaacaactcaagaagtggttctcagtctagatctgtctctagaaacaggtctcaatccagaggaagacaacaatccaataatcagaataatgttgaggatacaattgtagctgtgcttcagaaattaggtgttactgaaaagcaaaggtcacgttctaaatctagagatcgtggtgactctaaacctagagacacaacacctaataatgccaacaaacacacctggaagaagactgcaggtaaaggtgatgtgacaaatttctatggtgctagaagtgcttcagctaactttggtgatagtgatctcgttgccaacggtaacgctgccaaatcctaccctcagatagctgaatgcgttccatcagtgtctagcatgctcttcggtagtcaatggtctgctgaagatgatggtgatcaagtgaaagtcacgctcactcatacctattacctgccaaaagatgatgccaaaaccagccaattcctagaacagattgacgcttacaagcggccatctcaagtggctaaagatcagaggcaaagaaaatctcgttctaagtctgctgagaagaagcctgaggaattgtctgtaactcttgtagaggcatatacggatgtgtttgatgacacacaggttgagatgattgatgaggttacgaacggcagcggcgaaggccgcggcagcctgctgacctgcggcgatgtggaagaaaacccgggcccgatgtctatatataattacacaagtgagaggactcgtgacactgcaattgacagtaacgatgttgattgtgaacctgtcataacctattctaatataggtgtttgtaaaaatggtgctttggtttttattaacgtcacacattctgacggagacgtgcaaccaattagcactggtaatgtcacgatacctacaaattttaccatatctgtgcaagttgaatacatgcaggtttacactacaccagtatcaatagattgtgcaagatacgtttgtaatggtaaccctagatgtaacaaattgttaacacaatatgtgtctgcatgtcaaactattgaacaagcacttgcaatgggtgccagacttgaaaacatggaggttgattccatgttgtttgtctcggaaaatgcccttaaattggcatctgttgaggcgttcaatagtacagaaaatttagattctatttacaaagaatggcctagcataggtggttcttggctaggaggtctaaaagatatactaccgtcccataatagcaaacgtaagtatggttctgctatagaagatttgctttttgataaagttgtaacatctggtttaggtacagttgatgaagattataaacgttgtactggtggttacgacatagcagacttggtgtgtgctcaatattacaatggcatcatggttctaccaggtgtagctaatgctgacaagatgactatgtacacagcatcacttgcaggtggtataacattaggtgcacttggtggtggcgccgtggctataccttttgcagtagcagtacaggctagacttaattatgttgctctacaaactgatgtattgaataaaaaccaacagatcctggctaatgccttcaatcaagctattggtaacattacacaggcttttggtaaggttaatgatgctatacatcaaacatcacaaggtcttgccactgttgctaaagcgttggcaaaagtgcaagatgttgtcaacacacaagggcaagctttaagtcaccttacagtacaattgcaaaataattttcaagccattagtagttctattagtgatatttataacaggcttgacgaactgagtgctgatgcacaagttgataggctgattacaggtagacttacagcacttaatgcatttgtgtctcagactctaaccagacaagcagaggttagggctagtagacaacttgccaaagacaaggttaatgaatgtgttaggtctcagtctcagagattcggattctgtggtaatggtacacatttgttttcactagcaaatgcagcaccaaatggcatgattttctttcatacagtactattaccaacagcttatgaaactgtaacagcttggtcaggtatttgtgcttcagatggcgatcgcactttcggacttgtcgttaaagatgtgcagttgacgttgtttcgtaatctagatgacaagttctatttgacccccagaactatgtatcagcctagagttgcaactagttctgattttgttcaaattgaagggtgtgatgtgttgtttgtcaacgcgactgtaattgatttgcctagtattatacctgactatattgacattaatcaaactgttcaagacatattagaaaattacagaccaaactggactgtacctgaatttacacttgatattttcaacgcaacctatttaaatctgactggtgaaattgatgacttagagtttaggtcagaaaagctacataacactacagtagaacttgccattctcattgataacattaataatacattagtcaatcttgaatggctcaatagaattgaaacttatgtaaaatggccttggtatgtgtggctactgataggtttagtagtagtattttgcataccattactgctattttgctgttttagcacaggttgttgtggatgcataggttgtttaggaagttgttgtcactctatatgtagtagaagacaatttgaaaattatgaaccaattgaaaaagtgcatgtccacggcagcggcgaaggccgcggcagcctgctgacctgcggcgatgtggaagaaaacccgggcccgatgaagtacattttgttaatactcgcgtgcattattgcatgcgtttatggagaacgctactgtgccatgcaaaatacaggctcgcagtgcattaatggcacagattcatcatgtagcacctgttttgaacgtggtggtcttatttggcatctggctaactggaacttcagctggtctgtaatattgattgtttttataacagtgttaaaatatggaagaccgcaattcagctggctcgtttatggcattaaaatgctgatcatgtggctattatggcctattgttctagcgcttacgatttttaatgcatactctgagtaccaagtttccagatatgtaatgttcggctttagtgttgcaggtgcagttgtaacgtttgcactatggatgatgtattttgtgagatctattcagctgtatagacggaccaaatcatggtggtcttttaatcctgaaaccaatgcgattctttgtgtcaatgcattgggtagaagctatgtactccctcttgatggcactcctacaggtgttactcttaccctactttcaggaaatctatacgctgaaggttttaaaatggctggtggtcttaccatcgagcatttgcctaaatatgtcatgattgctacgcctagtagaaccatcgtttacacattagttggaaaacaactaaaggcaactactgccactggatgggcttactatgtaaaatctaaagctggtgattactcaacagaagcacgtactgataatttgagtgaacatgaaaaattattacatatggtgtaa

SEQ ID NO: 20 - DNA, 6405 bp, synthetic construct
  source 1..6405: mol_type = other DNA
atggccacacagggacaacgcgtcaactggggagatgaaccttccaaaagacgtggtcgttctaactctcgtggtcggaagaataacactatacctctttcattcttcaatcccatccaactcgaaccaggatcaaaattttggagcgtatgtccgagagattttgttcccaagggaataggtaacaaggatcaacaaattggttattggaatagacaagagcgttaccgcattgtcaaaggtcagcgtaaggaacttcctgagaggtggtttttctacttcttaggcacaggacctcaagctgatgctaaatttaaagacaagattgatggagtcttctgggttgcaaaggatggtgccatgaataaaccaacaacacttggcactcgtggtaccaacaatgaatccaaaccactgaaatttgatggtaagataccaccgcaatttcagcttgaagtgaaccgatctaggaacaactcaagaagtggttctcagtctagatctgtctctagaaacaggtctcaatccagaggaagacaacaatccaataatcagaataatgttgaggatacaattgtagctgtgcttcagaaattaggtgttactgaaaagcaaaggtcacgttctaaatctagagatcgtggtgactctaaacctagagacacaacacctaataatgccaacaaacacacctggaagaagactgcaggtaaaggtgatgtgacaaatttctatggtgctagaagtgcttcagctaactttggtgatagtgatctcgttgccaacggtaacgctgccaaatcctaccctcagatagctgaatgcgttccatcagtgtctagcatgctcttcggtagtcaatggtctgctgaagatgatggtgatcaagtgaaagtcacgctcactcatacctattacctgccaaaagatgatgccaaaaccagccaattcctagaacagattgacgcttacaagcggccatctcaagtggctaaagatcagaggcaaagaaaatctcgttctaagtctgctgagaagaagcctgaggaattgtctgtaactcttgtagaggcatatacggatgtgtttgatgacacacaggttgagatgattgatgaggttacgaacggcagcggcgcgaccaactttagcctgctgaaacaggcgggcgatgtggaagaaaacccgggcccgatgaagtacattttgttaatactcgcgtgcattattgcatgcgtttatggagaacgctactgtgccatgcaaaatacaggctcgcagtgcattaatggcacagattcatcatgtagcacctgttttgaacgtggtggtcttatttggcatctggctaactggaacttcagctggtctgtaatattgattgtttttataacagtgttaaaatatggaagaccgcaattcagctggctcgtttatggcattaaaatgctgatcatgtggctattatggcctattgttctagcgcttacgatttttaatgcatactctgagtaccaagtttccagatatgtaatgttcggctttagtgttgcaggtgcagttgtaacgtttgcactatggatgatgtattttgtgagatctattcagctgtatagacggaccaaatcatggtggtcttttaatcctgaaaccaatgcgattctttgtgtcaatgcattgggtagaagctatgtactccctcttgatggcactcctacaggtgttactcttaccctactttcaggaaatctatacgctgaaggttttaaaatggctggtggtcttaccatcgagcatttgcctaaatatgtcatgattgctacgcctagtagaaccatcgtttacacattagttggaaaacaactaaaggcaactactgccactggatgggcttactatgtaaaatctaaagctggtgattactcaacagaagcacgtactgataatttgagtgaacatgaaaaattattacatatggtgggcagcggcgcgaccaactttagcctgctgaaacaggcgggcgatgtggaagaaaacccgggcccgatgattgtgctcgtaacttgcctcttgttgttatgttcataccacacagttttgagtacaacaaataatgaatgcatacaagttaacgtaacacaattggctggcaatgaaaaccttatcagagattttctgtttagtaactttaaagaagaaggaagtgtagttgttggtggttattaccctacagaggtgtggtacaactgctctagaacagctcgaactactgcctttcagtattttaataatatacatgccttttattttgttatggaagccatggaaaatagcactggtaatgcacgtggtaaaccattattatttcatgtgcatggtgagcctgttagtgttattatatcggcttatagggatgatgtgcaacaaaggccccttttaaaacatgggttagtgtgcataactaaaaatcgccatattaactatgaacaattcacctccaaccagtggaattccacatgtacgggtgctgacagaaaaattcctttctctgtcatacccacggacaatggaacaaaaatctatggtcttgagtggaatgatgactttgttacagcttatattagtggtcgttcttatcacttgaacatcaatactaattggtttaacaatgtcacacttttgtattcacgctcaagcactgctacctgggaatacagtgctgcatatgcttaccaaggtgtttctaacttcacttattacaagttaaataacaccaatggtctaaaaacctatgaattatgtgaagattatgaacattgcactggctatgctaccaatgtatttgctccgacatcaggtggttacatacctgatggatttagttttaacaattggttcttgcttacaaatagttccacttttgttagtggcaggtttgtaacaaatcaaccattattgattaattgcttgtggccagtgcccagttttggtgtagcagcacaagaattttgttttgaaggtgcacagtttagccaatgtaatggtgtgtctttaaataacacagtggatgttattagattcaaccttaatttcactgcagatgtacaatctggtatgggtgctacagtattttcactgaatacaacaggtggtgtcattcttgaaatttcatgttatagtgacacagtgagtgagtctagttcttacagttatggtgaaatcccgttcggcataactgacggaccacgatactgttatgtactttacaatggcacagctcttaaatatttaggaacattaccacccagtgtaaaggaaattgctattagtaagtggggccatttttatattaatggttacaatttctttagcacatttcctattggttgtatatcttttaatttaaccactggtgttagtggagctttttggacaattgcttacacatcgtatactgaagcattagtacaagttgaaaacacagctattaaaaatgtgacgtattgtaacagtcacattaataacattaaatgttctcaacttactgctaatttgaataatggattttatcctgttgcttcaagtgaagtaggtttcgttaataagagtgttgtgttattacctagctttttcacatacaccgctgtcaatataaccattgatcttggtatgaagcttagtggttatggtcaacccatagcctcgacactaagtaacatcacactaccaatgcaggataacaatactgatgtgtactgtattcgttctaaccaattctcagtttatgttcattccacttgcaaaagttctttatgggacaatatttttaatcaagactgcacggatgttttagaggctacagctgttataaaaactggtacttgtcctttctcatttgataaattgaacaattacttgacttttaacaagttctgtttgtcgttgagtcctgttggtgctaattgcaagtttgatgttgctgcacgtacaagaaccaatgagcaggttgttagaagtctatatgtaatatatgaagaaggagacaacatagtgggtgtaccgtctgataatagcggtctgcacgatttgtctgtgctacacctagactcctgtacagattacaatatatatggtagaactggtgttggtattattagacgaactaacagtacgctacttagtggcttatattacacatcactatcaggtgatttgttaggctttaaaaatgttagtgatggtgtcatttattctgtgacgccatgtgatgtaagcgcacaagcggctgttattgatggtgccatagttggagctatgacttccattaacagtgaactgttaggtctaacacattggacaacgacacctaatttttattactactctatatataattacacaagtgagaggactcgtgacactgcaattgacagtaacgatgttgattgtgaacctgtcataacctattctaatataggtgtttgtaaaaatggtgctttggtttttattaacgtcacacattctgacggagacgtgcaaccaattagcactggtaatgtcacgatacctacaaattttaccatatctgtgcaagttgaatacatgcaggtttacactacaccagtatcaatagattgtgcaagatacgtttgtaatggtaaccctagatgtaacaaattgttaacacaatatgtgtctgcatgtcaaactattgaacaagcacttgcaatgggtgccagacttgaaaacatggaggttgattccatgttgtttgtctcggaaaatgcccttaaattggcatctgttgaggcgttcaatagtacagaaaatttagattctatttacaaagaatggcctagcataggtggttcttggctaggaggtctaaaagatatactaccgtcccataatagcaaacgtaagtatggttctgctatagaagatttgctttttgataaagttgtaacatctggtttaggtacagttgatgaagattataaacgttgtactggtggttacgacatagcagacttggtgtgtgctcaatattacaatggcatcatggttctaccaggtgtagctaatgctgacaagatgactatgtacacagcatcacttgcaggtggtataacattaggtgcacttggtggtggcgccgtggctataccttttgcagtagcagtacaggctagacttaattatgttgctctacaaactgatgtattgaataaaaaccaacagatcctggctaatgccttcaatcaagctattggtaacattacacaggcttttggtaaggttaatgatgctatacatcaaacatcacaaggtcttgccactgttgctaaagcgttggcaaaagtgcaagatgttgtcaacacacaagggcaagctttaagtcaccttacagtacaattgcaaaataattttcaagccattagtagttctattagtgatatttataacaggcttgacgaactgagtgctgatgcacaagttgataggctgattacaggtagacttacagcacttaatgcatttgtgtctcagactctaaccagacaagcagaggttagggctagtagacaacttgccaaagacaaggttaatgaatgtgttaggtctcagtctcagagattcggattctgtggtaatggtacacatttgttttcactagcaaatgcagcaccaaatggcatgattttctttcatacagtactattaccaacagcttatgaaactgtaacagcttggtcaggtatttgtgcttcagatggcgatcgcactttcggacttgtcgttaaagatgtgcagttgacgttgtttcgtaatctagatgacaagttctatttgacccccagaactatgtatcagcctagagttgcaactagttctgattttgttcaaattgaagggtgtgatgtgttgtttgtcaacgcgactgtaattgatttgcctagtattatacctgactatattgacattaatcaaactgttcaagacatattagaaaattacagaccaaactggactgtacctgaatttacacttgatattttcaacgcaacctatttaaatctgactggtgaaattgatgacttagagtttaggtcagaaaagctacataacactacagtagaacttgccattctcattgataacattaataatacattagtcaatcttgaatggctcaatagaattgaaacttatgtaaaatggccttggtatgtgtggctactgataggtttagtagtagtattttgcataccattactgctattttgctgttttagcacaggttgttgtggatgcataggttgtttaggaagttgttgtcactctatatgtagtagaagacaatttgaaaattatgaaccaattgaaaaagtgcatgtccactaa

SEQ ID NO: 21 - DNA, 6408 bp, synthetic construct
  source 1..6408: mol_type = other DNA
atggccacacagggacaacgcgtcaactggggagatgaaccttccaaaagacgtggtcgttctaactctcgtggtcggaagaataacactatacctctttcattcttcaatcccatccaactcgaaccaggatcaaaattttggagcgtatgtccgagagattttgttcccaagggaataggtaacaaggatcaacaaattggttattggaatagacaagagcgttaccgcattgtcaaaggtcagcgtaaggaacttcctgagaggtggtttttctacttcttaggcacaggacctcaagctgatgctaaatttaaagacaagattgatggagtcttctgggttgcaaaggatggtgccatgaataaaccaacaacacttggcactcgtggtaccaacaatgaatccaaaccactgaaatttgatggtaagataccaccgcaatttcagcttgaagtgaaccgatctaggaacaactcaagaagtggttctcagtctagatctgtctctagaaacaggtctcaatccagaggaagacaacaatccaataatcagaataatgttgaggatacaattgtagctgtgcttcagaaattaggtgttactgaaaagcaaaggtcacgttctaaatctagagatcgtggtgactctaaacctagagacacaacacctaataatgccaacaaacacacctggaagaagactgcaggtaaaggtgatgtgacaaatttctatggtgctagaagtgcttcagctaactttggtgatagtgatctcgttgccaacggtaacgctgccaaatcctaccctcagatagctgaatgcgttccatcagtgtctagcatgctcttcggtagtcaatggtctgctgaagatgatggtgatcaagtgaaagtcacgctcactcatacctattacctgccaaaagatgatgccaaaaccagccaattcctagaacagattgacgcttacaagcggccatctcaagtggctaaagatcagaggcaaagaaaatctcgttctaagtctgctgagaagaagcctgaggaattgtctgtaactcttgtagaggcatatacggatgtgtttgatgacacacaggttgagatgattgatgaggttacgaacggcagcggcgcgaccaactttagcctgctgaaacaggcgggcgatgtggaagaaaacccgggcccgatgattgtgctcgtaacttgcctcttgttgttatgttcataccacacagttttgagtacaacaaataatgaatgcatacaagttaacgtaacacaattggctggcaatgaaaaccttatcagagattttctgtttagtaactttaaagaagaaggaagtgtagttgttggtggttattaccctacagaggtgtggtacaactgctctagaacagctcgaactactgcctttcagtattttaataatatacatgccttttattttgttatggaagccatggaaaatagcactggtaatgcacgtggtaaaccattattatttcatgtgcatggtgagcctgttagtgttattatatcggcttatagggatgatgtgcaacaaaggccccttttaaaacatgggttagtgtgcataactaaaaatcgccatattaactatgaacaattcacctccaaccagtggaattccacatgtacgggtgctgacagaaaaattcctttctctgtcatacccacggacaatggaacaaaaatctatggtcttgagtggaatgatgactttgttacagcttatattagtggtcgttcttatcacttgaacatcaatactaattggtttaacaatgtcacacttttgtattcacgctcaagcactgctacctgggaatacagtgctgcatatgcttaccaaggtgtttctaacttcacttattacaagttaaataacaccaatggtctaaaaacctatgaattatgtgaagattatgaacattgcactggctatgctaccaatgtatttgctccgacatcaggtggttacatacctgatggatttagttttaacaattggttcttgcttacaaatagttccacttttgttagtggcaggtttgtaacaaatcaaccattattgattaattgcttgtggccagtgcccagttttggtgtagcagcacaagaattttgttttgaaggtgcacagtttagccaatgtaatggtgtgtctttaaataacacagtggatgttattagattcaaccttaatttcactgcagatgtacaatctggtatgggtgctacagtattttcactgaatacaacaggtggtgtcattcttgaaatttcatgttatagtgacacagtgagtgagtctagttcttacagttatggtgaaatcccgttcggcataactgacggaccacgatactgttatgtactttacaatggcacagctcttaaatatttaggaacattaccacccagtgtaaaggaaattgctattagtaagtggggccatttttatattaatggttacaatttctttagcacatttcctattggttgtatatcttttaatttaaccactggtgttagtggagctttttggacaattgcttacacatcgtatactgaagcattagtacaagttgaaaacacagctattaaaaatgtgacgtattgtaacagtcacattaataacattaaatgttctcaacttactgctaatttgaataatggattttatcctgttgcttcaagtgaagtaggtttcgttaataagagtgttgtgttattacctagctttttcacatacaccgctgtcaatataaccattgatcttggtatgaagcttagtggttatggtcaacccatagcctcgacactaagtaacatcacactaccaatgcaggataacaatactgatgtgtactgtattcgttctaaccaattctcagtttatgttcattccacttgcaaaagttctttatgggacaatatttttaatcaagactgcacggatgttttagaggctacagctgttataaaaactggtacttgtcctttctcatttgataaattgaacaattacttgacttttaacaagttctgtttgtcgttgagtcctgttggtgctaattgcaagtttgatgttgctgcacgtacaagaaccaatgagcaggttgttagaagtctatatgtaatatatgaagaaggagacaacatagtgggtgtaccgtctgataatagcggtctgcacgatttgtctgtgctacacctagactcctgtacagattacaatatatatggtagaactggtgttggtattattagacgaactaacagtacgctacttagtggcttatattacacatcactatcaggtgatttgttaggctttaaaaatgttagtgatggtgtcatttattctgtgacgccatgtgatgtaagcgcacaagcggctgttattgatggtgccatagttggagctatgacttccattaacagtgaactgttaggtctaacacattggacaacgacacctaatttttattactactctatatataattacacaagtgagaggactcgtgacactgcaattgacagtaacgatgttgattgtgaacctgtcataacctattctaatataggtgtttgtaaaaatggtgctttggtttttattaacgtcacacattctgacggagacgtgcaaccaattagcactggtaatgtcacgatacctacaaattttaccatatctgtgcaagttgaatacatgcaggtttacactacaccagtatcaatagattgtgcaagatacgtttgtaatggtaaccctagatgtaacaaattgttaacacaatatgtgtctgcatgtcaaactattgaacaagcacttgcaatgggtgccagacttgaaaacatggaggttgattccatgttgtttgtctcggaaaatgcccttaaattggcatctgttgaggcgttcaatagtacagaaaatttagattctatttacaaagaatggcctagcataggtggttcttggctaggaggtctaaaagatatactaccgtcccataatagcaaacgtaagtatggttctgctatagaagatttgctttttgataaagttgtaacatctggtttaggtacagttgatgaagattataaacgttgtactggtggttacgacatagcagacttggtgtgtgctcaatattacaatggcatcatggttctaccaggtgtagctaatgctgacaagatgactatgtacacagcatcacttgcaggtggtataacattaggtgcacttggtggtggcgccgtggctataccttttgcagtagcagtacaggctagacttaattatgttgctctacaaactgatgtattgaataaaaaccaacagatcctggctaatgccttcaatcaagctattggtaacattacacaggcttttggtaaggttaatgatgctatacatcaaacatcacaaggtcttgccactgttgctaaagcgttggcaaaagtgcaagatgttgtcaacacacaagggcaagctttaagtcaccttacagtacaattgcaaaataattttcaagccattagtagttctattagtgatatttataacaggcttgacgaactgagtgctgatgcacaagttgataggctgattacaggtagacttacagcacttaatgcatttgtgtctcagactctaaccagacaagcagaggttagggctagtagacaacttgccaaagacaaggttaatgaatgtgttaggtctcagtctcagagattcggattctgtggtaatggtacacatttgttttcactagcaaatgcagcaccaaatggcatgattttctttcatacagtactattaccaacagcttatgaaactgtaacagcttggtcaggtatttgtgcttcagatggcgatcgcactttcggacttgtcgttaaagatgtgcagttgacgttgtttcgtaatctagatgacaagttctatttgacccccagaactatgtatcagcctagagttgcaactagttctgattttgttcaaattgaagggtgtgatgtgttgtttgtcaacgcgactgtaattgatttgcctagtattatacctgactatattgacattaatcaaactgttcaagacatattagaaaattacagaccaaactggactgtacctgaatttacacttgatattttcaacgcaacctatttaaatctgactggtgaaattgatgacttagagtttaggtcagaaaagctacataacactacagtagaacttgccattctcattgataacattaataatacattagtcaatcttgaatggctcaatagaattgaaacttatgtaaaatggccttggtatgtgtggctactgataggtttagtagtagtattttgcataccattactgctattttgctgttttagcacaggttgttgtggatgcataggttgtttaggaagttgttgtcactctatatgtagtagaagacaatttgaaaattatgaaccaattgaaaaagtgcatgtccactaaggcagcggcgcgaccaactttagcctgctgaaacaggcgggcgatgtggaagaaaacccgggcccgatgaagtacattttgttaatactcgcgtgcattattgcatgcgtttatggagaacgctactgtgccatgcaaaatacaggctcgcagtgcattaatggcacagattcatcatgtagcacctgttttgaacgtggtggtcttatttggcatctggctaactggaacttcagctggtctgtaatattgattgtttttataacagtgttaaaatatggaagaccgcaattcagctggctcgtttatggcattaaaatgctgatcatgtggctattatggcctattgttctagcgcttacgatttttaatgcatactctgagtaccaagtttccagatatgtaatgttcggctttagtgttgcaggtgcagttgtaacgtttgcactatggatgatgtattttgtgagatctattcagctgtatagacggaccaaatcatggtggtcttttaatcctgaaaccaatgcgattctttgtgtcaatgcattgggtagaagctatgtactccctcttgatggcactcctacaggtgttactcttaccctactttcaggaaatctatacgctgaaggttttaaaatggctggtggtcttaccatcgagcatttgcctaaatatgtcatgattgctacgcctagtagaaccatcgtttacacattagttggaaaacaactaaaggcaactactgccactggatgggcttactatgtaaaatctaaagctggtgattactcaacagaagcacgtactgataatttgagtgaacatgaaaaattattacatatggtgtaa

SEQ ID NO: 22 - DNA, 4071 bp, synthetic construct
  source 1..4071: mol_type = other DNA
atggccacacagggacaacgcgtcaactggggagatgaaccttccaaaagacgtggtcgttctaactctcgtggtcggaagaataacactatacctctttcattcttcaatcccatccaactcgaaccaggatcaaaattttggagcgtatgtccgagagattttgttcccaagggaataggtaacaaggatcaacaaattggttattggaatagacaagagcgttaccgcattgtcaaaggtcagcgtaaggaacttcctgagaggtggtttttctacttcttaggcacaggacctcaagctgatgctaaatttaaagacaagattgatggagtcttctgggttgcaaaggatggtgccatgaataaaccaacaacacttggcactcgtggtaccaacaatgaatccaaaccactgaaatttgatggtaagataccaccgcaatttcagcttgaagtgaaccgatctaggaacaactcaagaagtggttctcagtctagatctgtctctagaaacaggtctcaatccagaggaagacaacaatccaataatcagaataatgttgaggatacaattgtagctgtgcttcagaaattaggtgttactgaaaagcaaaggtcacgttctaaatctagagatcgtggtgactctaaacctagagacacaacacctaataatgccaacaaacacacctggaagaagactgcaggtaaaggtgatgtgacaaatttctatggtgctagaagtgcttcagctaactttggtgatagtgatctcgttgccaacggtaacgctgccaaatcctaccctcagatagctgaatgcgttccatcagtgtctagcatgctcttcggtagtcaatggtctgctgaagatgatggtgatcaagtgaaagtcacgctcactcatacctattacctgccaaaagatgatgccaaaaccagccaattcctagaacagattgacgcttacaagcggccatctcaagtggctaaagatcagaggcaaagaaaatctcgttctaagtctgctgagaagaagcctgaggaattgtctgtaactcttgtagaggcatatacggatgtgtttgatgacacacaggttgagatgattgatgaggttacgaacggcagcggcgcgaccaactttagcctgctgaaacaggcgggcgatgtggaagaaaacccgggcccgatgaagtacattttgttaatactcgcgtgcattattgcatgcgtttatggagaacgctactgtgccatgcaaaatacaggctcgcagtgcattaatggcacagattcatcatgtagcacctgttttgaacgtggtggtcttatttggcatctggctaactggaacttcagctggtctgtaatattgattgtttttataacagtgttaaaatatggaagaccgcaattcagctggctcgtttatggcattaaaatgctgatcatgtggctattatggcctattgttctagcgcttacgatttttaatgcatactctgagtaccaagtttccagatatgtaatgttcggctttagtgttgcaggtgcagttgtaacgtttgcactatggatgatgtattttgtgagatctattcagctgtatagacggaccaaatcatggtggtcttttaatcctgaaaccaatgcgattctttgtgtcaatgcattgggtagaagctatgtactccctcttgatggcactcctacaggtgttactcttaccctactttcaggaaatctatacgctgaaggttttaaaatggctggtggtcttaccatcgagcatttgcctaaatatgtcatgattgctacgcctagtagaaccatcgtttacacattagttggaaaacaactaaaggcaactactgccactggatgggcttactatgtaaaatctaaagctggtgattactcaacagaagcacgtactgataatttgagtgaacatgaaaaattattacatatggtgggcagcggcgcgaccaactttagcctgctgaaacaggcgggcgatgtggaagaaaacccgggcccgatgtctatatataattacacaagtgagaggactcgtgacactgcaattgacagtaacgatgttgattgtgaacctgtcataacctattctaatataggtgtttgtaaaaatggtgctttggtttttattaacgtcacacattctgacggagacgtgcaaccaattagcactggtaatgtcacgatacctacaaattttaccatatctgtgcaagttgaatacatgcaggtttacactacaccagtatcaatagattgtgcaagatacgtttgtaatggtaaccctagatgtaacaaattgttaacacaatatgtgtctgcatgtcaaactattgaacaagcacttgcaatgggtgccagacttgaaaacatggaggttgattccatgttgtttgtctcggaaaatgcccttaaattggcatctgttgaggcgttcaatagtacagaaaatttagattctatttacaaagaatggcctagcataggtggttcttggctaggaggtctaaaagatatactaccgtcccataatagcaaacgtaagtatggttctgctatagaagatttgctttttgataaagttgtaacatctggtttaggtacagttgatgaagattataaacgttgtactggtggttacgacatagcagacttggtgtgtgctcaatattacaatggcatcatggttctaccaggtgtagctaatgctgacaagatgactatgtacacagcatcacttgcaggtggtataacattaggtgcacttggtggtggcgccgtggctataccttttgcagtagcagtacaggctagacttaattatgttgctctacaaactgatgtattgaataaaaaccaacagatcctggctaatgccttcaatcaagctattggtaacattacacaggcttttggtaaggttaatgatgctatacatcaaacatcacaaggtcttgccactgttgctaaagcgttggcaaaagtgcaagatgttgtcaacacacaagggcaagctttaagtcaccttacagtacaattgcaaaataattttcaagccattagtagttctattagtgatatttataacaggcttgacgaactgagtgctgatgcacaagttgataggctgattacaggtagacttacagcacttaatgcatttgtgtctcagactctaaccagacaagcagaggttagggctagtagacaacttgccaaagacaaggttaatgaatgtgttaggtctcagtctcagagattcggattctgtggtaatggtacacatttgttttcactagcaaatgcagcaccaaatggcatgattttctttcatacagtactattaccaacagcttatgaaactgtaacagcttggtcaggtatttgtgcttcagatggcgatcgcactttcggacttgtcgttaaagatgtgcagttgacgttgtttcgtaatctagatgacaagttctatttgacccccagaactatgtatcagcctagagttgcaactagttctgattttgttcaaattgaagggtgtgatgtgttgtttgtcaacgcgactgtaattgatttgcctagtattatacctgactatattgacattaatcaaactgttcaagacatattagaaaattacagaccaaactggactgtacctgaatttacacttgatattttcaacgcaacctatttaaatctgactggtgaaattgatgacttagagtttaggtcagaaaagctacataacactacagtagaacttgccattctcattgataacattaataatacattagtcaatcttgaatggctcaatagaattgaaacttatgtaaaatggccttggtatgtgtggctactgataggtttagtagtagtattttgcataccattactgctattttgctgttttagcacaggttgttgtggatgcataggttgtttaggaagttgttgtcactctatatgtagtagaagacaatttgaaaattatgaaccaattgaaaaagtgcatgtccactaa

SEQ ID NO: 23 - DNA, 4071 bp, synthetic construct
  source 1..4071: mol_type = other DNA
atggccacacagggacaacgcgtcaactggggagatgaaccttccaaaagacgtggtcgttctaactctcgtggtcggaagaataacactatacctctttcattcttcaatcccatccaactcgaaccaggatcaaaattttggagcgtatgtccgagagattttgttcccaagggaataggtaacaaggatcaacaaattggttattggaatagacaagagcgttaccgcattgtcaaaggtcagcgtaaggaacttcctgagaggtggtttttctacttcttaggcacaggacctcaagctgatgctaaatttaaagacaagattgatggagtcttctgggttgcaaaggatggtgccatgaataaaccaacaacacttggcactcgtggtaccaacaatgaatccaaaccactgaaatttgatggtaagataccaccgcaatttcagcttgaagtgaaccgatctaggaacaactcaagaagtggttctcagtctagatctgtctctagaaacaggtctcaatccagaggaagacaacaatccaataatcagaataatgttgaggatacaattgtagctgtgcttcagaaattaggtgttactgaaaagcaaaggtcacgttctaaatctagagatcgtggtgactctaaacctagagacacaacacctaataatgccaacaaacacacctggaagaagactgcaggtaaaggtgatgtgacaaatttctatggtgctagaagtgcttcagctaactttggtgatagtgatctcgttgccaacggtaacgctgccaaatcctaccctcagatagctgaatgcgttccatcagtgtctagcatgctcttcggtagtcaatggtctgctgaagatgatggtgatcaagtgaaagtcacgctcactcatacctattacctgccaaaagatgatgccaaaaccagccaattcctagaacagattgacgcttacaagcggccatctcaagtggctaaagatcagaggcaaagaaaatctcgttctaagtctgctgagaagaagcctgaggaattgtctgtaactcttgtagaggcatatacggatgtgtttgatgacacacaggttgagatgattgatgaggttacgaacggcagcggcgcgaccaactttagcctgctgaaacaggcgggcgatgtggaagaaaacccgggcccgatgtctatatataattacacaagtgagaggactcgtgacactgcaattgacagtaacgatgttgattgtgaacctgtcataacctattctaatataggtgtttgtaaaaatggtgctttggtttttattaacgtcacacattctgacggagacgtgcaaccaattagcactggtaatgtcacgatacctacaaattttaccatatctgtgcaagttgaatacatgcaggtttacactacaccagtatcaatagattgtgcaagatacgtttgtaatggtaaccctagatgtaacaaattgttaacacaatatgtgtctgcatgtcaaactattgaacaagcacttgcaatgggtgccagacttgaaaacatggaggttgattccatgttgtttgtctcggaaaatgcccttaaattggcatctgttgaggcgttcaatagtacagaaaatttagattctatttacaaagaatggcctagcataggtggttcttggctaggaggtctaaaagatatactaccgtcccataatagcaaacgtaagtatggttctgctatagaagatttgctttttgataaagttgtaacatctggtttaggtacagttgatgaagattataaacgttgtactggtggttacgacatagcagacttggtgtgtgctcaatattacaatggcatcatggttctaccaggtgtagctaatgctgacaagatgactatgtacacagcatcacttgcaggtggtataacattaggtgcacttggtggtggcgccgtggctataccttttgcagtagcagtacaggctagacttaattatgttgctctacaaactgatgtattgaataaaaaccaacagatcctggctaatgccttcaatcaagctattggtaacattacacaggcttttggtaaggttaatgatgctatacatcaaacatcacaaggtcttgccactgttgctaaagcgttggcaaaagtgcaagatgttgtcaacacacaagggcaagctttaagtcaccttacagtacaattgcaaaataattttcaagccattagtagttctattagtgatatttataacaggcttgacgaactgagtgctgatgcacaagttgataggctgattacaggtagacttacagcacttaatgcatttgtgtctcagactctaaccagacaagcagaggttagggctagtagacaacttgccaaagacaaggttaatgaatgtgttaggtctcagtctcagagattcggattctgtggtaatggtacacatttgttttcactagcaaatgcagcaccaaatggcatgattttctttcatacagtactattaccaacagcttatgaaactgtaacagcttggtcaggtatttgtgcttcagatggcgatcgcactttcggacttgtcgttaaagatgtgcagttgacgttgtttcgtaatctagatgacaagttctatttgacccccagaactatgtatcagcctagagttgcaactagttctgattttgttcaaattgaagggtgtgatgtgttgtttgtcaacgcgactgtaattgatttgcctagtattatacctgactatattgacattaatcaaactgttcaagacatattagaaaattacagaccaaactggactgtacctgaatttacacttgatattttcaacgcaacctatttaaatctgactggtgaaattgatgacttagagtttaggtcagaaaagctacataacactacagtagaacttgccattctcattgataacattaataatacattagtcaatcttgaatggctcaatagaattgaaacttatgtaaaatggccttggtatgtgtggctactgataggtttagtagtagtattttgcataccattactgctattttgctgttttagcacaggttgttgtggatgcataggttgtttaggaagttgttgtcactctatatgtagtagaagacaatttgaaaattatgaaccaattgaaaaagtgcatgtccacggcagcggcgcgaccaactttagcctgctgaaacaggcgggcgatgtggaagaaaacccgggcccgatgaagtacattttgttaatactcgcgtgcattattgcatgcgtttatggagaacgctactgtgccatgcaaaatacaggctcgcagtgcattaatggcacagattcatcatgtagcacctgttttgaacgtggtggtcttatttggcatctggctaactggaacttcagctggtctgtaatattgattgtttttataacagtgttaaaatatggaagaccgcaattcagctggctcgtttatggcattaaaatgctgatcatgtggctattatggcctattgttctagcgcttacgatttttaatgcatactctgagtaccaagtttccagatatgtaatgttcggctttagtgttgcaggtgcagttgtaacgtttgcactatggatgatgtattttgtgagatctattcagctgtatagacggaccaaatcatggtggtcttttaatcctgaaaccaatgcgattctttgtgtcaatgcattgggtagaagctatgtactccctcttgatggcactcctacaggtgttactcttaccctactttcaggaaatctatacgctgaaggttttaaaatggctggtggtcttaccatcgagcatttgcctaaatatgtcatgattgctacgcctagtagaaccatcgtttacacattagttggaaaacaactaaaggcaactactgccactggatgggcttactatgtaaaatctaaagctggtgattactcaacagaagcacgtactgataatttgagtgaacatgaaaaattattacatatggtgtaa

SEQ ID NO: 24 - DNA, 1089 bp, synthetic construct
  source 1..1089: mol_type = other DNA
ggatagctaccagcttacacttgcttctgacacaactgtgttcgctatcaaccacacaaacagacaccgccaccatgaagtacattttgttaatactcgcgtgcattattgcatgcgtttatggagaacgctactgtgccatgcaaaatacaggctcgcagtgcattaatggcacagattcatcatgtagcacctgttttgaacgtggtggtcttatttggcatctggctaactggaacttcagctggtctgtaatattgattgtttttataacagtgttaaaatatggaagaccgcaattcagctggctcgtttatggcattaaaatgctgatcatgtggctattatggcctattgttctagcgcttacgatttttaatgcatactctgagtaccaagtttccagatatgtaatgttcggctttagtgttgcaggtgcagttgtaacgtttgcactatggatgatgtattttgtgagatctattcagctgtatagacggaccaaatcatggtggtcttttaatcctgaaaccaatgcgattctttgtgtcaatgcattgggtagaagctatgtactccctcttgatggcactcctacaggtgttactcttaccctactttcaggaaatctatacgctgaaggttttaaaatggctggtggtcttaccatcgagcatttgcctaaatatgtcatgattgctacgcctagtagaaccatcgtttacacattagttggaaaacaactaaaggcaactactgccactggatgggcttactatgtaaaatctaaagctggtgattactcaacagaagcacgtactgataatttgagtgaacatgaaaaattattacatatggtgtaagctccctttcttgctttccagggaaagtcccttggtccccagaccctaatacctggacatgtctaaatcatgaaattctttgaacatctggctcctgcctaataaagaatatttattttcattgcaaaaaaaaaaaaaaaaaaaaaaaaaaaaaaaaaaaaaaaaaaaaaaaaaaaaaaaaaaaaaaaaaaaaaaaaaaaaaaaaaaaaaaaaaaaaaaaaaaaaa

SEQ ID NO: 25 - DNA, 1431 bp, synthetic construct
  source 1..1431: mol_type = other DNA
ggatagctaccagcttacacttgcttctgacacaactgtgttcgctatcaaccacacaaacagacaccgccaccatggccacacagggacaacgcgtcaactggggagatgaaccttccaaaagacgtggtcgttctaactctcgtggtcggaagaataacactatacctctttcattcttcaatcccatccaactcgaaccaggatcaaaattttggagcgtatgtccgagagattttgttcccaagggaataggtaacaaggatcaacaaattggttattggaatagacaagagcgttaccgcattgtcaaaggtcagcgtaaggaacttcctgagaggtggtttttctacttcttaggcacaggacctcaagctgatgctaaatttaaagacaagattgatggagtcttctgggttgcaaaggatggtgccatgaataaaccaacaacacttggcactcgtggtaccaacaatgaatccaaaccactgaaatttgatggtaagataccaccgcaatttcagcttgaagtgaaccgatctaggaacaactcaagaagtggttctcagtctagatctgtctctagaaacaggtctcaatccagaggaagacaacaatccaataatcagaataatgttgaggatacaattgtagctgtgcttcagaaattaggtgttactgaaaagcaaaggtcacgttctaaatctagagatcgtggtgactctaaacctagagacacaacacctaataatgccaacaaacacacctggaagaagactgcaggtaaaggtgatgtgacaaatttctatggtgctagaagtgcttcagctaactttggtgatagtgatctcgttgccaacggtaacgctgccaaatcctaccctcagatagctgaatgcgttccatcagtgtctagcatgctcttcggtagtcaatggtctgctgaagatgatggtgatcaagtgaaagtcacgctcactcatacctattacctgccaaaagatgatgccaaaaccagccaattcctagaacagattgacgcttacaagcggccatctcaagtggctaaagatcagaggcaaagaaaatctcgttctaagtctgctgagaagaagcctgaggaattgtctgtaactcttgtagaggcatatacggatgtgtttgatgacacacaggttgagatgattgatgaggttacgaactaagctccctttcttgctttccagggaaagtcccttggtccccagaccctaatacctggacatgtctaaatcatgaaattctttgaacatctggctcctgcctaataaagaatatttattttcattgcaaaaaaaaaaaaaaaaaaaaaaaaaaaaaaaaaaaaaaaaaaaaaaaaaaaaaaaaaaaaaaaaaaaaaaaaaaaaaaaaaaaaaaaaaaaaaaaaaaaaa

SEQ ID NO: 26 - DNA, 4659 bp, synthetic construct
  source 1..4659: mol_type = other DNA
ggatagctaccagcttacacttgcttctgacacaactgtgttcgctatcaaccacacaaacagacaccgccaccatgattgtgctcgtaacttgcctcttgttgttatgttcataccacacagttttgagtacaacaaataatgaatgcatacaagttaacgtaacacaattggctggcaatgaaaaccttatcagagattttctgtttagtaactttaaagaagaaggaagtgtagttgttggtggttattaccctacagaggtgtggtacaactgctctagaacagctcgaactactgcctttcagtattttaataatatacatgccttttattttgttatggaagccatggaaaatagcactggtaatgcacgtggtaaaccattattatttcatgtgcatggtgagcctgttagtgttattatatcggcttatagggatgatgtgcaacaaaggccccttttaaaacatgggttagtgtgcataactaaaaatcgccatattaactatgaacaattcacctccaaccagtggaattccacatgtacgggtgctgacagaaaaattcctttctctgtcatacccacggacaatggaacaaaaatctatggtcttgagtggaatgatgactttgttacagcttatattagtggtcgttcttatcacttgaacatcaatactaattggtttaacaatgtcacacttttgtattcacgctcaagcactgctacctgggaatacagtgctgcatatgcttaccaaggtgtttctaacttcacttattacaagttaaataacaccaatggtctaaaaacctatgaattatgtgaagattatgaacattgcactggctatgctaccaatgtatttgctccgacatcaggtggttacatacctgatggatttagttttaacaattggttcttgcttacaaatagttccacttttgttagtggcaggtttgtaacaaatcaaccattattgattaattgcttgtggccagtgcccagttttggtgtagcagcacaagaattttgttttgaaggtgcacagtttagccaatgtaatggtgtgtctttaaataacacagtggatgttattagattcaaccttaatttcactgcagatgtacaatctggtatgggtgctacagtattttcactgaatacaacaggtggtgtcattcttgaaatttcatgttatagtgacacagtgagtgagtctagttcttacagttatggtgaaatcccgttcggcataactgacggaccacgatactgttatgtactttacaatggcacagctcttaaatatttaggaacattaccacccagtgtaaaggaaattgctattagtaagtggggccatttttatattaatggttacaatttctttagcacatttcctattggttgtatatcttttaatttaaccactggtgttagtggagctttttggacaattgcttacacatcgtatactgaagcattagtacaagttgaaaacacagctattaaaaatgtgacgtattgtaacagtcacattaataacattaaatgttctcaacttactgctaatttgaataatggattttatcctgttgcttcaagtgaagtaggtttcgttaataagagtgttgtgttattacctagctttttcacatacaccgctgtcaatataaccattgatcttggtatgaagcttagtggttatggtcaacccatagcctcgacactaagtaacatcacactaccaatgcaggataacaatactgatgtgtactgtattcgttctaaccaattctcagtttatgttcattccacttgcaaaagttctttatgggacaatatttttaatcaagactgcacggatgttttagaggctacagctgttataaaaactggtacttgtcctttctcatttgataaattgaacaattacttgacttttaacaagttctgtttgtcgttgagtcctgttggtgctaattgcaagtttgatgttgctgcacgtacaagaaccaatgagcaggttgttagaagtctatatgtaatatatgaagaaggagacaacatagtgggtgtaccgtctgataatagcggtctgcacgatttgtctgtgctacacctagactcctgtacagattacaatatatatggtagaactggtgttggtattattagacgaactaacagtacgctacttagtggcttatattacacatcactatcaggtgatttgttaggctttaaaaatgttagtgatggtgtcatttattctgtgacgccatgtgatgtaagcgcacaagcggctgttattgatggtgccatagttggagctatgacttccattaacagtgaactgttaggtctaacacattggacaacgacacctaatttttattactactctatatataattacacaagtgagaggactcgtgacactgcaattgacagtaacgatgttgattgtgaacctgtcataacctattctaatataggtgtttgtaaaaatggtgctttggtttttattaacgtcacacattctgacggagacgtgcaaccaattagcactggtaatgtcacgatacctacaaattttaccatatctgtgcaagttgaatacatgcaggtttacactacaccagtatcaatagattgtgcaagatacgtttgtaatggtaaccctagatgtaacaaattgttaacacaatatgtgtctgcatgtcaaactattgaacaagcacttgcaatgggtgccagacttgaaaacatggaggttgattccatgttgtttgtctcggaaaatgcccttaaattggcatctgttgaggcgttcaatagtacagaaaatttagattctatttacaaagaatggcctagcataggtggttcttggctaggaggtctaaaagatatactaccgtcccataatagcaaacgtaagtatggttctgctatagaagatttgctttttgataaagttgtaacatctggtttaggtacagttgatgaagattataaacgttgtactggtggttacgacatagcagacttggtgtgtgctcaatattacaatggcatcatggttctaccaggtgtagctaatgctgacaagatgactatgtacacagcatcacttgcaggtggtataacattaggtgcacttggtggtggcgccgtggctataccttttgcagtagcagtacaggctagacttaattatgttgctctacaaactgatgtattgaataaaaaccaacagatcctggctaatgccttcaatcaagctattggtaacattacacaggcttttggtaaggttaatgatgctatacatcaaacatcacaaggtcttgccactgttgctaaagcgttggcaaaagtgcaagatgttgtcaacacacaagggcaagctttaagtcaccttacagtacaattgcaaaataattttcaagccattagtagttctattagtgatatttataacaggcttgacgaactgagtgctgatgcacaagttgataggctgattacaggtagacttacagcacttaatgcatttgtgtctcagactctaaccagacaagcagaggttagggctagtagacaacttgccaaagacaaggttaatgaatgtgttaggtctcagtctcagagattcggattctgtggtaatggtacacatttgttttcactagcaaatgcagcaccaaatggcatgattttctttcatacagtactattaccaacagcttatgaaactgtaacagcttggtcaggtatttgtgcttcagatggcgatcgcactttcggacttgtcgttaaagatgtgcagttgacgttgtttcgtaatctagatgacaagttctatttgacccccagaactatgtatcagcctagagttgcaactagttctgattttgttcaaattgaagggtgtgatgtgttgtttgtcaacgcgactgtaattgatttgcctagtattatacctgactatattgacattaatcaaactgttcaagacatattagaaaattacagaccaaactggactgtacctgaatttacacttgatattttcaacgcaacctatttaaatctgactggtgaaattgatgacttagagtttaggtcagaaaagctacataacactacagtagaacttgccattctcattgataacattaataatacattagtcaatcttgaatggctcaatagaattgaaacttatgtaaaatggccttggtatgtgtggctactgataggtttagtagtagtattttgcataccattactgctattttgctgttttagcacaggttgttgtggatgcataggttgtttaggaagttgttgtcactctatatgtagtagaagacaatttgaaaattatgaaccaattgaaaaagtgcatgtccactaagctccctttcttgctttccagggaaagtcccttggtccccagaccctaatacctggacatgtctaaatcatgaaattctttgaacatctggctcctgcctaataaagaatatttattttcattgcaaaaaaaaaaaaaaaaaaaaaaaaaaaaaaaaaaaaaaaaaaaaaaaaaaaaaaaaaaaaaaaaaaaaaaaaaaaaaaaaaaaaaaaaaaaaaaaaaaaaa

SEQ ID NO: 27 - DNA, 2637 bp, synthetic construct
  source 1..2637: mol_type = other DNA
ggatagctaccagcttacacttgcttctgacacaactgtgttcgctatcaaccacacaaacagacaccgccaccatgattgtgctcgtaacttgcctcttgttgttatgttcataccacacagttttgagtacaacaaataatgaatgcatacaagttaacgtaacacaattggctggcaatgaaaaccttatcagagattttctgtttagtaactttaaagaagaaggaagtgtagttgttggtggttattaccctacagaggtgtggtacaactgctctagaacagctcgaactactgcctttcagtattttaataatatacatgccttttattttgttatggaagccatggaaaatagcactggtaatgcacgtggtaaaccattattatttcatgtgcatggtgagcctgttagtgttattatatcggcttatagggatgatgtgcaacaaaggccccttttaaaacatgggttagtgtgcataactaaaaatcgccatattaactatgaacaattcacctccaaccagtggaattccacatgtacgggtgctgacagaaaaattcctttctctgtcatacccacggacaatggaacaaaaatctatggtcttgagtggaatgatgactttgttacagcttatattagtggtcgttcttatcacttgaacatcaatactaattggtttaacaatgtcacacttttgtattcacgctcaagcactgctacctgggaatacagtgctgcatatgcttaccaaggtgtttctaacttcacttattacaagttaaataacaccaatggtctaaaaacctatgaattatgtgaagattatgaacattgcactggctatgctaccaatgtatttgctccgacatcaggtggttacatacctgatggatttagttttaacaattggttcttgcttacaaatagttccacttttgttagtggcaggtttgtaacaaatcaaccattattgattaattgcttgtggccagtgcccagttttggtgtagcagcacaagaattttgttttgaaggtgcacagtttagccaatgtaatggtgtgtctttaaataacacagtggatgttattagattcaaccttaatttcactgcagatgtacaatctggtatgggtgctacagtattttcactgaatacaacaggtggtgtcattcttgaaatttcatgttatagtgacacagtgagtgagtctagttcttacagttatggtgaaatcccgttcggcataactgacggaccacgatactgttatgtactttacaatggcacagctcttaaatatttaggaacattaccacccagtgtaaaggaaattgctattagtaagtggggccatttttatattaatggttacaatttctttagcacatttcctattggttgtatatcttttaatttaaccactggtgttagtggagctttttggacaattgcttacacatcgtatactgaagcattagtacaagttgaaaacacagctattaaaaatgtgacgtattgtaacagtcacattaataacattaaatgttctcaacttactgctaatttgaataatggattttatcctgttgcttcaagtgaagtaggtttcgttaataagagtgttgtgttattacctagctttttcacatacaccgctgtcaatataaccattgatcttggtatgaagcttagtggttatggtcaacccatagcctcgacactaagtaacatcacactaccaatgcaggataacaatactgatgtgtactgtattcgttctaaccaattctcagtttatgttcattccacttgcaaaagttctttatgggacaatatttttaatcaagactgcacggatgttttagaggctacagctgttataaaaactggtacttgtcctttctcatttgataaattgaacaattacttgacttttaacaagttctgtttgtcgttgagtcctgttggtgctaattgcaagtttgatgttgctgcacgtacaagaaccaatgagcaggttgttagaagtctatatgtaatatatgaagaaggagacaacatagtgggtgtaccgtctgataatagcggtctgcacgatttgtctgtgctacacctagactcctgtacagattacaatatatatggtagaactggtgttggtattattagacgaactaacagtacgctacttagtggcttatattacacatcactatcaggtgatttgttaggctttaaaaatgttagtgatggtgtcatttattctgtgacgccatgtgatgtaagcgcacaagcggctgttattgatggtgccatagttggagctatgacttccattaacagtgaactgttaggtctaacacattggacaacgacacctaatttttattactacgctccctttcttgctttccagggaaagtcccttggtccccagaccctaatacctggacatgtctaaatcatgaaattctttgaacatctggctcctgcctaataaagaatatttattttcattgcaaaaaaaaaaaaaaaaaaaaaaaaaaaaaaaaaaaaaaaaaaaaaaaaaaaaaaaaaaaaaaaaaaaaaaaaaaaaaaaaaaaaaaaaaaaaaaaaaaaaa

SEQ ID NO: 28 - DNA, 2325 bp, synthetic construct
  source 1..2325: mol_type = other DNA
ggatagctaccagcttacacttgcttctgacacaactgtgttcgctatcaaccacacaaacagacaccgccaccatgtctatatataattacacaagtgagaggactcgtgacactgcaattgacagtaacgatgttgattgtgaacctgtcataacctattctaatataggtgtttgtaaaaatggtgctttggtttttattaacgtcacacattctgacggagacgtgcaaccaattagcactggtaatgtcacgatacctacaaattttaccatatctgtgcaagttgaatacatgcaggtttacactacaccagtatcaatagattgtgcaagatacgtttgtaatggtaaccctagatgtaacaaattgttaacacaatatgtgtctgcatgtcaaactattgaacaagcacttgcaatgggtgccagacttgaaaacatggaggttgattccatgttgtttgtctcggaaaatgcccttaaattggcatctgttgaggcgttcaatagtacagaaaatttagattctatttacaaagaatggcctagcataggtggttcttggctaggaggtctaaaagatatactaccgtcccataatagcaaacgtaagtatggttctgctatagaagatttgctttttgataaagttgtaacatctggtttaggtacagttgatgaagattataaacgttgtactggtggttacgacatagcagacttggtgtgtgctcaatattacaatggcatcatggttctaccaggtgtagctaatgctgacaagatgactatgtacacagcatcacttgcaggtggtataacattaggtgcacttggtggtggcgccgtggctataccttttgcagtagcagtacaggctagacttaattatgttgctctacaaactgatgtattgaataaaaaccaacagatcctggctaatgccttcaatcaagctattggtaacattacacaggcttttggtaaggttaatgatgctatacatcaaacatcacaaggtcttgccactgttgctaaagcgttggcaaaagtgcaagatgttgtcaacacacaagggcaagctttaagtcaccttacagtacaattgcaaaataattttcaagccattagtagttctattagtgatatttataacaggcttgacgaactgagtgctgatgcacaagttgataggctgattacaggtagacttacagcacttaatgcatttgtgtctcagactctaaccagacaagcagaggttagggctagtagacaacttgccaaagacaaggttaatgaatgtgttaggtctcagtctcagagattcggattctgtggtaatggtacacatttgttttcactagcaaatgcagcaccaaatggcatgattttctttcatacagtactattaccaacagcttatgaaactgtaacagcttggtcaggtatttgtgcttcagatggcgatcgcactttcggacttgtcgttaaagatgtgcagttgacgttgtttcgtaatctagatgacaagttctatttgacccccagaactatgtatcagcctagagttgcaactagttctgattttgttcaaattgaagggtgtgatgtgttgtttgtcaacgcgactgtaattgatttgcctagtattatacctgactatattgacattaatcaaactgttcaagacatattagaaaattacagaccaaactggactgtacctgaatttacacttgatattttcaacgcaacctatttaaatctgactggtgaaattgatgacttagagtttaggtcagaaaagctacataacactacagtagaacttgccattctcattgataacattaataatacattagtcaatcttgaatggctcaatagaattgaaacttatgtaaaatggccttggtatgtgtggctactgataggtttagtagtagtattttgcataccattactgctattttgctgttttagcacaggttgttgtggatgcataggttgtttaggaagttgttgtcactctatatgtagtagaagacaatttgaaaattatgaaccaattgaaaaagtgcatgtccactaagctccctttcttgctttccagggaaagtcccttggtccccagaccctaatacctggacatgtctaaatcatgaaattctttgaacatctggctcctgcctaataaagaatatttattttcattgcaaaaaaaaaaaaaaaaaaaaaaaaaaaaaaaaaaaaaaaaaaaaaaaaaaaaaaaaaaaaaaaaaaaaaaaaaaaaaaaaaaaaaaaaaaaaaaaaaaaaa

SEQ ID NO: 29 - DNA, 2280 bp, synthetic construct
  source 1..2280: mol_type = other DNA
ggatagctaccagcttacacttgcttctgacacaactgtgttcgctatcaaccacacaaacagacaccgccaccatgaagtacattttgttaatactcgcgtgcattattgcatgcgtttatggagaacgctactgtgccatgcaaaatacaggctcgcagtgcattaatggcacagattcatcatgtagcacctgttttgaacgtggtggtcttatttggcatctggctaactggaacttcagctggtctgtaatattgattgtttttataacagtgttaaaatatggaagaccgcaattcagctggctcgtttatggcattaaaatgctgatcatgtggctattatggcctattgttctagcgcttacgatttttaatgcatactctgagtaccaagtttccagatatgtaatgttcggctttagtgttgcaggtgcagttgtaacgtttgcactatggatgatgtattttgtgagatctattcagctgtatagacggaccaaatcatggtggtcttttaatcctgaaaccaatgcgattctttgtgtcaatgcattgggtagaagctatgtactccctcttgatggcactcctacaggtgttactcttaccctactttcaggaaatctatacgctgaaggttttaaaatggctggtggtcttaccatcgagcatttgcctaaatatgtcatgattgctacgcctagtagaaccatcgtttacacattagttggaaaacaactaaaggcaactactgccactggatgggcttactatgtaaaatctaaagctggtgattactcaacagaagcacgtactgataatttgagtgaacatgaaaaattattacatatggtgggcagcggcgaaggccgcggcagcctgctgacctgcggcgatgtggaagaaaacccgggcccgatggccacacagggacaacgcgtcaactggggagatgaaccttccaaaagacgtggtcgttctaactctcgtggtcggaagaataacactatacctctttcattcttcaatcccatccaactcgaaccaggatcaaaattttggagcgtatgtccgagagattttgttcccaagggaataggtaacaaggatcaacaaattggttattggaatagacaagagcgttaccgcattgtcaaaggtcagcgtaaggaacttcctgagaggtggtttttctacttcttaggcacaggacctcaagctgatgctaaatttaaagacaagattgatggagtcttctgggttgcaaaggatggtgccatgaataaaccaacaacacttggcactcgtggtaccaacaatgaatccaaaccactgaaatttgatggtaagataccaccgcaatttcagcttgaagtgaaccgatctaggaacaactcaagaagtggttctcagtctagatctgtctctagaaacaggtctcaatccagaggaagacaacaatccaataatcagaataatgttgaggatacaattgtagctgtgcttcagaaattaggtgttactgaaaagcaaaggtcacgttctaaatctagagatcgtggtgactctaaacctagagacacaacacctaataatgccaacaaacacacctggaagaagactgcaggtaaaggtgatgtgacaaatttctatggtgctagaagtgcttcagctaactttggtgatagtgatctcgttgccaacggtaacgctgccaaatcctaccctcagatagctgaatgcgttccatcagtgtctagcatgctcttcggtagtcaatggtctgctgaagatgatggtgatcaagtgaaagtcacgctcactcatacctattacctgccaaaagatgatgccaaaaccagccaattcctagaacagattgacgcttacaagcggccatctcaagtggctaaagatcagaggcaaagaaaatctcgttctaagtctgctgagaagaagcctgaggaattgtctgtaactcttgtagaggcatatacggatgtgtttgatgacacacaggttgagatgattgatgaggttacgaactaagctccctttcttgctttccagggaaagtcccttggtccccagaccctaatacctggacatgtctaaatcatgaaattctttgaacatctggctcctgcctaataaagaatatttattttcattgcaaaaaaaaaaaaaaaaaaaaaaaaaaaaaaaaaaaaaaaaaaaaaaaaaaaaaaaaaaaaaaaaaaaaaaaaaaaaaaaaaaaaaaaaaaaaaaaaaaaaa

SEQ ID NO: 30 - DNA, 2280 bp, synthetic construct
  source 1..2280: mol_type = other DNA
ggatagctaccagcttacacttgcttctgacacaactgtgttcgctatcaaccacacaaacagacaccgccaccatggccacacagggacaacgcgtcaactggggagatgaaccttccaaaagacgtggtcgttctaactctcgtggtcggaagaataacactatacctctttcattcttcaatcccatccaactcgaaccaggatcaaaattttggagcgtatgtccgagagattttgttcccaagggaataggtaacaaggatcaacaaattggttattggaatagacaagagcgttaccgcattgtcaaaggtcagcgtaaggaacttcctgagaggtggtttttctacttcttaggcacaggacctcaagctgatgctaaatttaaagacaagattgatggagtcttctgggttgcaaaggatggtgccatgaataaaccaacaacacttggcactcgtggtaccaacaatgaatccaaaccactgaaatttgatggtaagataccaccgcaatttcagcttgaagtgaaccgatctaggaacaactcaagaagtggttctcagtctagatctgtctctagaaacaggtctcaatccagaggaagacaacaatccaataatcagaataatgttgaggatacaattgtagctgtgcttcagaaattaggtgttactgaaaagcaaaggtcacgttctaaatctagagatcgtggtgactctaaacctagagacacaacacctaataatgccaacaaacacacctggaagaagactgcaggtaaaggtgatgtgacaaatttctatggtgctagaagtgcttcagctaactttggtgatagtgatctcgttgccaacggtaacgctgccaaatcctaccctcagatagctgaatgcgttccatcagtgtctagcatgctcttcggtagtcaatggtctgctgaagatgatggtgatcaagtgaaagtcacgctcactcatacctattacctgccaaaagatgatgccaaaaccagccaattcctagaacagattgacgcttacaagcggccatctcaagtggctaaagatcagaggcaaagaaaatctcgttctaagtctgctgagaagaagcctgaggaattgtctgtaactcttgtagaggcatatacggatgtgtttgatgacacacaggttgagatgattgatgaggttacgaacggcagcggcgaaggccgcggcagcctgctgacctgcggcgatgtggaagaaaacccgggcccgatgaagtacattttgttaatactcgcgtgcattattgcatgcgtttatggagaacgctactgtgccatgcaaaatacaggctcgcagtgcattaatggcacagattcatcatgtagcacctgttttgaacgtggtggtcttatttggcatctggctaactggaacttcagctggtctgtaatattgattgtttttataacagtgttaaaatatggaagaccgcaattcagctggctcgtttatggcattaaaatgctgatcatgtggctattatggcctattgttctagcgcttacgatttttaatgcatactctgagtaccaagtttccagatatgtaatgttcggctttagtgttgcaggtgcagttgtaacgtttgcactatggatgatgtattttgtgagatctattcagctgtatagacggaccaaatcatggtggtcttttaatcctgaaaccaatgcgattctttgtgtcaatgcattgggtagaagctatgtactccctcttgatggcactcctacaggtgttactcttaccctactttcaggaaatctatacgctgaaggttttaaaatggctggtggtcttaccatcgagcatttgcctaaatatgtcatgattgctacgcctagtagaaccatcgtttacacattagttggaaaacaactaaaggcaactactgccactggatgggcttactatgtaaaatctaaagctggtgattactcaacagaagcacgtactgataatttgagtgaacatgaaaaattattacatatggtgtaagctccctttcttgctttccagggaaagtcccttggtccccagaccctaatacctggacatgtctaaatcatgaaattctttgaacatctggctcctgcctaataaagaatatttattttcattgcaaaaaaaaaaaaaaaaaaaaaaaaaaaaaaaaaaaaaaaaaaaaaaaaaaaaaaaaaaaaaaaaaaaaaaaaaaaaaaaaaaaaaaaaaaaaaaaaaaaaa

SEQ ID NO: 31 - DNA, 2283 bp, synthetic construct
  source 1..2283: mol_type = other DNA
ggatagctaccagcttacacttgcttctgacacaactgtgttcgctatcaaccacacaaacagacaccgccaccatgaagtacattttgttaatactcgcgtgcattattgcatgcgtttatggagaacgctactgtgccatgcaaaatacaggctcgcagtgcattaatggcacagattcatcatgtagcacctgttttgaacgtggtggtcttatttggcatctggctaactggaacttcagctggtctgtaatattgattgtttttataacagtgttaaaatatggaagaccgcaattcagctggctcgtttatggcattaaaatgctgatcatgtggctattatggcctattgttctagcgcttacgatttttaatgcatactctgagtaccaagtttccagatatgtaatgttcggctttagtgttgcaggtgcagttgtaacgtttgcactatggatgatgtattttgtgagatctattcagctgtatagacggaccaaatcatggtggtcttttaatcctgaaaccaatgcgattctttgtgtcaatgcattgggtagaagctatgtactccctcttgatggcactcctacaggtgttactcttaccctactttcaggaaatctatacgctgaaggttttaaaatggctggtggtcttaccatcgagcatttgcctaaatatgtcatgattgctacgcctagtagaaccatcgtttacacattagttggaaaacaactaaaggcaactactgccactggatgggcttactatgtaaaatctaaagctggtgattactcaacagaagcacgtactgataatttgagtgaacatgaaaaattattacatatggtgggcagcggcgcgaccaactttagcctgctgaaacaggcgggcgatgtggaagaaaacccgggcccgatggccacacagggacaacgcgtcaactggggagatgaaccttccaaaagacgtggtcgttctaactctcgtggtcggaagaataacactatacctctttcattcttcaatcccatccaactcgaaccaggatcaaaattttggagcgtatgtccgagagattttgttcccaagggaataggtaacaaggatcaacaaattggttattggaatagacaagagcgttaccgcattgtcaaaggtcagcgtaaggaacttcctgagaggtggtttttctacttcttaggcacaggacctcaagctgatgctaaatttaaagacaagattgatggagtcttctgggttgcaaaggatggtgccatgaataaaccaacaacacttggcactcgtggtaccaacaatgaatccaaaccactgaaatttgatggtaagataccaccgcaatttcagcttgaagtgaaccgatctaggaacaactcaagaagtggttctcagtctagatctgtctctagaaacaggtctcaatccagaggaagacaacaatccaataatcagaataatgttgaggatacaattgtagctgtgcttcagaaattaggtgttactgaaaagcaaaggtcacgttctaaatctagagatcgtggtgactctaaacctagagacacaacacctaataatgccaacaaacacacctggaagaagactgcaggtaaaggtgatgtgacaaatttctatggtgctagaagtgcttcagctaactttggtgatagtgatctcgttgccaacggtaacgctgccaaatcctaccctcagatagctgaatgcgttccatcagtgtctagcatgctcttcggtagtcaatggtctgctgaagatgatggtgatcaagtgaaagtcacgctcactcatacctattacctgccaaaagatgatgccaaaaccagccaattcctagaacagattgacgcttacaagcggccatctcaagtggctaaagatcagaggcaaagaaaatctcgttctaagtctgctgagaagaagcctgaggaattgtctgtaactcttgtagaggcatatacggatgtgtttgatgacacacaggttgagatgattgatgaggttacgaactaagctccctttcttgctttccagggaaagtcccttggtccccagaccctaatacctggacatgtctaaatcatgaaattctttgaacatctggctcctgcctaataaagaatatttattttcattgcaaaaaaaaaaaaaaaaaaaaaaaaaaaaaaaaaaaaaaaaaaaaaaaaaaaaaaaaaaaaaaaaaaaaaaaaaaaaaaaaaaaaaaaaaaaaaaaaaaaaa

SEQ ID NO: 32 - DNA, 2283 bp, synthetic construct
  source 1..2283: mol_type = other DNA
ggatagctaccagcttacacttgcttctgacacaactgtgttcgctatcaaccacacaaacagacaccgccaccatggccacacagggacaacgcgtcaactggggagatgaaccttccaaaagacgtggtcgttctaactctcgtggtcggaagaataacactatacctctttcattcttcaatcccatccaactcgaaccaggatcaaaattttggagcgtatgtccgagagattttgttcccaagggaataggtaacaaggatcaacaaattggttattggaatagacaagagcgttaccgcattgtcaaaggtcagcgtaaggaacttcctgagaggtggtttttctacttcttaggcacaggacctcaagctgatgctaaatttaaagacaagattgatggagtcttctgggttgcaaaggatggtgccatgaataaaccaacaacacttggcactcgtggtaccaacaatgaatccaaaccactgaaatttgatggtaagataccaccgcaatttcagcttgaagtgaaccgatctaggaacaactcaagaagtggttctcagtctagatctgtctctagaaacaggtctcaatccagaggaagacaacaatccaataatcagaataatgttgaggatacaattgtagctgtgcttcagaaattaggtgttactgaaaagcaaaggtcacgttctaaatctagagatcgtggtgactctaaacctagagacacaacacctaataatgccaacaaacacacctggaagaagactgcaggtaaaggtgatgtgacaaatttctatggtgctagaagtgcttcagctaactttggtgatagtgatctcgttgccaacggtaacgctgccaaatcctaccctcagatagctgaatgcgttccatcagtgtctagcatgctcttcggtagtcaatggtctgctgaagatgatggtgatcaagtgaaagtcacgctcactcatacctattacctgccaaaagatgatgccaaaaccagccaattcctagaacagattgacgcttacaagcggccatctcaagtggctaaagatcagaggcaaagaaaatctcgttctaagtctgctgagaagaagcctgaggaattgtctgtaactcttgtagaggcatatacggatgtgtttgatgacacacaggttgagatgattgatgaggttacgaacggcagcggcgcgaccaactttagcctgctgaaacaggcgggcgatgtggaagaaaacccgggcccgatgaagtacattttgttaatactcgcgtgcattattgcatgcgtttatggagaacgctactgtgccatgcaaaatacaggctcgcagtgcattaatggcacagattcatcatgtagcacctgttttgaacgtggtggtcttatttggcatctggctaactggaacttcagctggtctgtaatattgattgtttttataacagtgttaaaatatggaagaccgcaattcagctggctcgtttatggcattaaaatgctgatcatgtggctattatggcctattgttctagcgcttacgatttttaatgcatactctgagtaccaagtttccagatatgtaatgttcggctttagtgttgcaggtgcagttgtaacgtttgcactatggatgatgtattttgtgagatctattcagctgtatagacggaccaaatcatggtggtcttttaatcctgaaaccaatgcgattctttgtgtcaatgcattgggtagaagctatgtactccctcttgatggcactcctacaggtgttactcttaccctactttcaggaaatctatacgctgaaggttttaaaatggctggtggtcttaccatcgagcatttgcctaaatatgtcatgattgctacgcctagtagaaccatcgtttacacattagttggaaaacaactaaaggcaactactgccactggatgggcttactatgtaaaatctaaagctggtgattactcaacagaagcacgtactgataatttgagtgaacatgaaaaattattacatatggtgtaagctccctttcttgctttccagggaaagtcccttggtccccagaccctaatacctggacatgtctaaatcatgaaattctttgaacatctggctcctgcctaataaagaatatttattttcattgcaaaaaaaaaaaaaaaaaaaaaaaaaaaaaaaaaaaaaaaaaaaaaaaaaaaaaaaaaaaaaaaaaaaaaaaaaaaaaaaaaaaaaaaaaaaaaaaaaaaaa

SEQ ID NO: 33 - DNA, 6699 bp, synthetic construct
  source 1..6699: mol_type = other DNA
ggatagctaccagcttacacttgcttctgacacaactgtgttcgctatcaaccacacaaacagacaccgccaccatggccacacagggacaacgcgtcaactggggagatgaaccttccaaaagacgtggtcgttctaactctcgtggtcggaagaataacactatacctctttcattcttcaatcccatccaactcgaaccaggatcaaaattttggagcgtatgtccgagagattttgttcccaagggaataggtaacaaggatcaacaaattggttattggaatagacaagagcgttaccgcattgtcaaaggtcagcgtaaggaacttcctgagaggtggtttttctacttcttaggcacaggacctcaagctgatgctaaatttaaagacaagattgatggagtcttctgggttgcaaaggatggtgccatgaataaaccaacaacacttggcactcgtggtaccaacaatgaatccaaaccactgaaatttgatggtaagataccaccgcaatttcagcttgaagtgaaccgatctaggaacaactcaagaagtggttctcagtctagatctgtctctagaaacaggtctcaatccagaggaagacaacaatccaataatcagaataatgttgaggatacaattgtagctgtgcttcagaaattaggtgttactgaaaagcaaaggtcacgttctaaatctagagatcgtggtgactctaaacctagagacacaacacctaataatgccaacaaacacacctggaagaagactgcaggtaaaggtgatgtgacaaatttctatggtgctagaagtgcttcagctaactttggtgatagtgatctcgttgccaacggtaacgctgccaaatcctaccctcagatagctgaatgcgttccatcagtgtctagcatgctcttcggtagtcaatggtctgctgaagatgatggtgatcaagtgaaagtcacgctcactcatacctattacctgccaaaagatgatgccaaaaccagccaattcctagaacagattgacgcttacaagcggccatctcaagtggctaaagatcagaggcaaagaaaatctcgttctaagtctgctgagaagaagcctgaggaattgtctgtaactcttgtagaggcatatacggatgtgtttgatgacacacaggttgagatgattgatgaggttacgaacggcagcggcgaaggccgcggcagcctgctgacctgcggcgatgtggaagaaaacccgggcccgatgaagtacattttgttaatactcgcgtgcattattgcatgcgtttatggagaacgctactgtgccatgcaaaatacaggctcgcagtgcattaatggcacagattcatcatgtagcacctgttttgaacgtggtggtcttatttggcatctggctaactggaacttcagctggtctgtaatattgattgtttttataacagtgttaaaatatggaagaccgcaattcagctggctcgtttatggcattaaaatgctgatcatgtggctattatggcctattgttctagcgcttacgatttttaatgcatactctgagtaccaagtttccagatatgtaatgttcggctttagtgttgcaggtgcagttgtaacgtttgcactatggatgatgtattttgtgagatctattcagctgtatagacggaccaaatcatggtggtcttttaatcctgaaaccaatgcgattctttgtgtcaatgcattgggtagaagctatgtactccctcttgatggcactcctacaggtgttactcttaccctactttcaggaaatctatacgctgaaggttttaaaatggctggtggtcttaccatcgagcatttgcctaaatatgtcatgattgctacgcctagtagaaccatcgtttacacattagttggaaaacaactaaaggcaactactgccactggatgggcttactatgtaaaatctaaagctggtgattactcaacagaagcacgtactgataatttgagtgaacatgaaaaattattacatatggtgggcagcggcgaaggccgcggcagcctgctgacctgcggcgatgtggaagaaaacccgggcccgatgattgtgctcgtaacttgcctcttgttgttatgttcataccacacagttttgagtacaacaaataatgaatgcatacaagttaacgtaacacaattggctggcaatgaaaaccttatcagagattttctgtttagtaactttaaagaagaaggaagtgtagttgttggtggttattaccctacagaggtgtggtacaactgctctagaacagctcgaactactgcctttcagtattttaataatatacatgccttttattttgttatggaagccatggaaaatagcactggtaatgcacgtggtaaaccattattatttcatgtgcatggtgagcctgttagtgttattatatcggcttatagggatgatgtgcaacaaaggccccttttaaaacatgggttagtgtgcataactaaaaatcgccatattaactatgaacaattcacctccaaccagtggaattccacatgtacgggtgctgacagaaaaattcctttctctgtcatacccacggacaatggaacaaaaatctatggtcttgagtggaatgatgactttgttacagcttatattagtggtcgttcttatcacttgaacatcaatactaattggtttaacaatgtcacacttttgtattcacgctcaagcactgctacctgggaatacagtgctgcatatgcttaccaaggtgtttctaacttcacttattacaagttaaataacaccaatggtctaaaaacctatgaattatgtgaagattatgaacattgcactggctatgctaccaatgtatttgctccgacatcaggtggttacatacctgatggatttagttttaacaattggttcttgcttacaaatagttccacttttgttagtggcaggtttgtaacaaatcaaccattattgattaattgcttgtggccagtgcccagttttggtgtagcagcacaagaattttgttttgaaggtgcacagtttagccaatgtaatggtgtgtctttaaataacacagtggatgttattagattcaaccttaatttcactgcagatgtacaatctggtatgggtgctacagtattttcactgaatacaacaggtggtgtcattcttgaaatttcatgttatagtgacacagtgagtgagtctagttcttacagttatggtgaaatcccgttcggcataactgacggaccacgatactgttatgtactttacaatggcacagctcttaaatatttaggaacattaccacccagtgtaaaggaaattgctattagtaagtggggccatttttatattaatggttacaatttctttagcacatttcctattggttgtatatcttttaatttaaccactggtgttagtggagctttttggacaattgcttacacatcgtatactgaagcattagtacaagttgaaaacacagctattaaaaatgtgacgtattgtaacagtcacattaataacattaaatgttctcaacttactgctaatttgaataatggattttatcctgttgcttcaagtgaagtaggtttcgttaataagagtgttgtgttattacctagctttttcacatacaccgctgtcaatataaccattgatcttggtatgaagcttagtggttatggtcaacccatagcctcgacactaagtaacatcacactaccaatgcaggataacaatactgatgtgtactgtattcgttctaaccaattctcagtttatgttcattccacttgcaaaagttctttatgggacaatatttttaatcaagactgcacggatgttttagaggctacagctgttataaaaactggtacttgtcctttctcatttgataaattgaacaattacttgacttttaacaagttctgtttgtcgttgagtcctgttggtgctaattgcaagtttgatgttgctgcacgtacaagaaccaatgagcaggttgttagaagtctatatgtaatatatgaagaaggagacaacatagtgggtgtaccgtctgataatagcggtctgcacgatttgtctgtgctacacctagactcctgtacagattacaatatatatggtagaactggtgttggtattattagacgaactaacagtacgctacttagtggcttatattacacatcactatcaggtgatttgttaggctttaaaaatgttagtgatggtgtcatttattctgtgacgccatgtgatgtaagcgcacaagcggctgttattgatggtgccatagttggagctatgacttccattaacagtgaactgttaggtctaacacattggacaacgacacctaatttttattactactctatatataattacacaagtgagaggactcgtgacactgcaattgacagtaacgatgttgattgtgaacctgtcataacctattctaatataggtgtttgtaaaaatggtgctttggtttttattaacgtcacacattctgacggagacgtgcaaccaattagcactggtaatgtcacgatacctacaaattttaccatatctgtgcaagttgaatacatgcaggtttacactacaccagtatcaatagattgtgcaagatacgtttgtaatggtaaccctagatgtaacaaattgttaacacaatatgtgtctgcatgtcaaactattgaacaagcacttgcaatgggtgccagacttgaaaacatggaggttgattccatgttgtttgtctcggaaaatgcccttaaattggcatctgttgaggcgttcaatagtacagaaaatttagattctatttacaaagaatggcctagcataggtggttcttggctaggaggtctaaaagatatactaccgtcccataatagcaaacgtaagtatggttctgctatagaagatttgctttttgataaagttgtaacatctggtttaggtacagttgatgaagattataaacgttgtactggtggttacgacatagcagacttggtgtgtgctcaatattacaatggcatcatggttctaccaggtgtagctaatgctgacaagatgactatgtacacagcatcacttgcaggtggtataacattaggtgcacttggtggtggcgccgtggctataccttttgcagtagcagtacaggctagacttaattatgttgctctacaaactgatgtattgaataaaaaccaacagatcctggctaatgccttcaatcaagctattggtaacattacacaggcttttggtaaggttaatgatgctatacatcaaacatcacaaggtcttgccactgttgctaaagcgttggcaaaagtgcaagatgttgtcaacacacaagggcaagctttaagtcaccttacagtacaattgcaaaataattttcaagccattagtagttctattagtgatatttataacaggcttgacgaactgagtgctgatgcacaagttgataggctgattacaggtagacttacagcacttaatgcatttgtgtctcagactctaaccagacaagcagaggttagggctagtagacaacttgccaaagacaaggttaatgaatgtgttaggtctcagtctcagagattcggattctgtggtaatggtacacatttgttttcactagcaaatgcagcaccaaatggcatgattttctttcatacagtactattaccaacagcttatgaaactgtaacagcttggtcaggtatttgtgcttcagatggcgatcgcactttcggacttgtcgttaaagatgtgcagttgacgttgtttcgtaatctagatgacaagttctatttgacccccagaactatgtatcagcctagagttgcaactagttctgattttgttcaaattgaagggtgtgatgtgttgtttgtcaacgcgactgtaattgatttgcctagtattatacctgactatattgacattaatcaaactgttcaagacatattagaaaattacagaccaaactggactgtacctgaatttacacttgatattttcaacgcaacctatttaaatctgactggtgaaattgatgacttagagtttaggtcagaaaagctacataacactacagtagaacttgccattctcattgataacattaataatacattagtcaatcttgaatggctcaatagaattgaaacttatgtaaaatggccttggtatgtgtggctactgataggtttagtagtagtattttgcataccattactgctattttgctgttttagcacaggttgttgtggatgcataggttgtttaggaagttgttgtcactctatatgtagtagaagacaatttgaaaattatgaaccaattgaaaaagtgcatgtccactaagctccctttcttgctttccagggaaagtcccttggtccccagaccctaatacctggacatgtctaaatcatgaaattctttgaacatctggctcctgcctaataaagaatatttattttcattgcaaaaaaaaaaaaaaaaaaaaaaaaaaaaaaaaaaaaaaaaaaaaaaaaaaaaaaaaaaaaaaaaaaaaaaaaaaaaaaaaaaaaaaaaaaaaaaaaaaaaa

SEQ ID NO: 34 - DNA, 6702 bp, synthetic construct
  source 1..6702: mol_type = other DNA
ggatagctaccagcttacacttgcttctgacacaactgtgttcgctatcaaccacacaaacagacaccgccaccatggccacacagggacaacgcgtcaactggggagatgaaccttccaaaagacgtggtcgttctaactctcgtggtcggaagaataacactatacctctttcattcttcaatcccatccaactcgaaccaggatcaaaattttggagcgtatgtccgagagattttgttcccaagggaataggtaacaaggatcaacaaattggttattggaatagacaagagcgttaccgcattgtcaaaggtcagcgtaaggaacttcctgagaggtggtttttctacttcttaggcacaggacctcaagctgatgctaaatttaaagacaagattgatggagtcttctgggttgcaaaggatggtgccatgaataaaccaacaacacttggcactcgtggtaccaacaatgaatccaaaccactgaaatttgatggtaagataccaccgcaatttcagcttgaagtgaaccgatctaggaacaactcaagaagtggttctcagtctagatctgtctctagaaacaggtctcaatccagaggaagacaacaatccaataatcagaataatgttgaggatacaattgtagctgtgcttcagaaattaggtgttactgaaaagcaaaggtcacgttctaaatctagagatcgtggtgactctaaacctagagacacaacacctaataatgccaacaaacacacctggaagaagactgcaggtaaaggtgatgtgacaaatttctatggtgctagaagtgcttcagctaactttggtgatagtgatctcgttgccaacggtaacgctgccaaatcctaccctcagatagctgaatgcgttccatcagtgtctagcatgctcttcggtagtcaatggtctgctgaagatgatggtgatcaagtgaaagtcacgctcactcatacctattacctgccaaaagatgatgccaaaaccagccaattcctagaacagattgacgcttacaagcggccatctcaagtggctaaagatcagaggcaaagaaaatctcgttctaagtctgctgagaagaagcctgaggaattgtctgtaactcttgtagaggcatatacggatgtgtttgatgacacacaggttgagatgattgatgaggttacgaacggcagcggcgaaggccgcggcagcctgctgacctgcggcgatgtggaagaaaacccgggcccgatgattgtgctcgtaacttgcctcttgttgttatgttcataccacacagttttgagtacaacaaataatgaatgcatacaagttaacgtaacacaattggctggcaatgaaaaccttatcagagattttctgtttagtaactttaaagaagaaggaagtgtagttgttggtggttattaccctacagaggtgtggtacaactgctctagaacagctcgaactactgcctttcagtattttaataatatacatgccttttattttgttatggaagccatggaaaatagcactggtaatgcacgtggtaaaccattattatttcatgtgcatggtgagcctgttagtgttattatatcggcttatagggatgatgtgcaacaaaggccccttttaaaacatgggttagtgtgcataactaaaaatcgccatattaactatgaacaattcacctccaaccagtggaattccacatgtacgggtgctgacagaaaaattcctttctctgtcatacccacggacaatggaacaaaaatctatggtcttgagtggaatgatgactttgttacagcttatattagtggtcgttcttatcacttgaacatcaatactaattggtttaacaatgtcacacttttgtattcacgctcaagcactgctacctgggaatacagtgctgcatatgcttaccaaggtgtttctaacttcacttattacaagttaaataacaccaatggtctaaaaacctatgaattatgtgaagattatgaacattgcactggctatgctaccaatgtatttgctccgacatcaggtggttacatacctgatggatttagttttaacaattggttcttgcttacaaatagttccacttttgttagtggcaggtttgtaacaaatcaaccattattgattaattgcttgtggccagtgcccagttttggtgtagcagcacaagaattttgttttgaaggtgcacagtttagccaatgtaatggtgtgtctttaaataacacagtggatgttattagattcaaccttaatttcactgcagatgtacaatctggtatgggtgctacagtattttcactgaatacaacaggtggtgtcattcttgaaatttcatgttatagtgacacagtgagtgagtctagttcttacagttatggtgaaatcccgttcggcataactgacggaccacgatactgttatgtactttacaatggcacagctcttaaatatttaggaacattaccacccagtgtaaaggaaattgctattagtaagtggggccatttttatattaatggttacaatttctttagcacatttcctattggttgtatatcttttaatttaaccactggtgttagtggagctttttggacaattgcttacacatcgtatactgaagcattagtacaagttgaaaacacagctattaaaaatgtgacgtattgtaacagtcacattaataacattaaatgttctcaacttactgctaatttgaataatggattttatcctgttgcttcaagtgaagtaggtttcgttaataagagtgttgtgttattacctagctttttcacatacaccgctgtcaatataaccattgatcttggtatgaagcttagtggttatggtcaacccatagcctcgacactaagtaacatcacactaccaatgcaggataacaatactgatgtgtactgtattcgttctaaccaattctcagtttatgttcattccacttgcaaaagttctttatgggacaatatttttaatcaagactgcacggatgttttagaggctacagctgttataaaaactggtacttgtcctttctcatttgataaattgaacaattacttgacttttaacaagttctgtttgtcgttgagtcctgttggtgctaattgcaagtttgatgttgctgcacgtacaagaaccaatgagcaggttgttagaagtctatatgtaatatatgaagaaggagacaacatagtgggtgtaccgtctgataatagcggtctgcacgatttgtctgtgctacacctagactcctgtacagattacaatatatatggtagaactggtgttggtattattagacgaactaacagtacgctacttagtggcttatattacacatcactatcaggtgatttgttaggctttaaaaatgttagtgatggtgtcatttattctgtgacgccatgtgatgtaagcgcacaagcggctgttattgatggtgccatagttggagctatgacttccattaacagtgaactgttaggtctaacacattggacaacgacacctaatttttattactactctatatataattacacaagtgagaggactcgtgacactgcaattgacagtaacgatgttgattgtgaacctgtcataacctattctaatataggtgtttgtaaaaatggtgctttggtttttattaacgtcacacattctgacggagacgtgcaaccaattagcactggtaatgtcacgatacctacaaattttaccatatctgtgcaagttgaatacatgcaggtttacactacaccagtatcaatagattgtgcaagatacgtttgtaatggtaaccctagatgtaacaaattgttaacacaatatgtgtctgcatgtcaaactattgaacaagcacttgcaatgggtgccagacttgaaaacatggaggttgattccatgttgtttgtctcggaaaatgcccttaaattggcatctgttgaggcgttcaatagtacagaaaatttagattctatttacaaagaatggcctagcataggtggttcttggctaggaggtctaaaagatatactaccgtcccataatagcaaacgtaagtatggttctgctatagaagatttgctttttgataaagttgtaacatctggtttaggtacagttgatgaagattataaacgttgtactggtggttacgacatagcagacttggtgtgtgctcaatattacaatggcatcatggttctaccaggtgtagctaatgctgacaagatgactatgtacacagcatcacttgcaggtggtataacattaggtgcacttggtggtggcgccgtggctataccttttgcagtagcagtacaggctagacttaattatgttgctctacaaactgatgtattgaataaaaaccaacagatcctggctaatgccttcaatcaagctattggtaacattacacaggcttttggtaaggttaatgatgctatacatcaaacatcacaaggtcttgccactgttgctaaagcgttggcaaaagtgcaagatgttgtcaacacacaagggcaagctttaagtcaccttacagtacaattgcaaaataattttcaagccattagtagttctattagtgatatttataacaggcttgacgaactgagtgctgatgcacaagttgataggctgattacaggtagacttacagcacttaatgcatttgtgtctcagactctaaccagacaagcagaggttagggctagtagacaacttgccaaagacaaggttaatgaatgtgttaggtctcagtctcagagattcggattctgtggtaatggtacacatttgttttcactagcaaatgcagcaccaaatggcatgattttctttcatacagtactattaccaacagcttatgaaactgtaacagcttggtcaggtatttgtgcttcagatggcgatcgcactttcggacttgtcgttaaagatgtgcagttgacgttgtttcgtaatctagatgacaagttctatttgacccccagaactatgtatcagcctagagttgcaactagttctgattttgttcaaattgaagggtgtgatgtgttgtttgtcaacgcgactgtaattgatttgcctagtattatacctgactatattgacattaatcaaactgttcaagacatattagaaaattacagaccaaactggactgtacctgaatttacacttgatattttcaacgcaacctatttaaatctgactggtgaaattgatgacttagagtttaggtcagaaaagctacataacactacagtagaacttgccattctcattgataacattaataatacattagtcaatcttgaatggctcaatagaattgaaacttatgtaaaatggccttggtatgtgtggctactgataggtttagtagtagtattttgcataccattactgctattttgctgttttagcacaggttgttgtggatgcataggttgtttaggaagttgttgtcactctatatgtagtagaagacaatttgaaaattatgaaccaattgaaaaagtgcatgtccactaaggcagcggcgaaggccgcggcagcctgctgacctgcggcgatgtggaagaaaacccgggcccgatgaagtacattttgttaatactcgcgtgcattattgcatgcgtttatggagaacgctactgtgccatgcaaaatacaggctcgcagtgcattaatggcacagattcatcatgtagcacctgttttgaacgtggtggtcttatttggcatctggctaactggaacttcagctggtctgtaatattgattgtttttataacagtgttaaaatatggaagaccgcaattcagctggctcgtttatggcattaaaatgctgatcatgtggctattatggcctattgttctagcgcttacgatttttaatgcatactctgagtaccaagtttccagatatgtaatgttcggctttagtgttgcaggtgcagttgtaacgtttgcactatggatgatgtattttgtgagatctattcagctgtatagacggaccaaatcatggtggtcttttaatcctgaaaccaatgcgattctttgtgtcaatgcattgggtagaagctatgtactccctcttgatggcactcctacaggtgttactcttaccctactttcaggaaatctatacgctgaaggttttaaaatggctggtggtcttaccatcgagcatttgcctaaatatgtcatgattgctacgcctagtagaaccatcgtttacacattagttggaaaacaactaaaggcaactactgccactggatgggcttactatgtaaaatctaaagctggtgattactcaacagaagcacgtactgataatttgagtgaacatgaaaaattattacatatggtgtaagctccctttcttgctttccagggaaagtcccttggtccccagaccctaatacctggacatgtctaaatcatgaaattctttgaacatctggctcctgcctaataaagaatatttattttcattgcaaaaaaaaaaaaaaaaaaaaaaaaaaaaaaaaaaaaaaaaaaaaaaaaaaaaaaaaaaaaaaaaaaaaaaaaaaaaaaaaaaaaaaaaaaaaaaaaaaaaa

SEQ ID NO: 35 - DNA, 4365 bp, synthetic construct
  source 1..4365: mol_type = other DNA
ggatagctaccagcttacacttgcttctgacacaactgtgttcgctatcaaccacacaaacagacaccgccaccatggccacacagggacaacgcgtcaactggggagatgaaccttccaaaagacgtggtcgttctaactctcgtggtcggaagaataacactatacctctttcattcttcaatcccatccaactcgaaccaggatcaaaattttggagcgtatgtccgagagattttgttcccaagggaataggtaacaaggatcaacaaattggttattggaatagacaagagcgttaccgcattgtcaaaggtcagcgtaaggaacttcctgagaggtggtttttctacttcttaggcacaggacctcaagctgatgctaaatttaaagacaagattgatggagtcttctgggttgcaaaggatggtgccatgaataaaccaacaacacttggcactcgtggtaccaacaatgaatccaaaccactgaaatttgatggtaagataccaccgcaatttcagcttgaagtgaaccgatctaggaacaactcaagaagtggttctcagtctagatctgtctctagaaacaggtctcaatccagaggaagacaacaatccaataatcagaataatgttgaggatacaattgtagctgtgcttcagaaattaggtgttactgaaaagcaaaggtcacgttctaaatctagagatcgtggtgactctaaacctagagacacaacacctaataatgccaacaaacacacctggaagaagactgcaggtaaaggtgatgtgacaaatttctatggtgctagaagtgcttcagctaactttggtgatagtgatctcgttgccaacggtaacgctgccaaatcctaccctcagatagctgaatgcgttccatcagtgtctagcatgctcttcggtagtcaatggtctgctgaagatgatggtgatcaagtgaaagtcacgctcactcatacctattacctgccaaaagatgatgccaaaaccagccaattcctagaacagattgacgcttacaagcggccatctcaagtggctaaagatcagaggcaaagaaaatctcgttctaagtctgctgagaagaagcctgaggaattgtctgtaactcttgtagaggcatatacggatgtgtttgatgacacacaggttgagatgattgatgaggttacgaacggcagcggcgaaggccgcggcagcctgctgacctgcggcgatgtggaagaaaacccgggcccgatgaagtacattttgttaatactcgcgtgcattattgcatgcgtttatggagaacgctactgtgccatgcaaaatacaggctcgcagtgcattaatggcacagattcatcatgtagcacctgttttgaacgtggtggtcttatttggcatctggctaactggaacttcagctggtctgtaatattgattgtttttataacagtgttaaaatatggaagaccgcaattcagctggctcgtttatggcattaaaatgctgatcatgtggctattatggcctattgttctagcgcttacgatttttaatgcatactctgagtaccaagtttccagatatgtaatgttcggctttagtgttgcaggtgcagttgtaacgtttgcactatggatgatgtattttgtgagatctattcagctgtatagacggaccaaatcatggtggtcttttaatcctgaaaccaatgcgattctttgtgtcaatgcattgggtagaagctatgtactccctcttgatggcactcctacaggtgttactcttaccctactttcaggaaatctatacgctgaaggttttaaaatggctggtggtcttaccatcgagcatttgcctaaatatgtcatgattgctacgcctagtagaaccatcgtttacacattagttggaaaacaactaaaggcaactactgccactggatgggcttactatgtaaaatctaaagctggtgattactcaacagaagcacgtactgataatttgagtgaacatgaaaaattattacatatggtgggcagcggcgaaggccgcggcagcctgctgacctgcggcgatgtggaagaaaacccgggcccgatgtctatatataattacacaagtgagaggactcgtgacactgcaattgacagtaacgatgttgattgtgaacctgtcataacctattctaatataggtgtttgtaaaaatggtgctttggtttttattaacgtcacacattctgacggagacgtgcaaccaattagcactggtaatgtcacgatacctacaaattttaccatatctgtgcaagttgaatacatgcaggtttacactacaccagtatcaatagattgtgcaagatacgtttgtaatggtaaccctagatgtaacaaattgttaacacaatatgtgtctgcatgtcaaactattgaacaagcacttgcaatgggtgccagacttgaaaacatggaggttgattccatgttgtttgtctcggaaaatgcccttaaattggcatctgttgaggcgttcaatagtacagaaaatttagattctatttacaaagaatggcctagcataggtggttcttggctaggaggtctaaaagatatactaccgtcccataatagcaaacgtaagtatggttctgctatagaagatttgctttttgataaagttgtaacatctggtttaggtacagttgatgaagattataaacgttgtactggtggttacgacatagcagacttggtgtgtgctcaatattacaatggcatcatggttctaccaggtgtagctaatgctgacaagatgactatgtacacagcatcacttgcaggtggtataacattaggtgcacttggtggtggcgccgtggctataccttttgcagtagcagtacaggctagacttaattatgttgctctacaaactgatgtattgaataaaaaccaacagatcctggctaatgccttcaatcaagctattggtaacattacacaggcttttggtaaggttaatgatgctatacatcaaacatcacaaggtcttgccactgttgctaaagcgttggcaaaagtgcaagatgttgtcaacacacaagggcaagctttaagtcaccttacagtacaattgcaaaataattttcaagccattagtagttctattagtgatatttataacaggcttgacgaactgagtgctgatgcacaagttgataggctgattacaggtagacttacagcacttaatgcatttgtgtctcagactctaaccagacaagcagaggttagggctagtagacaacttgccaaagacaaggttaatgaatgtgttaggtctcagtctcagagattcggattctgtggtaatggtacacatttgttttcactagcaaatgcagcaccaaatggcatgattttctttcatacagtactattaccaacagcttatgaaactgtaacagcttggtcaggtatttgtgcttcagatggcgatcgcactttcggacttgtcgttaaagatgtgcagttgacgttgtttcgtaatctagatgacaagttctatttgacccccagaactatgtatcagcctagagttgcaactagttctgattttgttcaaattgaagggtgtgatgtgttgtttgtcaacgcgactgtaattgatttgcctagtattatacctgactatattgacattaatcaaactgttcaagacatattagaaaattacagaccaaactggactgtacctgaatttacacttgatattttcaacgcaacctatttaaatctgactggtgaaattgatgacttagagtttaggtcagaaaagctacataacactacagtagaacttgccattctcattgataacattaataatacattagtcaatcttgaatggctcaatagaattgaaacttatgtaaaatggccttggtatgtgtggctactgataggtttagtagtagtattttgcataccattactgctattttgctgttttagcacaggttgttgtggatgcataggttgtttaggaagttgttgtcactctatatgtagtagaagacaatttgaaaattatgaaccaattgaaaaagtgcatgtccactaagctccctttcttgctttccagggaaagtcccttggtccccagaccctaatacctggacatgtctaaatcatgaaattctttgaacatctggctcctgcctaataaagaatatttattttcattgcaaaaaaaaaaaaaaaaaaaaaaaaaaaaaaaaaaaaaaaaaaaaaaaaaaaaaaaaaaaaaaaaaaaaaaaaaaaaaaaaaaaaaaaaaaaaaaaaaaaaa

SEQ ID NO: 36 - DNA, 4365 bp, synthetic construct
  source 1..4365: mol_type = other DNA
ggatagctaccagcttacacttgcttctgacacaactgtgttcgctatcaaccacacaaacagacaccgccaccatggccacacagggacaacgcgtcaactggggagatgaaccttccaaaagacgtggtcgttctaactctcgtggtcggaagaataacactatacctctttcattcttcaatcccatccaactcgaaccaggatcaaaattttggagcgtatgtccgagagattttgttcccaagggaataggtaacaaggatcaacaaattggttattggaatagacaagagcgttaccgcattgtcaaaggtcagcgtaaggaacttcctgagaggtggtttttctacttcttaggcacaggacctcaagctgatgctaaatttaaagacaagattgatggagtcttctgggttgcaaaggatggtgccatgaataaaccaacaacacttggcactcgtggtaccaacaatgaatccaaaccactgaaatttgatggtaagataccaccgcaatttcagcttgaagtgaaccgatctaggaacaactcaagaagtggttctcagtctagatctgtctctagaaacaggtctcaatccagaggaagacaacaatccaataatcagaataatgttgaggatacaattgtagctgtgcttcagaaattaggtgttactgaaaagcaaaggtcacgttctaaatctagagatcgtggtgactctaaacctagagacacaacacctaataatgccaacaaacacacctggaagaagactgcaggtaaaggtgatgtgacaaatttctatggtgctagaagtgcttcagctaactttggtgatagtgatctcgttgccaacggtaacgctgccaaatcctaccctcagatagctgaatgcgttccatcagtgtctagcatgctcttcggtagtcaatggtctgctgaagatgatggtgatcaagtgaaagtcacgctcactcatacctattacctgccaaaagatgatgccaaaaccagccaattcctagaacagattgacgcttacaagcggccatctcaagtggctaaagatcagaggcaaagaaaatctcgttctaagtctgctgagaagaagcctgaggaattgtctgtaactcttgtagaggcatatacggatgtgtttgatgacacacaggttgagatgattgatgaggttacgaacggcagcggcgaaggccgcggcagcctgctgacctgcggcgatgtggaagaaaacccgggcccgatgtctatatataattacacaagtgagaggactcgtgacactgcaattgacagtaacgatgttgattgtgaacctgtcataacctattctaatataggtgtttgtaaaaatggtgctttggtttttattaacgtcacacattctgacggagacgtgcaaccaattagcactggtaatgtcacgatacctacaaattttaccatatctgtgcaagttgaatacatgcaggtttacactacaccagtatcaatagattgtgcaagatacgtttgtaatggtaaccctagatgtaacaaattgttaacacaatatgtgtctgcatgtcaaactattgaacaagcacttgcaatgggtgccagacttgaaaacatggaggttgattccatgttgtttgtctcggaaaatgcccttaaattggcatctgttgaggcgttcaatagtacagaaaatttagattctatttacaaagaatggcctagcataggtggttcttggctaggaggtctaaaagatatactaccgtcccataatagcaaacgtaagtatggttctgctatagaagatttgctttttgataaagttgtaacatctggtttaggtacagttgatgaagattataaacgttgtactggtggttacgacatagcagacttggtgtgtgctcaatattacaatggcatcatggttctaccaggtgtagctaatgctgacaagatgactatgtacacagcatcacttgcaggtggtataacattaggtgcacttggtggtggcgccgtggctataccttttgcagtagcagtacaggctagacttaattatgttgctctacaaactgatgtattgaataaaaaccaacagatcctggctaatgccttcaatcaagctattggtaacattacacaggcttttggtaaggttaatgatgctatacatcaaacatcacaaggtcttgccactgttgctaaagcgttggcaaaagtgcaagatgttgtcaacacacaagggcaagctttaagtcaccttacagtacaattgcaaaataattttcaagccattagtagttctattagtgatatttataacaggcttgacgaactgagtgctgatgcacaagttgataggctgattacaggtagacttacagcacttaatgcatttgtgtctcagactctaaccagacaagcagaggttagggctagtagacaacttgccaaagacaaggttaatgaatgtgttaggtctcagtctcagagattcggattctgtggtaatggtacacatttgttttcactagcaaatgcagcaccaaatggcatgattttctttcatacagtactattaccaacagcttatgaaactgtaacagcttggtcaggtatttgtgcttcagatggcgatcgcactttcggacttgtcgttaaagatgtgcagttgacgttgtttcgtaatctagatgacaagttctatttgacccccagaactatgtatcagcctagagttgcaactagttctgattttgttcaaattgaagggtgtgatgtgttgtttgtcaacgcgactgtaattgatttgcctagtattatacctgactatattgacattaatcaaactgttcaagacatattagaaaattacagaccaaactggactgtacctgaatttacacttgatattttcaacgcaacctatttaaatctgactggtgaaattgatgacttagagtttaggtcagaaaagctacataacactacagtagaacttgccattctcattgataacattaataatacattagtcaatcttgaatggctcaatagaattgaaacttatgtaaaatggccttggtatgtgtggctactgataggtttagtagtagtattttgcataccattactgctattttgctgttttagcacaggttgttgtggatgcataggttgtttaggaagttgttgtcactctatatgtagtagaagacaatttgaaaattatgaaccaattgaaaaagtgcatgtccacggcagcggcgaaggccgcggcagcctgctgacctgcggcgatgtggaagaaaacccgggcccgatgaagtacattttgttaatactcgcgtgcattattgcatgcgtttatggagaacgctactgtgccatgcaaaatacaggctcgcagtgcattaatggcacagattcatcatgtagcacctgttttgaacgtggtggtcttatttggcatctggctaactggaacttcagctggtctgtaatattgattgtttttataacagtgttaaaatatggaagaccgcaattcagctggctcgtttatggcattaaaatgctgatcatgtggctattatggcctattgttctagcgcttacgatttttaatgcatactctgagtaccaagtttccagatatgtaatgttcggctttagtgttgcaggtgcagttgtaacgtttgcactatggatgatgtattttgtgagatctattcagctgtatagacggaccaaatcatggtggtcttttaatcctgaaaccaatgcgattctttgtgtcaatgcattgggtagaagctatgtactccctcttgatggcactcctacaggtgttactcttaccctactttcaggaaatctatacgctgaaggttttaaaatggctggtggtcttaccatcgagcatttgcctaaatatgtcatgattgctacgcctagtagaaccatcgtttacacattagttggaaaacaactaaaggcaactactgccactggatgggcttactatgtaaaatctaaagctggtgattactcaacagaagcacgtactgataatttgagtgaacatgaaaaattattacatatggtgtaagctccctttcttgctttccagggaaagtcccttggtccccagaccctaatacctggacatgtctaaatcatgaaattctttgaacatctggctcctgcctaataaagaatatttattttcattgcaaaaaaaaaaaaaaaaaaaaaaaaaaaaaaaaaaaaaaaaaaaaaaaaaaaaaaaaaaaaaaaaaaaaaaaaaaaaaaaaaaaaaaaaaaaaaaaaaaaaa

SEQ ID NO: 37 - DNA, 6705 bp, synthetic construct
  source 1..6705: mol_type = other DNA
ggatagctaccagcttacacttgcttctgacacaactgtgttcgctatcaaccacacaaacagacaccgccaccatggccacacagggacaacgcgtcaactggggagatgaaccttccaaaagacgtggtcgttctaactctcgtggtcggaagaataacactatacctctttcattcttcaatcccatccaactcgaaccaggatcaaaattttggagcgtatgtccgagagattttgttcccaagggaataggtaacaaggatcaacaaattggttattggaatagacaagagcgttaccgcattgtcaaaggtcagcgtaaggaacttcctgagaggtggtttttctacttcttaggcacaggacctcaagctgatgctaaatttaaagacaagattgatggagtcttctgggttgcaaaggatggtgccatgaataaaccaacaacacttggcactcgtggtaccaacaatgaatccaaaccactgaaatttgatggtaagataccaccgcaatttcagcttgaagtgaaccgatctaggaacaactcaagaagtggttctcagtctagatctgtctctagaaacaggtctcaatccagaggaagacaacaatccaataatcagaataatgttgaggatacaattgtagctgtgcttcagaaattaggtgttactgaaaagcaaaggtcacgttctaaatctagagatcgtggtgactctaaacctagagacacaacacctaataatgccaacaaacacacctggaagaagactgcaggtaaaggtgatgtgacaaatttctatggtgctagaagtgcttcagctaactttggtgatagtgatctcgttgccaacggtaacgctgccaaatcctaccctcagatagctgaatgcgttccatcagtgtctagcatgctcttcggtagtcaatggtctgctgaagatgatggtgatcaagtgaaagtcacgctcactcatacctattacctgccaaaagatgatgccaaaaccagccaattcctagaacagattgacgcttacaagcggccatctcaagtggctaaagatcagaggcaaagaaaatctcgttctaagtctgctgagaagaagcctgaggaattgtctgtaactcttgtagaggcatatacggatgtgtttgatgacacacaggttgagatgattgatgaggttacgaacggcagcggcgcgaccaactttagcctgctgaaacaggcgggcgatgtggaagaaaacccgggcccgatgaagtacattttgttaatactcgcgtgcattattgcatgcgtttatggagaacgctactgtgccatgcaaaatacaggctcgcagtgcattaatggcacagattcatcatgtagcacctgttttgaacgtggtggtcttatttggcatctggctaactggaacttcagctggtctgtaatattgattgtttttataacagtgttaaaatatggaagaccgcaattcagctggctcgtttatggcattaaaatgctgatcatgtggctattatggcctattgttctagcgcttacgatttttaatgcatactctgagtaccaagtttccagatatgtaatgttcggctttagtgttgcaggtgcagttgtaacgtttgcactatggatgatgtattttgtgagatctattcagctgtatagacggaccaaatcatggtggtcttttaatcctgaaaccaatgcgattctttgtgtcaatgcattgggtagaagctatgtactccctcttgatggcactcctacaggtgttactcttaccctactttcaggaaatctatacgctgaaggttttaaaatggctggtggtcttaccatcgagcatttgcctaaatatgtcatgattgctacgcctagtagaaccatcgtttacacattagttggaaaacaactaaaggcaactactgccactggatgggcttactatgtaaaatctaaagctggtgattactcaacagaagcacgtactgataatttgagtgaacatgaaaaattattacatatggtgggcagcggcgcgaccaactttagcctgctgaaacaggcgggcgatgtggaagaaaacccgggcccgatgattgtgctcgtaacttgcctcttgttgttatgttcataccacacagttttgagtacaacaaataatgaatgcatacaagttaacgtaacacaattggctggcaatgaaaaccttatcagagattttctgtttagtaactttaaagaagaaggaagtgtagttgttggtggttattaccctacagaggtgtggtacaactgctctagaacagctcgaactactgcctttcagtattttaataatatacatgccttttattttgttatggaagccatggaaaatagcactggtaatgcacgtggtaaaccattattatttcatgtgcatggtgagcctgttagtgttattatatcggcttatagggatgatgtgcaacaaaggccccttttaaaacatgggttagtgtgcataactaaaaatcgccatattaactatgaacaattcacctccaaccagtggaattccacatgtacgggtgctgacagaaaaattcctttctctgtcatacccacggacaatggaacaaaaatctatggtcttgagtggaatgatgactttgttacagcttatattagtggtcgttcttatcacttgaacatcaatactaattggtttaacaatgtcacacttttgtattcacgctcaagcactgctacctgggaatacagtgctgcatatgcttaccaaggtgtttctaacttcacttattacaagttaaataacaccaatggtctaaaaacctatgaattatgtgaagattatgaacattgcactggctatgctaccaatgtatttgctccgacatcaggtggttacatacctgatggatttagttttaacaattggttcttgcttacaaatagttccacttttgttagtggcaggtttgtaacaaatcaaccattattgattaattgcttgtggccagtgcccagttttggtgtagcagcacaagaattttgttttgaaggtgcacagtttagccaatgtaatggtgtgtctttaaataacacagtggatgttattagattcaaccttaatttcactgcagatgtacaatctggtatgggtgctacagtattttcactgaatacaacaggtggtgtcattcttgaaatttcatgttatagtgacacagtgagtgagtctagttcttacagttatggtgaaatcccgttcggcataactgacggaccacgatactgttatgtactttacaatggcacagctcttaaatatttaggaacattaccacccagtgtaaaggaaattgctattagtaagtggggccatttttatattaatggttacaatttctttagcacatttcctattggttgtatatcttttaatttaaccactggtgttagtggagctttttggacaattgcttacacatcgtatactgaagcattagtacaagttgaaaacacagctattaaaaatgtgacgtattgtaacagtcacattaataacattaaatgttctcaacttactgctaatttgaataatggattttatcctgttgcttcaagtgaagtaggtttcgttaataagagtgttgtgttattacctagctttttcacatacaccgctgtcaatataaccattgatcttggtatgaagcttagtggttatggtcaacccatagcctcgacactaagtaacatcacactaccaatgcaggataacaatactgatgtgtactgtattcgttctaaccaattctcagtttatgttcattccacttgcaaaagttctttatgggacaatatttttaatcaagactgcacggatgttttagaggctacagctgttataaaaactggtacttgtcctttctcatttgataaattgaacaattacttgacttttaacaagttctgtttgtcgttgagtcctgttggtgctaattgcaagtttgatgttgctgcacgtacaagaaccaatgagcaggttgttagaagtctatatgtaatatatgaagaaggagacaacatagtgggtgtaccgtctgataatagcggtctgcacgatttgtctgtgctacacctagactcctgtacagattacaatatatatggtagaactggtgttggtattattagacgaactaacagtacgctacttagtggcttatattacacatcactatcaggtgatttgttaggctttaaaaatgttagtgatggtgtcatttattctgtgacgccatgtgatgtaagcgcacaagcggctgttattgatggtgccatagttggagctatgacttccattaacagtgaactgttaggtctaacacattggacaacgacacctaatttttattactactctatatataattacacaagtgagaggactcgtgacactgcaattgacagtaacgatgttgattgtgaacctgtcataacctattctaatataggtgtttgtaaaaatggtgctttggtttttattaacgtcacacattctgacggagacgtgcaaccaattagcactggtaatgtcacgatacctacaaattttaccatatctgtgcaagttgaatacatgcaggtttacactacaccagtatcaatagattgtgcaagatacgtttgtaatggtaaccctagatgtaacaaattgttaacacaatatgtgtctgcatgtcaaactattgaacaagcacttgcaatgggtgccagacttgaaaacatggaggttgattccatgttgtttgtctcggaaaatgcccttaaattggcatctgttgaggcgttcaatagtacagaaaatttagattctatttacaaagaatggcctagcataggtggttcttggctaggaggtctaaaagatatactaccgtcccataatagcaaacgtaagtatggttctgctatagaagatttgctttttgataaagttgtaacatctggtttaggtacagttgatgaagattataaacgttgtactggtggttacgacatagcagacttggtgtgtgctcaatattacaatggcatcatggttctaccaggtgtagctaatgctgacaagatgactatgtacacagcatcacttgcaggtggtataacattaggtgcacttggtggtggcgccgtggctataccttttgcagtagcagtacaggctagacttaattatgttgctctacaaactgatgtattgaataaaaaccaacagatcctggctaatgccttcaatcaagctattggtaacattacacaggcttttggtaaggttaatgatgctatacatcaaacatcacaaggtcttgccactgttgctaaagcgttggcaaaagtgcaagatgttgtcaacacacaagggcaagctttaagtcaccttacagtacaattgcaaaataattttcaagccattagtagttctattagtgatatttataacaggcttgacgaactgagtgctgatgcacaagttgataggctgattacaggtagacttacagcacttaatgcatttgtgtctcagactctaaccagacaagcagaggttagggctagtagacaacttgccaaagacaaggttaatgaatgtgttaggtctcagtctcagagattcggattctgtggtaatggtacacatttgttttcactagcaaatgcagcaccaaatggcatgattttctttcatacagtactattaccaacagcttatgaaactgtaacagcttggtcaggtatttgtgcttcagatggcgatcgcactttcggacttgtcgttaaagatgtgcagttgacgttgtttcgtaatctagatgacaagttctatttgacccccagaactatgtatcagcctagagttgcaactagttctgattttgttcaaattgaagggtgtgatgtgttgtttgtcaacgcgactgtaattgatttgcctagtattatacctgactatattgacattaatcaaactgttcaagacatattagaaaattacagaccaaactggactgtacctgaatttacacttgatattttcaacgcaacctatttaaatctgactggtgaaattgatgacttagagtttaggtcagaaaagctacataacactacagtagaacttgccattctcattgataacattaataatacattagtcaatcttgaatggctcaatagaattgaaacttatgtaaaatggccttggtatgtgtggctactgataggtttagtagtagtattttgcataccattactgctattttgctgttttagcacaggttgttgtggatgcataggttgtttaggaagttgttgtcactctatatgtagtagaagacaatttgaaaattatgaaccaattgaaaaagtgcatgtccactaagctccctttcttgctttccagggaaagtcccttggtccccagaccctaatacctggacatgtctaaatcatgaaattctttgaacatctggctcctgcctaataaagaatatttattttcattgcaaaaaaaaaaaaaaaaaaaaaaaaaaaaaaaaaaaaaaaaaaaaaaaaaaaaaaaaaaaaaaaaaaaaaaaaaaaaaaaaaaaaaaaaaaaaaaaaaaaaa

SEQ ID NO: 38 - DNA, 6708 bp, synthetic construct
  source 1..6708: mol_type = other DNA
ggatagctaccagcttacacttgcttctgacacaactgtgttcgctatcaaccacacaaacagacaccgccaccatggccacacagggacaacgcgtcaactggggagatgaaccttccaaaagacgtggtcgttctaactctcgtggtcggaagaataacactatacctctttcattcttcaatcccatccaactcgaaccaggatcaaaattttggagcgtatgtccgagagattttgttcccaagggaataggtaacaaggatcaacaaattggttattggaatagacaagagcgttaccgcattgtcaaaggtcagcgtaaggaacttcctgagaggtggtttttctacttcttaggcacaggacctcaagctgatgctaaatttaaagacaagattgatggagtcttctgggttgcaaaggatggtgccatgaataaaccaacaacacttggcactcgtggtaccaacaatgaatccaaaccactgaaatttgatggtaagataccaccgcaatttcagcttgaagtgaaccgatctaggaacaactcaagaagtggttctcagtctagatctgtctctagaaacaggtctcaatccagaggaagacaacaatccaataatcagaataatgttgaggatacaattgtagctgtgcttcagaaattaggtgttactgaaaagcaaaggtcacgttctaaatctagagatcgtggtgactctaaacctagagacacaacacctaataatgccaacaaacacacctggaagaagactgcaggtaaaggtgatgtgacaaatttctatggtgctagaagtgcttcagctaactttggtgatagtgatctcgttgccaacggtaacgctgccaaatcctaccctcagatagctgaatgcgttccatcagtgtctagcatgctcttcggtagtcaatggtctgctgaagatgatggtgatcaagtgaaagtcacgctcactcatacctattacctgccaaaagatgatgccaaaaccagccaattcctagaacagattgacgcttacaagcggccatctcaagtggctaaagatcagaggcaaagaaaatctcgttctaagtctgctgagaagaagcctgaggaattgtctgtaactcttgtagaggcatatacggatgtgtttgatgacacacaggttgagatgattgatgaggttacgaacggcagcggcgcgaccaactttagcctgctgaaacaggcgggcgatgtggaagaaaacccgggcccgatgattgtgctcgtaacttgcctcttgttgttatgttcataccacacagttttgagtacaacaaataatgaatgcatacaagttaacgtaacacaattggctggcaatgaaaaccttatcagagattttctgtttagtaactttaaagaagaaggaagtgtagttgttggtggttattaccctacagaggtgtggtacaactgctctagaacagctcgaactactgcctttcagtattttaataatatacatgccttttattttgttatggaagccatggaaaatagcactggtaatgcacgtggtaaaccattattatttcatgtgcatggtgagcctgttagtgttattatatcggcttatagggatgatgtgcaacaaaggccccttttaaaacatgggttagtgtgcataactaaaaatcgccatattaactatgaacaattcacctccaaccagtggaattccacatgtacgggtgctgacagaaaaattcctttctctgtcatacccacggacaatggaacaaaaatctatggtcttgagtggaatgatgactttgttacagcttatattagtggtcgttcttatcacttgaacatcaatactaattggtttaacaatgtcacacttttgtattcacgctcaagcactgctacctgggaatacagtgctgcatatgcttaccaaggtgtttctaacttcacttattacaagttaaataacaccaatggtctaaaaacctatgaattatgtgaagattatgaacattgcactggctatgctaccaatgtatttgctccgacatcaggtggttacatacctgatggatttagttttaacaattggttcttgcttacaaatagttccacttttgttagtggcaggtttgtaacaaatcaaccattattgattaattgcttgtggccagtgcccagttttggtgtagcagcacaagaattttgttttgaaggtgcacagtttagccaatgtaatggtgtgtctttaaataacacagtggatgttattagattcaaccttaatttcactgcagatgtacaatctggtatgggtgctacagtattttcactgaatacaacaggtggtgtcattcttgaaatttcatgttatagtgacacagtgagtgagtctagttcttacagttatggtgaaatcccgttcggcataactgacggaccacgatactgttatgtactttacaatggcacagctcttaaatatttaggaacattaccacccagtgtaaaggaaattgctattagtaagtggggccatttttatattaatggttacaatttctttagcacatttcctattggttgtatatcttttaatttaaccactggtgttagtggagctttttggacaattgcttacacatcgtatactgaagcattagtacaagttgaaaacacagctattaaaaatgtgacgtattgtaacagtcacattaataacattaaatgttctcaacttactgctaatttgaataatggattttatcctgttgcttcaagtgaagtaggtttcgttaataagagtgttgtgttattacctagctttttcacatacaccgctgtcaatataaccattgatcttggtatgaagcttagtggttatggtcaacccatagcctcgacactaagtaacatcacactaccaatgcaggataacaatactgatgtgtactgtattcgttctaaccaattctcagtttatgttcattccacttgcaaaagttctttatgggacaatatttttaatcaagactgcacggatgttttagaggctacagctgttataaaaactggtacttgtcctttctcatttgataaattgaacaattacttgacttttaacaagttctgtttgtcgttgagtcctgttggtgctaattgcaagtttgatgttgctgcacgtacaagaaccaatgagcaggttgttagaagtctatatgtaatatatgaagaaggagacaacatagtgggtgtaccgtctgataatagcggtctgcacgatttgtctgtgctacacctagactcctgtacagattacaatatatatggtagaactggtgttggtattattagacgaactaacagtacgctacttagtggcttatattacacatcactatcaggtgatttgttaggctttaaaaatgttagtgatggtgtcatttattctgtgacgccatgtgatgtaagcgcacaagcggctgttattgatggtgccatagttggagctatgacttccattaacagtgaactgttaggtctaacacattggacaacgacacctaatttttattactactctatatataattacacaagtgagaggactcgtgacactgcaattgacagtaacgatgttgattgtgaacctgtcataacctattctaatataggtgtttgtaaaaatggtgctttggtttttattaacgtcacacattctgacggagacgtgcaaccaattagcactggtaatgtcacgatacctacaaattttaccatatctgtgcaagttgaatacatgcaggtttacactacaccagtatcaatagattgtgcaagatacgtttgtaatggtaaccctagatgtaacaaattgttaacacaatatgtgtctgcatgtcaaactattgaacaagcacttgcaatgggtgccagacttgaaaacatggaggttgattccatgttgtttgtctcggaaaatgcccttaaattggcatctgttgaggcgttcaatagtacagaaaatttagattctatttacaaagaatggcctagcataggtggttcttggctaggaggtctaaaagatatactaccgtcccataatagcaaacgtaagtatggttctgctatagaagatttgctttttgataaagttgtaacatctggtttaggtacagttgatgaagattataaacgttgtactggtggttacgacatagcagacttggtgtgtgctcaatattacaatggcatcatggttctaccaggtgtagctaatgctgacaagatgactatgtacacagcatcacttgcaggtggtataacattaggtgcacttggtggtggcgccgtggctataccttttgcagtagcagtacaggctagacttaattatgttgctctacaaactgatgtattgaataaaaaccaacagatcctggctaatgccttcaatcaagctattggtaacattacacaggcttttggtaaggttaatgatgctatacatcaaacatcacaaggtcttgccactgttgctaaagcgttggcaaaagtgcaagatgttgtcaacacacaagggcaagctttaagtcaccttacagtacaattgcaaaataattttcaagccattagtagttctattagtgatatttataacaggcttgacgaactgagtgctgatgcacaagttgataggctgattacaggtagacttacagcacttaatgcatttgtgtctcagactctaaccagacaagcagaggttagggctagtagacaacttgccaaagacaaggttaatgaatgtgttaggtctcagtctcagagattcggattctgtggtaatggtacacatttgttttcactagcaaatgcagcaccaaatggcatgattttctttcatacagtactattaccaacagcttatgaaactgtaacagcttggtcaggtatttgtgcttcagatggcgatcgcactttcggacttgtcgttaaagatgtgcagttgacgttgtttcgtaatctagatgacaagttctatttgacccccagaactatgtatcagcctagagttgcaactagttctgattttgttcaaattgaagggtgtgatgtgttgtttgtcaacgcgactgtaattgatttgcctagtattatacctgactatattgacattaatcaaactgttcaagacatattagaaaattacagaccaaactggactgtacctgaatttacacttgatattttcaacgcaacctatttaaatctgactggtgaaattgatgacttagagtttaggtcagaaaagctacataacactacagtagaacttgccattctcattgataacattaataatacattagtcaatcttgaatggctcaatagaattgaaacttatgtaaaatggccttggtatgtgtggctactgataggtttagtagtagtattttgcataccattactgctattttgctgttttagcacaggttgttgtggatgcataggttgtttaggaagttgttgtcactctatatgtagtagaagacaatttgaaaattatgaaccaattgaaaaagtgcatgtccactaaggcagcggcgcgaccaactttagcctgctgaaacaggcgggcgatgtggaagaaaacccgggcccgatgaagtacattttgttaatactcgcgtgcattattgcatgcgtttatggagaacgctactgtgccatgcaaaatacaggctcgcagtgcattaatggcacagattcatcatgtagcacctgttttgaacgtggtggtcttatttggcatctggctaactggaacttcagctggtctgtaatattgattgtttttataacagtgttaaaatatggaagaccgcaattcagctggctcgtttatggcattaaaatgctgatcatgtggctattatggcctattgttctagcgcttacgatttttaatgcatactctgagtaccaagtttccagatatgtaatgttcggctttagtgttgcaggtgcagttgtaacgtttgcactatggatgatgtattttgtgagatctattcagctgtatagacggaccaaatcatggtggtcttttaatcctgaaaccaatgcgattctttgtgtcaatgcattgggtagaagctatgtactccctcttgatggcactcctacaggtgttactcttaccctactttcaggaaatctatacgctgaaggttttaaaatggctggtggtcttaccatcgagcatttgcctaaatatgtcatgattgctacgcctagtagaaccatcgtttacacattagttggaaaacaactaaaggcaactactgccactggatgggcttactatgtaaaatctaaagctggtgattactcaacagaagcacgtactgataatttgagtgaacatgaaaaattattacatatggtgtaagctccctttcttgctttccagggaaagtcccttggtccccagaccctaatacctggacatgtctaaatcatgaaattctttgaacatctggctcctgcctaataaagaatatttattttcattgcaaaaaaaaaaaaaaaaaaaaaaaaaaaaaaaaaaaaaaaaaaaaaaaaaaaaaaaaaaaaaaaaaaaaaaaaaaaaaaaaaaaaaaaaaaaaaaaaaaaaa

SEQ ID NO: 39 - DNA, 4371 bp, synthetic construct
  source 1..4371: mol_type = other DNA
ggatagctaccagcttacacttgcttctgacacaactgtgttcgctatcaaccacacaaacagacaccgccaccatggccacacagggacaacgcgtcaactggggagatgaaccttccaaaagacgtggtcgttctaactctcgtggtcggaagaataacactatacctctttcattcttcaatcccatccaactcgaaccaggatcaaaattttggagcgtatgtccgagagattttgttcccaagggaataggtaacaaggatcaacaaattggttattggaatagacaagagcgttaccgcattgtcaaaggtcagcgtaaggaacttcctgagaggtggtttttctacttcttaggcacaggacctcaagctgatgctaaatttaaagacaagattgatggagtcttctgggttgcaaaggatggtgccatgaataaaccaacaacacttggcactcgtggtaccaacaatgaatccaaaccactgaaatttgatggtaagataccaccgcaatttcagcttgaagtgaaccgatctaggaacaactcaagaagtggttctcagtctagatctgtctctagaaacaggtctcaatccagaggaagacaacaatccaataatcagaataatgttgaggatacaattgtagctgtgcttcagaaattaggtgttactgaaaagcaaaggtcacgttctaaatctagagatcgtggtgactctaaacctagagacacaacacctaataatgccaacaaacacacctggaagaagactgcaggtaaaggtgatgtgacaaatttctatggtgctagaagtgcttcagctaactttggtgatagtgatctcgttgccaacggtaacgctgccaaatcctaccctcagatagctgaatgcgttccatcagtgtctagcatgctcttcggtagtcaatggtctgctgaagatgatggtgatcaagtgaaagtcacgctcactcatacctattacctgccaaaagatgatgccaaaaccagccaattcctagaacagattgacgcttacaagcggccatctcaagtggctaaagatcagaggcaaagaaaatctcgttctaagtctgctgagaagaagcctgaggaattgtctgtaactcttgtagaggcatatacggatgtgtttgatgacacacaggttgagatgattgatgaggttacgaacggcagcggcgcgaccaactttagcctgctgaaacaggcgggcgatgtggaagaaaacccgggcccgatgaagtacattttgttaatactcgcgtgcattattgcatgcgtttatggagaacgctactgtgccatgcaaaatacaggctcgcagtgcattaatggcacagattcatcatgtagcacctgttttgaacgtggtggtcttatttggcatctggctaactggaacttcagctggtctgtaatattgattgtttttataacagtgttaaaatatggaagaccgcaattcagctggctcgtttatggcattaaaatgctgatcatgtggctattatggcctattgttctagcgcttacgatttttaatgcatactctgagtaccaagtttccagatatgtaatgttcggctttagtgttgcaggtgcagttgtaacgtttgcactatggatgatgtattttgtgagatctattcagctgtatagacggaccaaatcatggtggtcttttaatcctgaaaccaatgcgattctttgtgtcaatgcattgggtagaagctatgtactccctcttgatggcactcctacaggtgttactcttaccctactttcaggaaatctatacgctgaaggttttaaaatggctggtggtcttaccatcgagcatttgcctaaatatgtcatgattgctacgcctagtagaaccatcgtttacacattagttggaaaacaactaaaggcaactactgccactggatgggcttactatgtaaaatctaaagctggtgattactcaacagaagcacgtactgataatttgagtgaacatgaaaaattattacatatggtgggcagcggcgcgaccaactttagcctgctgaaacaggcgggcgatgtggaagaaaacccgggcccgatgtctatatataattacacaagtgagaggactcgtgacactgcaattgacagtaacgatgttgattgtgaacctgtcataacctattctaatataggtgtttgtaaaaatggtgctttggtttttattaacgtcacacattctgacggagacgtgcaaccaattagcactggtaatgtcacgatacctacaaattttaccatatctgtgcaagttgaatacatgcaggtttacactacaccagtatcaatagattgtgcaagatacgtttgtaatggtaaccctagatgtaacaaattgttaacacaatatgtgtctgcatgtcaaactattgaacaagcacttgcaatgggtgccagacttgaaaacatggaggttgattccatgttgtttgtctcggaaaatgcccttaaattggcatctgttgaggcgttcaatagtacagaaaatttagattctatttacaaagaatggcctagcataggtggttcttggctaggaggtctaaaagatatactaccgtcccataatagcaaacgtaagtatggttctgctatagaagatttgctttttgataaagttgtaacatctggtttaggtacagttgatgaagattataaacgttgtactggtggttacgacatagcagacttggtgtgtgctcaatattacaatggcatcatggttctaccaggtgtagctaatgctgacaagatgactatgtacacagcatcacttgcaggtggtataacattaggtgcacttggtggtggcgccgtggctataccttttgcagtagcagtacaggctagacttaattatgttgctctacaaactgatgtattgaataaaaaccaacagatcctggctaatgccttcaatcaagctattggtaacattacacaggcttttggtaaggttaatgatgctatacatcaaacatcacaaggtcttgccactgttgctaaagcgttggcaaaagtgcaagatgttgtcaacacacaagggcaagctttaagtcaccttacagtacaattgcaaaataattttcaagccattagtagttctattagtgatatttataacaggcttgacgaactgagtgctgatgcacaagttgataggctgattacaggtagacttacagcacttaatgcatttgtgtctcagactctaaccagacaagcagaggttagggctagtagacaacttgccaaagacaaggttaatgaatgtgttaggtctcagtctcagagattcggattctgtggtaatggtacacatttgttttcactagcaaatgcagcaccaaatggcatgattttctttcatacagtactattaccaacagcttatgaaactgtaacagcttggtcaggtatttgtgcttcagatggcgatcgcactttcggacttgtcgttaaagatgtgcagttgacgttgtttcgtaatctagatgacaagttctatttgacccccagaactatgtatcagcctagagttgcaactagttctgattttgttcaaattgaagggtgtgatgtgttgtttgtcaacgcgactgtaattgatttgcctagtattatacctgactatattgacattaatcaaactgttcaagacatattagaaaattacagaccaaactggactgtacctgaatttacacttgatattttcaacgcaacctatttaaatctgactggtgaaattgatgacttagagtttaggtcagaaaagctacataacactacagtagaacttgccattctcattgataacattaataatacattagtcaatcttgaatggctcaatagaattgaaacttatgtaaaatggccttggtatgtgtggctactgataggtttagtagtagtattttgcataccattactgctattttgctgttttagcacaggttgttgtggatgcataggttgtttaggaagttgttgtcactctatatgtagtagaagacaatttgaaaattatgaaccaattgaaaaagtgcatgtccactaagctccctttcttgctttccagggaaagtcccttggtccccagaccctaatacctggacatgtctaaatcatgaaattctttgaacatctggctcctgcctaataaagaatatttattttcattgcaaaaaaaaaaaaaaaaaaaaaaaaaaaaaaaaaaaaaaaaaaaaaaaaaaaaaaaaaaaaaaaaaaaaaaaaaaaaaaaaaaaaaaaaaaaaaaaaaaaaa

SEQ ID NO: 40 - DNA, 4371 bp, synthetic construct
  source 1..4371: mol_type = other DNA
ggatagctaccagcttacacttgcttctgacacaactgtgttcgctatcaaccacacaaacagacaccgccaccatggccacacagggacaacgcgtcaactggggagatgaaccttccaaaagacgtggtcgttctaactctcgtggtcggaagaataacactatacctctttcattcttcaatcccatccaactcgaaccaggatcaaaattttggagcgtatgtccgagagattttgttcccaagggaataggtaacaaggatcaacaaattggttattggaatagacaagagcgttaccgcattgtcaaaggtcagcgtaaggaacttcctgagaggtggtttttctacttcttaggcacaggacctcaagctgatgctaaatttaaagacaagattgatggagtcttctgggttgcaaaggatggtgccatgaataaaccaacaacacttggcactcgtggtaccaacaatgaatccaaaccactgaaatttgatggtaagataccaccgcaatttcagcttgaagtgaaccgatctaggaacaactcaagaagtggttctcagtctagatctgtctctagaaacaggtctcaatccagaggaagacaacaatccaataatcagaataatgttgaggatacaattgtagctgtgcttcagaaattaggtgttactgaaaagcaaaggtcacgttctaaatctagagatcgtggtgactctaaacctagagacacaacacctaataatgccaacaaacacacctggaagaagactgcaggtaaaggtgatgtgacaaatttctatggtgctagaagtgcttcagctaactttggtgatagtgatctcgttgccaacggtaacgctgccaaatcctaccctcagatagctgaatgcgttccatcagtgtctagcatgctcttcggtagtcaatggtctgctgaagatgatggtgatcaagtgaaagtcacgctcactcatacctattacctgccaaaagatgatgccaaaaccagccaattcctagaacagattgacgcttacaagcggccatctcaagtggctaaagatcagaggcaaagaaaatctcgttctaagtctgctgagaagaagcctgaggaattgtctgtaactcttgtagaggcatatacggatgtgtttgatgacacacaggttgagatgattgatgaggttacgaacggcagcggcgcgaccaactttagcctgctgaaacaggcgggcgatgtggaagaaaacccgggcccgatgtctatatataattacacaagtgagaggactcgtgacactgcaattgacagtaacgatgttgattgtgaacctgtcataacctattctaatataggtgtttgtaaaaatggtgctttggtttttattaacgtcacacattctgacggagacgtgcaaccaattagcactggtaatgtcacgatacctacaaattttaccatatctgtgcaagttgaatacatgcaggtttacactacaccagtatcaatagattgtgcaagatacgtttgtaatggtaaccctagatgtaacaaattgttaacacaatatgtgtctgcatgtcaaactattgaacaagcacttgcaatgggtgccagacttgaaaacatggaggttgattccatgttgtttgtctcggaaaatgcccttaaattggcatctgttgaggcgttcaatagtacagaaaatttagattctatttacaaagaatggcctagcataggtggttcttggctaggaggtctaaaagatatactaccgtcccataatagcaaacgtaagtatggttctgctatagaagatttgctttttgataaagttgtaacatctggtttaggtacagttgatgaagattataaacgttgtactggtggttacgacatagcagacttggtgtgtgctcaatattacaatggcatcatggttctaccaggtgtagctaatgctgacaagatgactatgtacacagcatcacttgcaggtggtataacattaggtgcacttggtggtggcgccgtggctataccttttgcagtagcagtacaggctagacttaattatgttgctctacaaactgatgtattgaataaaaaccaacagatcctggctaatgccttcaatcaagctattggtaacattacacaggcttttggtaaggttaatgatgctatacatcaaacatcacaaggtcttgccactgttgctaaagcgttggcaaaagtgcaagatgttgtcaacacacaagggcaagctttaagtcaccttacagtacaattgcaaaataattttcaagccattagtagttctattagtgatatttataacaggcttgacgaactgagtgctgatgcacaagttgataggctgattacaggtagacttacagcacttaatgcatttgtgtctcagactctaaccagacaagcagaggttagggctagtagacaacttgccaaagacaaggttaatgaatgtgttaggtctcagtctcagagattcggattctgtggtaatggtacacatttgttttcactagcaaatgcagcaccaaatggcatgattttctttcatacagtactattaccaacagcttatgaaactgtaacagcttggtcaggtatttgtgcttcagatggcgatcgcactttcggacttgtcgttaaagatgtgcagttgacgttgtttcgtaatctagatgacaagttctatttgacccccagaactatgtatcagcctagagttgcaactagttctgattttgttcaaattgaagggtgtgatgtgttgtttgtcaacgcgactgtaattgatttgcctagtattatacctgactatattgacattaatcaaactgttcaagacatattagaaaattacagaccaaactggactgtacctgaatttacacttgatattttcaacgcaacctatttaaatctgactggtgaaattgatgacttagagtttaggtcagaaaagctacataacactacagtagaacttgccattctcattgataacattaataatacattagtcaatcttgaatggctcaatagaattgaaacttatgtaaaatggccttggtatgtgtggctactgataggtttagtagtagtattttgcataccattactgctattttgctgttttagcacaggttgttgtggatgcataggttgtttaggaagttgttgtcactctatatgtagtagaagacaatttgaaaattatgaaccaattgaaaaagtgcatgtccacggcagcggcgcgaccaactttagcctgctgaaacaggcgggcgatgtggaagaaaacccgggcccgatgaagtacattttgttaatactcgcgtgcattattgcatgcgtttatggagaacgctactgtgccatgcaaaatacaggctcgcagtgcattaatggcacagattcatcatgtagcacctgttttgaacgtggtggtcttatttggcatctggctaactggaacttcagctggtctgtaatattgattgtttttataacagtgttaaaatatggaagaccgcaattcagctggctcgtttatggcattaaaatgctgatcatgtggctattatggcctattgttctagcgcttacgatttttaatgcatactctgagtaccaagtttccagatatgtaatgttcggctttagtgttgcaggtgcagttgtaacgtttgcactatggatgatgtattttgtgagatctattcagctgtatagacggaccaaatcatggtggtcttttaatcctgaaaccaatgcgattctttgtgtcaatgcattgggtagaagctatgtactccctcttgatggcactcctacaggtgttactcttaccctactttcaggaaatctatacgctgaaggttttaaaatggctggtggtcttaccatcgagcatttgcctaaatatgtcatgattgctacgcctagtagaaccatcgtttacacattagttggaaaacaactaaaggcaactactgccactggatgggcttactatgtaaaatctaaagctggtgattactcaacagaagcacgtactgataatttgagtgaacatgaaaaattattacatatggtgtaagctccctttcttgctttccagggaaagtcccttggtccccagaccctaatacctggacatgtctaaatcatgaaattctttgaacatctggctcctgcctaataaagaatatttattttcattgcaaaaaaaaaaaaaaaaaaaaaaaaaaaaaaaaaaaaaaaaaaaaaaaaaaaaaaaaaaaaaaaaaaaaaaaaaaaaaaaaaaaaaaaaaaaaaaaaaaaaa

SEQ ID NO: 41-57 - skipped (17 entries)

SEQ ID NO: 58 - protein, 21 aa, synthetic construct
GSGEGRGSLLTCGDVEENPGP

SEQ ID NO: 59 - protein, 22 aa, synthetic construct
GSGATNFSLLKQAGDVEENPGP

SEQ ID NO: 60 - protein, 262 aa, Feline Coronavirus
MKYILLILACIIACVYGERYCAMQNTGSQCINGTDSSCSTCFERGGLIWHLANWNFSWSVILIVFITVLKYGRPQFSWLVYGIKMLIMWLLWPIVLALTIFNAYSEYQVSRYVMFGFSVAGAVVTFALWMMYFVRSIQLYRRTKSWWSFNPETNAILCVNALGRSYVLPLDGTPTGVTLTLLSGNLYAEGFKMAGGLTIEHLPKYVMIATPSRTIVYTLVGKQLKATTATGWAYYVKSKAGDYSTEARTDNLSEHEKLLHMV

SEQ ID NO: 61 - protein, 376 aa, Feline Coronavirus
MATQGQRVNWGDEPSKRRGRSNSRGRKNNTIPLSFFNPIQLEPGSKFWSVCPRDFVPKGIGNKDQQIGYWNRQERYRIVKGQRKELPERWFFYFLGTGPQADAKFKDKIDGVFWVAKDGAMNKPTTLGTRGTNNESKPLKFDGKIPPQFQLEVNRSRNNSRSGSQSRSVSRNRSQSRGRQQSNNQNNVEDTIVAVLQKLGVTEKQRSRSKSRDRGDSKPRDTTPNNANKHTWKKTAGKGDVTNFYGARSASANFGDSDLVANGNAAKSYPQIAECVPSVSSMLFGSQWSAEDDGDQVKVTLTHTYYLPKDDAKTSQFLEQIDAYKRPSQVAKDQRQRKSRSKSAEKKPEELSVTLVEAYTDVFDDTQVEMIDEVTN

SEQ ID NO: 62 - protein, 1452 aa, synthetic construct
MIVLVTCLLLLCSYHTVLSTTNNECIQVNVTQLAGNENLIRDFLFSNFKEEGSVVVGGYYPTEVWYNCSRTARTTAFQYFNNIHAFYFVMEAMENSTGNARGKPLLFHVHGEPVSVIISAYRDDVQQRPLLKHGLVCITKNRHINYEQFTSNQWNSTCTGADRKIPFSVIPTDNGTKIYGLEWNDDFVTAYISGRSYHLNINTNWFNNVTLLYSRSSTATWEYSAAYAYQGVSNFTYYKLNNTNGLKTYELCEDYEHCTGYATNVFAPTSGGYIPDGFSFNNWFLLTNSSTFVSGRFVTNQPLLINCLWPVPSFGVAAQEFCFEGAQFSQCNGVSLNNTVDVIRFNLNFTADVQSGMGATVFSLNTTGGVILEISCYSDTVSESSSYSYGEIPFGITDGPRYCYVLYNGTALKYLGTLPPSVKEIAISKWGHFYINGYNFFSTFPIGCISFNLTTGVSGAFWTIAYTSYTEALVQVENTAIKNVTYCNSHINNIKCSQLTANLNNGFYPVASSEVGFVNKSVVLLPSFFTYTAVNITIDLGMKLSGYGQPIASTLSNITLPMQDNNTDVYCIRSNQFSVYVHSTCKSSLWDNIFNQDCTDVLEATAVIKTGTCPFSFDKLNNYLTFNKFCLSLSPVGANCKFDVAARTRTNEQVVRSLYVIYEEGDNIVGVPSDNSGLHDLSVLHLDSCTDYNIYGRTGVGIIRRTNSTLLSGLYYTSLSGDLLGFKNVSDGVIYSVTPCDVSAQAAVIDGAIVGAMTSINSELLGLTHWTTTPNFYYYSIYNYTSERTRDTAIDSNDVDCEPVITYSNIGVCKNGALVFINVTHSDGDVQPISTGNVTIPTNFTISVQVEYMQVYTTPVSIDCARYVCNGNPRCNKLLTQYVSACQTIEQALAMGARLENMEVDSMLFVSENALKLASVEAFNSTENLDSIYKEWPSIGGSWLGGLKDILPSHNSKRKYGSAIEDLLFDKVVTSGLGTVDEDYKRCTGGYDIADLVCAQYYNGIMVLPGVANADKMTMYTASLAGGITLGALGGGAVAIPFAVAVQARLNYVALQTDVLNKNQQILANAFNQAIGNITQAFGKVNDAIHQTSQGLATVAKALAKVQDVVNTQGQALSHLTVQLQNNFQAISSSISDIYNRLDELSADAQVDRLITGRLTALNAFVSQTLTRQAEVRASRQLAKDKVNECVRSQSQRFGFCGNGTHLFSLANAAPNGMIFFHTVLLPTAYETVTAWSGICASDGDRTFGLVVKDVQLTLFRNLDDKFYLTPRTMYQPRVATSSDFVQIEGCDVLFVNATVIDLPSIIPDYIDINQTVQDILENYRPNWTVPEFTLDIFNATYLNLTGEIDDLEFRSEKLHNTTVELAILIDNINNTLVNLEWLNRIETYVKWPWYVWLLIGLVVVFCIPLLLFCCFSTGCCGCIGCLGSCCHSICSRRQFENYEPIEKVHVH

SEQ ID NO: 63 - protein, 779 aa, Feline Coronavirus
MIVLVTCLLLLCSYHTVLSTTNNECIQVNVTQLAGNENLIRDFLFSNFKEEGSVVVGGYYPTEVWYNCSRTARTTAFQYFNNIHAFYFVMEAMENSTGNARGKPLLFHVHGEPVSVIISAYRDDVQQRPLLKHGLVCITKNRHINYEQFTSNQWNSTCTGADRKIPFSVIPTDNGTKIYGLEWNDDFVTAYISGRSYHLNINTNWFNNVTLLYSRSSTATWEYSAAYAYQGVSNFTYYKLNNTNGLKTYELCEDYEHCTGYATNVFAPTSGGYIPDGFSFNNWFLLTNSSTFVSGRFVTNQPLLINCLWPVPSFGVAAQEFCFEGAQFSQCNGVSLNNTVDVIRFNLNFTADVQSGMGATVFSLNTTGGVILEISCYSDTVSESSSYSYGEIPFGITDGPRYCYVLYNGTALKYLGTLPPSVKEIAISKWGHFYINGYNFFSTFPIGCISFNLTTGVSGAFWTIAYTSYTEALVQVENTAIKNVTYCNSHINNIKCSQLTANLNNGFYPVASSEVGFVNKSVVLLPSFFTYTAVNITIDLGMKLSGYGQPIASTLSNITLPMQDNNTDVYCIRSNQFSVYVHSTCKSSLWDNIFNQDCTDVLEATAVIKTGTCPFSFDKLNNYLTFNKFCLSLSPVGANCKFDVAARTRTNEQVVRSLYVIYEEGDNIVGVPSDNSGLHDLSVLHLDSCTDYNIYGRTGVGIIRRTNSTLLSGLYYTSLSGDLLGFKNVSDGVIYSVTPCDVSAQAAVIDGAIVGAMTSINSELLGLTHWTTTPNFYYY

SEQ ID NO: 64 - protein, 674 aa, synthetic construct
MSIYNYTSERTRDTAIDSNDVDCEPVITYSNIGVCKNGALVFINVTHSDGDVQPISTGNVTIPTNFTISVQVEYMQVYTTPVSIDCARYVCNGNPRCNKLLTQYVSACQTIEQALAMGARLENMEVDSMLFVSENALKLASVEAFNSTENLDSIYKEWPSIGGSWLGGLKDILPSHNSKRKYGSAIEDLLFDKVVTSGLGTVDEDYKRCTGGYDIADLVCAQYYNGIMVLPGVANADKMTMYTASLAGGITLGALGGGAVAIPFAVAVQARLNYVALQTDVLNKNQQILANAFNQAIGNITQAFGKVNDAIHQTSQGLATVAKALAKVQDVVNTQGQALSHLTVQLQNNFQAISSSISDIYNRLDELSADAQVDRLITGRLTALNAFVSQTLTRQAEVRASRQLAKDKVNECVRSQSQRFGFCGNGTHLFSLANAAPNGMIFFHTVLLPTAYETVTAWSGICASDGDRTFGLVVKDVQLTLFRNLDDKFYLTPRTMYQPRVATSSDFVQIEGCDVLFVNATVIDLPSIIPDYIDINQTVQDILENYRPNWTVPEFTLDIFNATYLNLTGEIDDLEFRSEKLHNTTVELAILIDNINNTLVNLEWLNRIETYVKWPWYVWLLIGLVVVFCIPLLLFCCFSTGCCGCIGCLGSCCHSICSRRQFENYEPIEKVHVH

SEQ ID NO: 65 - protein, 659 aa, synthetic construct
MKYILLILACIIACVYGERYCAMQNTGSQCINGTDSSCSTCFERGGLIWHLANWNFSWSVILIVFITVLKYGRPQFSWLVYGIKMLIMWLLWPIVLALTIFNAYSEYQVSRYVMFGFSVAGAVVTFALWMMYFVRSIQLYRRTKSWWSFNPETNAILCVNALGRSYVLPLDGTPTGVTLTLLSGNLYAEGFKMAGGLTIEHLPKYVMIATPSRTIVYTLVGKQLKATTATGWAYYVKSKAGDYSTEARTDNLSEHEKLLHMVGSGEGRGSLLTCGDVEENPGPMATQGQRVNWGDEPSKRRGRSNSRGRKNNTIPLSFFNPIQLEPGSKFWSVCPRDFVPKGIGNKDQQIGYWNRQERYRIVKGQRKELPERWFFYFLGTGPQADAKFKDKIDGVFWVAKDGAMNKPTTLGTRGTNNESKPLKFDGKIPPQFQLEVNRSRNNSRSGSQSRSVSRNRSQSRGRQQSNNQNNVEDTIVAVLQKLGVTEKQRSRSKSRDRGDSKPRDTTPNNANKHTWKKTAGKGDVTNFYGARSASANFGDSDLVANGNAAKSYPQIAECVPSVSSMLFGSQWSAEDDGDQVKVTLTHTYYLPKDDAKTSQFLEQIDAYKRPSQVAKDQRQRKSRSKSAEKKPEELSVTLVEAYTDVFDDTQVEMIDEVTN

SEQ ID NO: 66 - protein, 659 aa, synthetic construct
MATQGQRVNWGDEPSKRRGRSNSRGRKNNTIPLSFFNPIQLEPGSKFWSVCPRDFVPKGIGNKDQQIGYWNRQERYRIVKGQRKELPERWFFYFLGTGPQADAKFKDKIDGVFWVAKDGAMNKPTTLGTRGTNNESKPLKFDGKIPPQFQLEVNRSRNNSRSGSQSRSVSRNRSQSRGRQQSNNQNNVEDTIVAVLQKLGVTEKQRSRSKSRDRGDSKPRDTTPNNANKHTWKKTAGKGDVTNFYGARSASANFGDSDLVANGNAAKSYPQIAECVPSVSSMLFGSQWSAEDDGDQVKVTLTHTYYLPKDDAKTSQFLEQIDAYKRPSQVAKDQRQRKSRSKSAEKKPEELSVTLVEAYTDVFDDTQVEMIDEVTNGSGEGRGSLLTCGDVEENPGPMKYILLILACIIACVYGERYCAMQNTGSQCINGTDSSCSTCFERGGLIWHLANWNFSWSVILIVFITVLKYGRPQFSWLVYGIKMLIMWLLWPIVLALTIFNAYSEYQVSRYVMFGFSVAGAVVTFALWMMYFVRSIQLYRRTKSWWSFNPETNAILCVNALGRSYVLPLDGTPTGVTLTLLSGNLYAEGFKMAGGLTIEHLPKYVMIATPSRTIVYTLVGKQLKATTATGWAYYVKSKAGDYSTEARTDNLSEHEKLLHMV

SEQ ID NO: 67 - protein, 660 aa, synthetic construct
MKYILLILACIIACVYGERYCAMQNTGSQCINGTDSSCSTCFERGGLIWHLANWNFSWSVILIVFITVLKYGRPQFSWLVYGIKMLIMWLLWPIVLALTIFNAYSEYQVSRYVMFGFSVAGAVVTFALWMMYFVRSIQLYRRTKSWWSFNPETNAILCVNALGRSYVLPLDGTPTGVTLTLLSGNLYAEGFKMAGGLTIEHLPKYVMIATPSRTIVYTLVGKQLKATTATGWAYYVKSKAGDYSTEARTDNLSEHEKLLHMVGSGATNFSLLKQAGDVEENPGPMATQGQRVNWGDEPSKRRGRSNSRGRKNNTIPLSFFNPIQLEPGSKFWSVCPRDFVPKGIGNKDQQIGYWNRQERYRIVKGQRKELPERWFFYFLGTGPQADAKFKDKIDGVFWVAKDGAMNKPTTLGTRGTNNESKPLKFDGKIPPQFQLEVNRSRNNSRSGSQSRSVSRNRSQSRGRQQSNNQNNVEDTIVAVLQKLGVTEKQRSRSKSRDRGDSKPRDTTPNNANKHTWKKTAGKGDVTNFYGARSASANFGDSDLVANGNAAKSYPQIAECVPSVSSMLFGSQWSAEDDGDQVKVTLTHTYYLPKDDAKTSQFLEQIDAYKRPSQVAKDQRQRKSRSKSAEKKPEELSVTLVEAYTDVFDDTQVEMIDEVTN

SEQ ID NO: 68 - protein, 660 aa, synthetic construct
MATQGQRVNWGDEPSKRRGRSNSRGRKNNTIPLSFFNPIQLEPGSKFWSVCPRDFVPKGIGNKDQQIGYWNRQERYRIVKGQRKELPERWFFYFLGTGPQADAKFKDKIDGVFWVAKDGAMNKPTTLGTRGTNNESKPLKFDGKIPPQFQLEVNRSRNNSRSGSQSRSVSRNRSQSRGRQQSNNQNNVEDTIVAVLQKLGVTEKQRSRSKSRDRGDSKPRDTTPNNANKHTWKKTAGKGDVTNFYGARSASANFGDSDLVANGNAAKSYPQIAECVPSVSSMLFGSQWSAEDDGDQVKVTLTHTYYLPKDDAKTSQFLEQIDAYKRPSQVAKDQRQRKSRSKSAEKKPEELSVTLVEAYTDVFDDTQVEMIDEVTNGSGATNFSLLKQAGDVEENPGPMKYILLILACIIACVYGERYCAMQNTGSQCINGTDSSCSTCFERGGLIWHLANWNFSWSVILIVFITVLKYGRPQFSWLVYGIKMLIMWLLWPIVLALTIFNAYSEYQVSRYVMFGFSVAGAVVTFALWMMYFVRSIQLYRRTKSWWSFNPETNAILCVNALGRSYVLPLDGTPTGVTLTLLSGNLYAEGFKMAGGLTIEHLPKYVMIATPSRTIVYTLVGKQLKATTATGWAYYVKSKAGDYSTEARTDNLSEHEKLLHMV

SEQ ID NO: 69 - protein, 2132 aa, synthetic construct
MATQGQRVNWGDEPSKRRGRSNSRGRKNNTIPLSFFNPIQLEPGSKFWSVCPRDFVPKGIGNKDQQIGYWNRQERYRIVKGQRKELPERWFFYFLGTGPQADAKFKDKIDGVFWVAKDGAMNKPTTLGTRGTNNESKPLKFDGKIPPQFQLEVNRSRNNSRSGSQSRSVSRNRSQSRGRQQSNNQNNVEDTIVAVLQKLGVTEKQRSRSKSRDRGDSKPRDTTPNNANKHTWKKTAGKGDVTNFYGARSASANFGDSDLVANGNAAKSYPQIAECVPSVSSMLFGSQWSAEDDGDQVKVTLTHTYYLPKDDAKTSQFLEQIDAYKRPSQVAKDQRQRKSRSKSAEKKPEELSVTLVEAYTDVFDDTQVEMIDEVTNGSGEGRGSLLTCGDVEENPGPMKYILLILACIIACVYGERYCAMQNTGSQCINGTDSSCSTCFERGGLIWHLANWNFSWSVILIVFITVLKYGRPQFSWLVYGIKMLIMWLLWPIVLALTIFNAYSEYQVSRYVMFGFSVAGAVVTFALWMMYFVRSIQLYRRTKSWWSFNPETNAILCVNALGRSYVLPLDGTPTGVTLTLLSGNLYAEGFKMAGGLTIEHLPKYVMIATPSRTIVYTLVGKQLKATTATGWAYYVKSKAGDYSTEARTDNLSEHEKLLHMVGSGEGRGSLLTCGDVEENPGPMIVLVTCLLLLCSYHTVLSTTNNECIQVNVTQLAGNENLIRDFLFSNFKEEGSVVVGGYYPTEVWYNCSRTARTTAFQYFNNIHAFYFVMEAMENSTGNARGKPLLFHVHGEPVSVIISAYRDDVQQRPLLKHGLVCITKNRHINYEQFTSNQWNSTCTGADRKIPFSVIPTDNGTKIYGLEWNDDFVTAYISGRSYHLNINTNWFNNVTLLYSRSSTATWEYSAAYAYQGVSNFTYYKLNNTNGLKTYELCEDYEHCTGYATNVFAPTSGGYIPDGFSFNNWFLLTNSSTFVSGRFVTNQPLLINCLWPVPSFGVAAQEFCFEGAQFSQCNGVSLNNTVDVIRFNLNFTADVQSGMGATVFSLNTTGGVILEISCYSDTVSESSSYSYGEIPFGITDGPRYCYVLYNGTALKYLGTLPPSVKEIAISKWGHFYINGYNFFSTFPIGCISFNLTTGVSGAFWTIAYTSYTEALVQVENTAIKNVTYCNSHINNIKCSQLTANLNNGFYPVASSEVGFVNKSVVLLPSFFTYTAVNITIDLGMKLSGYGQPIASTLSNITLPMQDNNTDVYCIRSNQFSVYVHSTCKSSLWDNIFNQDCTDVLEATAVIKTGTCPFSFDKLNNYLTFNKFCLSLSPVGANCKFDVAARTRTNEQVVRSLYVIYEEGDNIVGVPSDNSGLHDLSVLHLDSCTDYNIYGRTGVGIIRRTNSTLLSGLYYTSLSGDLLGFKNVSDGVIYSVTPCDVSAQAAVIDGAIVGAMTSINSELLGLTHWTTTPNFYYYSIYNYTSERTRDTAIDSNDVDCEPVITYSNIGVCKNGALVFINVTHSDGDVQPISTGNVTIPTNFTISVQVEYMQVYTTPVSIDCARYVCNGNPRCNKLLTQYVSACQTIEQALAMGARLENMEVDSMLFVSENALKLASVEAFNSTENLDSIYKEWPSIGGSWLGGLKDILPSHNSKRKYGSAIEDLLFDKVVTSGLGTVDEDYKRCTGGYDIADLVCAQYYNGIMVLPGVANADKMTMYTASLAGGITLGALGGGAVAIPFAVAVQARLNYVALQTDVLNKNQQILANAFNQAIGNITQAFGKVNDAIHQTSQGLATVAKALAKVQDVVNTQGQALSHLTVQLQNNFQAISSSISDIYNRLDELSADAQVDRLITGRLTALNAFVSQTLTRQAEVRASRQLAKDKVNECVRSQSQRFGFCGNGTHLFSLANAAPNGMIFFHTVLLPTAYETVTAWSGICASDGDRTFGLVVKDVQLTLFRNLDDKFYLTPRTMYQPRVATSSDFVQIEGCDVLFVNATVIDLPSIIPDYIDINQTVQDILENYRPNWTVPEFTLDIFNATYLNLTGEIDDLEFRSEKLHNTTVELAILIDNINNTLVNLEWLNRIETYVKWPWYVWLLIGLVVVFCIPLLLFCCFSTGCCGCIGCLGSCCHSICSRRQFENYEPIEKVHVH

SEQ ID NO: 70 - protein, 2132 aa, synthetic construct
MATQGQRVNWGDEPSKRRGRSNSRGRKNNTIPLSFFNPIQLEPGSKFWSVCPRDFVPKGIGNKDQQIGYWNRQERYRIVKGQRKELPERWFFYFLGTGPQADAKFKDKIDGVFWVAKDGAMNKPTTLGTRGTNNESKPLKFDGKIPPQFQLEVNRSRNNSRSGSQSRSVSRNRSQSRGRQQSNNQNNVEDTIVAVLQKLGVTEKQRSRSKSRDRGDSKPRDTTPNNANKHTWKKTAGKGDVTNFYGARSASANFGDSDLVANGNAAKSYPQIAECVPSVSSMLFGSQWSAEDDGDQVKVTLTHTYYLPKDDAKTSQFLEQIDAYKRPSQVAKDQRQRKSRSKSAEKKPEELSVTLVEAYTDVFDDTQVEMIDEVTNGSGEGRGSLLTCGDVEENPGPMIVLVTCLLLLCSYHTVLSTTNNECIQVNVTQLAGNENLIRDFLFSNFKEEGSVVVGGYYPTEVWYNCSRTARTTAFQYFNNIHAFYFVMEAMENSTGNARGKPLLFHVHGEPVSVIISAYRDDVQQRPLLKHGLVCITKNRHINYEQFTSNQWNSTCTGADRKIPFSVIPTDNGTKIYGLEWNDDFVTAYISGRSYHLNINTNWFNNVTLLYSRSSTATWEYSAAYAYQGVSNFTYYKLNNTNGLKTYELCEDYEHCTGYATNVFAPTSGGYIPDGFSFNNWFLLTNSSTFVSGRFVTNQPLLINCLWPVPSFGVAAQEFCFEGAQFSQCNGVSLNNTVDVIRFNLNFTADVQSGMGATVFSLNTTGGVILEISCYSDTVSESSSYSYGEIPFGITDGPRYCYVLYNGTALKYLGTLPPSVKEIAISKWGHFYINGYNFFSTFPIGCISFNLTTGVSGAFWTIAYTSYTEALVQVENTAIKNVTYCNSHINNIKCSQLTANLNNGFYPVASSEVGFVNKSVVLLPSFFTYTAVNITIDLGMKLSGYGQPIASTLSNITLPMQDNNTDVYCIRSNQFSVYVHSTCKSSLWDNIFNQDCTDVLEATAVIKTGTCPFSFDKLNNYLTFNKFCLSLSPVGANCKFDVAARTRTNEQVVRSLYVIYEEGDNIVGVPSDNSGLHDLSVLHLDSCTDYNIYGRTGVGIIRRTNSTLLSGLYYTSLSGDLLGFKNVSDGVIYSVTPCDVSAQAAVIDGAIVGAMTSINSELLGLTHWTTTPNFYYYSIYNYTSERTRDTAIDSNDVDCEPVITYSNIGVCKNGALVFINVTHSDGDVQPISTGNVTIPTNFTISVQVEYMQVYTTPVSIDCARYVCNGNPRCNKLLTQYVSACQTIEQALAMGARLENMEVDSMLFVSENALKLASVEAFNSTENLDSIYKEWPSIGGSWLGGLKDILPSHNSKRKYGSAIEDLLFDKVVTSGLGTVDEDYKRCTGGYDIADLVCAQYYNGIMVLPGVANADKMTMYTASLAGGITLGALGGGAVAIPFAVAVQARLNYVALQTDVLNKNQQILANAFNQAIGNITQAFGKVNDAIHQTSQGLATVAKALAKVQDVVNTQGQALSHLTVQLQNNFQAISSSISDIYNRLDELSADAQVDRLITGRLTALNAFVSQTLTRQAEVRASRQLAKDKVNECVRSQSQRFGFCGNGTHLFSLANAAPNGMIFFHTVLLPTAYETVTAWSGICASDGDRTFGLVVKDVQLTLFRNLDDKFYLTPRTMYQPRVATSSDFVQIEGCDVLFVNATVIDLPSIIPDYIDINQTVQDILENYRPNWTVPEFTLDIFNATYLNLTGEIDDLEFRSEKLHNTTVELAILIDNINNTLVNLEWLNRIETYVKWPWYVWLLIGLVVVFCIPLLLFCCFSTGCCGCIGCLGSCCHSICSRRQFENYEPIEKVHVHGSGEGRGSLLTCGDVEENPGPMKYILLILACIIACVYGERYCAMQNTGSQCINGTDSSCSTCFERGGLIWHLANWNFSWSVILIVFITVLKYGRPQFSWLVYGIKMLIMWLLWPIVLALTIFNAYSEYQVSRYVMFGFSVAGAVVTFALWMMYFVRSIQLYRRTKSWWSFNPETNAILCVNALGRSYVLPLDGTPTGVTLTLLSGNLYAEGFKMAGGLTIEHLPKYVMIATPSRTIVYTLVGKQLKATTATGWAYYVKSKAGDYSTEARTDNLSEHEKLLHMV

SEQ ID NO: 71 - protein, 1354 aa, synthetic construct
MATQGQRVNWGDEPSKRRGRSNSRGRKNNTIPLSFFNPIQLEPGSKFWSVCPRDFVPKGIGNKDQQIGYWNRQERYRIVKGQRKELPERWFFYFLGTGPQADAKFKDKIDGVFWVAKDGAMNKPTTLGTRGTNNESKPLKFDGKIPPQFQLEVNRSRNNSRSGSQSRSVSRNRSQSRGRQQSNNQNNVEDTIVAVLQKLGVTEKQRSRSKSRDRGDSKPRDTTPNNANKHTWKKTAGKGDVTNFYGARSASANFGDSDLVANGNAAKSYPQIAECVPSVSSMLFGSQWSAEDDGDQVKVTLTHTYYLPKDDAKTSQFLEQIDAYKRPSQVAKDQRQRKSRSKSAEKKPEELSVTLVEAYTDVFDDTQVEMIDEVTNGSGEGRGSLLTCGDVEENPGPMKYILLILACIIACVYGERYCAMQNTGSQCINGTDSSCSTCFERGGLIWHLANWNFSWSVILIVFITVLKYGRPQFSWLVYGIKMLIMWLLWPIVLALTIFNAYSEYQVSRYVMFGFSVAGAVVTFALWMMYFVRSIQLYRRTKSWWSFNPETNAILCVNALGRSYVLPLDGTPTGVTLTLLSGNLYAEGFKMAGGLTIEHLPKYVMIATPSRTIVYTLVGKQLKATTATGWAYYVKSKAGDYSTEARTDNLSEHEKLLHMVGSGEGRGSLLTCGDVEENPGPMSIYNYTSERTRDTAIDSNDVDCEPVITYSNIGVCKNGALVFINVTHSDGDVQPISTGNVTIPTNFTISVQVEYMQVYTTPVSIDCARYVCNGNPRCNKLLTQYVSACQTIEQALAMGARLENMEVDSMLFVSENALKLASVEAFNSTENLDSIYKEWPSIGGSWLGGLKDILPSHNSKRKYGSAIEDLLFDKVVTSGLGTVDEDYKRCTGGYDIADLVCAQYYNGIMVLPGVANADKMTMYTASLAGGITLGALGGGAVAIPFAVAVQARLNYVALQTDVLNKNQQILANAFNQAIGNITQAFGKVNDAIHQTSQGLATVAKALAKVQDVVNTQGQALSHLTVQLQNNFQAISSSISDIYNRLDELSADAQVDRLITGRLTALNAFVSQTLTRQAEVRASRQLAKDKVNECVRSQSQRFGFCGNGTHLFSLANAAPNGMIFFHTVLLPTAYETVTAWSGICASDGDRTFGLVVKDVQLTLFRNLDDKFYLTPRTMYQPRVATSSDFVQIEGCDVLFVNATVIDLPSIIPDYIDINQTVQDILENYRPNWTVPEFTLDIFNATYLNLTGEIDDLEFRSEKLHNTTVELAILIDNINNTLVNLEWLNRIETYVKWPWYVWLLIGLVVVFCIPLLLFCCFSTGCCGCIGCLGSCCHSICSRRQFENYEPIEKVHVH

SEQ ID NO: 72 - protein, 1354 aa, synthetic construct
MATQGQRVNWGDEPSKRRGRSNSRGRKNNTIPLSFFNPIQLEPGSKFWSVCPRDFVPKGIGNKDQQIGYWNRQERYRIVKGQRKELPERWFFYFLGTGPQADAKFKDKIDGVFWVAKDGAMNKPTTLGTRGTNNESKPLKFDGKIPPQFQLEVNRSRNNSRSGSQSRSVSRNRSQSRGRQQSNNQNNVEDTIVAVLQKLGVTEKQRSRSKSRDRGDSKPRDTTPNNANKHTWKKTAGKGDVTNFYGARSASANFGDSDLVANGNAAKSYPQIAECVPSVSSMLFGSQWSAEDDGDQVKVTLTHTYYLPKDDAKTSQFLEQIDAYKRPSQVAKDQRQRKSRSKSAEKKPEELSVTLVEAYTDVFDDTQVEMIDEVTNGSGEGRGSLLTCGDVEENPGPMSIYNYTSERTRDTAIDSNDVDCEPVITYSNIGVCKNGALVFINVTHSDGDVQPISTGNVTIPTNFTISVQVEYMQVYTTPVSIDCARYVCNGNPRCNKLLTQYVSACQTIEQALAMGARLENMEVDSMLFVSENALKLASVEAFNSTENLDSIYKEWPSIGGSWLGGLKDILPSHNSKRKYGSAIEDLLFDKVVTSGLGTVDEDYKRCTGGYDIADLVCAQYYNGIMVLPGVANADKMTMYTASLAGGITLGALGGGAVAIPFAVAVQARLNYVALQTDVLNKNQQILANAFNQAIGNITQAFGKVNDAIHQTSQGLATVAKALAKVQDVVNTQGQALSHLTVQLQNNFQAISSSISDIYNRLDELSADAQVDRLITGRLTALNAFVSQTLTRQAEVRASRQLAKDKVNECVRSQSQRFGFCGNGTHLFSLANAAPNGMIFFHTVLLPTAYETVTAWSGICASDGDRTFGLVVKDVQLTLFRNLDDKFYLTPRTMYQPRVATSSDFVQIEGCDVLFVNATVIDLPSIIPDYIDINQTVQDILENYRPNWTVPEFTLDIFNATYLNLTGEIDDLEFRSEKLHNTTVELAILIDNINNTLVNLEWLNRIETYVKWPWYVWLLIGLVVVFCIPLLLFCCFSTGCCGCIGCLGSCCHSICSRRQFENYEPIEKVHVHGSGEGRGSLLTCGDVEENPGPMKYILLILACIIACVYGERYCAMQNTGSQCINGTDSSCSTCFERGGLIWHLANWNFSWSVILIVFITVLKYGRPQFSWLVYGIKMLIMWLLWPIVLALTIFNAYSEYQVSRYVMFGFSVAGAVVTFALWMMYFVRSIQLYRRTKSWWSFNPETNAILCVNALGRSYVLPLDGTPTGVTLTLLSGNLYAEGFKMAGGLTIEHLPKYVMIATPSRTIVYTLVGKQLKATTATGWAYYVKSKAGDYSTEARTDNLSEHEKLLHMV

SEQ ID NO: 73 - protein, 2134 aa, synthetic construct
MATQGQRVNWGDEPSKRRGRSNSRGRKNNTIPLSFFNPIQLEPGSKFWSVCPRDFVPKGIGNKDQQIGYWNRQERYRIVKGQRKELPERWFFYFLGTGPQADAKFKDKIDGVFWVAKDGAMNKPTTLGTRGTNNESKPLKFDGKIPPQFQLEVNRSRNNSRSGSQSRSVSRNRSQSRGRQQSNNQNNVEDTIVAVLQKLGVTEKQRSRSKSRDRGDSKPRDTTPNNANKHTWKKTAGKGDVTNFYGARSASANFGDSDLVANGNAAKSYPQIAECVPSVSSMLFGSQWSAEDDGDQVKVTLTHTYYLPKDDAKTSQFLEQIDAYKRPSQVAKDQRQRKSRSKSAEKKPEELSVTLVEAYTDVFDDTQVEMIDEVTNGSGATNFSLLKQAGDVEENPGPMKYILLILACIIACVYGERYCAMQNTGSQCINGTDSSCSTCFERGGLIWHLANWNFSWSVILIVFITVLKYGRPQFSWLVYGIKMLIMWLLWPIVLALTIFNAYSEYQVSRYVMFGFSVAGAVVTFALWMMYFVRSIQLYRRTKSWWSFNPETNAILCVNALGRSYVLPLDGTPTGVTLTLLSGNLYAEGFKMAGGLTIEHLPKYVMIATPSRTIVYTLVGKQLKATTATGWAYYVKSKAGDYSTEARTDNLSEHEKLLHMVGSGATNFSLLKQAGDVEENPGPMIVLVTCLLLLCSYHTVLSTTNNECIQVNVTQLAGNENLIRDFLFSNFKEEGSVVVGGYYPTEVWYNCSRTARTTAFQYFNNIHAFYFVMEAMENSTGNARGKPLLFHVHGEPVSVIISAYRDDVQQRPLLKHGLVCITKNRHINYEQFTSNQWNSTCTGADRKIPFSVIPTDNGTKIYGLEWNDDFVTAYISGRSYHLNINTNWFNNVTLLYSRSSTATWEYSAAYAYQGVSNFTYYKLNNTNGLKTYELCEDYEHCTGYATNVFAPTSGGYIPDGFSFNNWFLLTNSSTFVSGRFVTNQPLLINCLWPVPSFGVAAQEFCFEGAQFSQCNGVSLNNTVDVIRFNLNFTADVQSGMGATVFSLNTTGGVILEISCYSDTVSESSSYSYGEIPFGITDGPRYCYVLYNGTALKYLGTLPPSVKEIAISKWGHFYINGYNFFSTFPIGCISFNLTTGVSGAFWTIAYTSYTEALVQVENTAIKNVTYCNSHINNIKCSQLTANLNNGFYPVASSEVGFVNKSVVLLPSFFTYTAVNITIDLGMKLSGYGQPIASTLSNITLPMQDNNTDVYCIRSNQFSVYVHSTCKSSLWDNIFNQDCTDVLEATAVIKTGTCPFSFDKLNNYLTFNKFCLSLSPVGANCKFDVAARTRTNEQVVRSLYVIYEEGDNIVGVPSDNSGLHDLSVLHLDSCTDYNIYGRTGVGIIRRTNSTLLSGLYYTSLSGDLLGFKNVSDGVIYSVTPCDVSAQAAVIDGAIVGAMTSINSELLGLTHWTTTPNFYYYSIYNYTSERTRDTAIDSNDVDCEPVITYSNIGVCKNGALVFINVTHSDGDVQPISTGNVTIPTNFTISVQVEYMQVYTTPVSIDCARYVCNGNPRCNKLLTQYVSACQTIEQALAMGARLENMEVDSMLFVSENALKLASVEAFNSTENLDSIYKEWPSIGGSWLGGLKDILPSHNSKRKYGSAIEDLLFDKVVTSGLGTVDEDYKRCTGGYDIADLVCAQYYNGIMVLPGVANADKMTMYTASLAGGITLGALGGGAVAIPFAVAVQARLNYVALQTDVLNKNQQILANAFNQAIGNITQAFGKVNDAIHQTSQGLATVAKALAKVQDVVNTQGQALSHLTVQLQNNFQAISSSISDIYNRLDELSADAQVDRLITGRLTALNAFVSQTLTRQAEVRASRQLAKDKVNECVRSQSQRFGFCGNGTHLFSLANAAPNGMIFFHTVLLPTAYETVTAWSGICASDGDRTFGLVVKDVQLTLFRNLDDKFYLTPRTMYQPRVATSSDFVQIEGCDVLFVNATVIDLPSIIPDYIDINQTVQDILENYRPNWTVPEFTLDIFNATYLNLTGEIDDLEFRSEKLHNTTVELAILIDNINNTLVNLEWLNRIETYVKWPWYVWLLIGLVVVFCIPLLLFCCFSTGCCGCIGCLGSCCHSICSRRQFENYEPIEKVHVH

SEQ ID NO: 74 - protein, 2134 aa, synthetic construct
MATQGQRVNWGDEPSKRRGRSNSRGRKNNTIPLSFFNPIQLEPGSKFWSVCPRDFVPKGIGNKDQQIGYWNRQERYRIVKGQRKELPERWFFYFLGTGPQADAKFKDKIDGVFWVAKDGAMNKPTTLGTRGTNNESKPLKFDGKIPPQFQLEVNRSRNNSRSGSQSRSVSRNRSQSRGRQQSNNQNNVEDTIVAVLQKLGVTEKQRSRSKSRDRGDSKPRDTTPNNANKHTWKKTAGKGDVTNFYGARSASANFGDSDLVANGNAAKSYPQIAECVPSVSSMLFGSQWSAEDDGDQVKVTLTHTYYLPKDDAKTSQFLEQIDAYKRPSQVAKDQRQRKSRSKSAEKKPEELSVTLVEAYTDVFDDTQVEMIDEVTNGSGATNFSLLKQAGDVEENPGPMIVLVTCLLLLCSYHTVLSTTNNECIQVNVTQLAGNENLIRDFLFSNFKEEGSVVVGGYYPTEVWYNCSRTARTTAFQYFNNIHAFYFVMEAMENSTGNARGKPLLFHVHGEPVSVIISAYRDDVQQRPLLKHGLVCITKNRHINYEQFTSNQWNSTCTGADRKIPFSVIPTDNGTKIYGLEWNDDFVTAYISGRSYHLNINTNWFNNVTLLYSRSSTATWEYSAAYAYQGVSNFTYYKLNNTNGLKTYELCEDYEHCTGYATNVFAPTSGGYIPDGFSFNNWFLLTNSSTFVSGRFVTNQPLLINCLWPVPSFGVAAQEFCFEGAQFSQCNGVSLNNTVDVIRFNLNFTADVQSGMGATVFSLNTTGGVILEISCYSDTVSESSSYSYGEIPFGITDGPRYCYVLYNGTALKYLGTLPPSVKEIAISKWGHFYINGYNFFSTFPIGCISFNLTTGVSGAFWTIAYTSYTEALVQVENTAIKNVTYCNSHINNIKCSQLTANLNNGFYPVASSEVGFVNKSVVLLPSFFTYTAVNITIDLGMKLSGYGQPIASTLSNITLPMQDNNTDVYCIRSNQFSVYVHSTCKSSLWDNIFNQDCTDVLEATAVIKTGTCPFSFDKLNNYLTFNKFCLSLSPVGANCKFDVAARTRTNEQVVRSLYVIYEEGDNIVGVPSDNSGLHDLSVLHLDSCTDYNIYGRTGVGIIRRTNSTLLSGLYYTSLSGDLLGFKNVSDGVIYSVTPCDVSAQAAVIDGAIVGAMTSINSELLGLTHWTTTPNFYYYSIYNYTSERTRDTAIDSNDVDCEPVITYSNIGVCKNGALVFINVTHSDGDVQPISTGNVTIPTNFTISVQVEYMQVYTTPVSIDCARYVCNGNPRCNKLLTQYVSACQTIEQALAMGARLENMEVDSMLFVSENALKLASVEAFNSTENLDSIYKEWPSIGGSWLGGLKDILPSHNSKRKYGSAIEDLLFDKVVTSGLGTVDEDYKRCTGGYDIADLVCAQYYNGIMVLPGVANADKMTMYTASLAGGITLGALGGGAVAIPFAVAVQARLNYVALQTDVLNKNQQILANAFNQAIGNITQAFGKVNDAIHQTSQGLATVAKALAKVQDVVNTQGQALSHLTVQLQNNFQAISSSISDIYNRLDELSADAQVDRLITGRLTALNAFVSQTLTRQAEVRASRQLAKDKVNECVRSQSQRFGFCGNGTHLFSLANAAPNGMIFFHTVLLPTAYETVTAWSGICASDGDRTFGLVVKDVQLTLFRNLDDKFYLTPRTMYQPRVATSSDFVQIEGCDVLFVNATVIDLPSIIPDYIDINQTVQDILENYRPNWTVPEFTLDIFNATYLNLTGEIDDLEFRSEKLHNTTVELAILIDNINNTLVNLEWLNRIETYVKWPWYVWLLIGLVVVFCIPLLLFCCFSTGCCGCIGCLGSCCHSICSRRQFENYEPIEKVHVHGSGATNFSLLKQAGDVEENPGPMKYILLILACIIACVYGERYCAMQNTGSQCINGTDSSCSTCFERGGLIWHLANWNFSWSVILIVFITVLKYGRPQFSWLVYGIKMLIMWLLWPIVLALTIFNAYSEYQVSRYVMFGFSVAGAVVTFALWMMYFVRSIQLYRRTKSWWSFNPETNAILCVNALGRSYVLPLDGTPTGVTLTLLSGNLYAEGFKMAGGLTIEHLPKYVMIATPSRTIVYTLVGKQLKATTATGWAYYVKSKAGDYSTEARTDNLSEHEKLLHMV

SEQ ID NO: 75 - protein, 1356 aa, synthetic construct
MATQGQRVNWGDEPSKRRGRSNSRGRKNNTIPLSFFNPIQLEPGSKFWSVCPRDFVPKGIGNKDQQIGYWNRQERYRIVKGQRKELPERWFFYFLGTGPQADAKFKDKIDGVFWVAKDGAMNKPTTLGTRGTNNESKPLKFDGKIPPQFQLEVNRSRNNSRSGSQSRSVSRNRSQSRGRQQSNNQNNVEDTIVAVLQKLGVTEKQRSRSKSRDRGDSKPRDTTPNNANKHTWKKTAGKGDVTNFYGARSASANFGDSDLVANGNAAKSYPQIAECVPSVSSMLFGSQWSAEDDGDQVKVTLTHTYYLPKDDAKTSQFLEQIDAYKRPSQVAKDQRQRKSRSKSAEKKPEELSVTLVEAYTDVFDDTQVEMIDEVTNGSGATNFSLLKQAGDVEENPGPMKYILLILACIIACVYGERYCAMQNTGSQCINGTDSSCSTCFERGGLIWHLANWNFSWSVILIVFITVLKYGRPQFSWLVYGIKMLIMWLLWPIVLALTIFNAYSEYQVSRYVMFGFSVAGAVVTFALWMMYFVRSIQLYRRTKSWWSFNPETNAILCVNALGRSYVLPLDGTPTGVTLTLLSGNLYAEGFKMAGGLTIEHLPKYVMIATPSRTIVYTLVGKQLKATTATGWAYYVKSKAGDYSTEARTDNLSEHEKLLHMVGSGATNFSLLKQAGDVEENPGPMSIYNYTSERTRDTAIDSNDVDCEPVITYSNIGVCKNGALVFINVTHSDGDVQPISTGNVTIPTNFTISVQVEYMQVYTTPVSIDCARYVCNGNPRCNKLLTQYVSACQTIEQALAMGARLENMEVDSMLFVSENALKLASVEAFNSTENLDSIYKEWPSIGGSWLGGLKDILPSHNSKRKYGSAIEDLLFDKVVTSGLGTVDEDYKRCTGGYDIADLVCAQYYNGIMVLPGVANADKMTMYTASLAGGITLGALGGGAVAIPFAVAVQARLNYVALQTDVLNKNQQILANAFNQAIGNITQAFGKVNDAIHQTSQGLATVAKALAKVQDVVNTQGQALSHLTVQLQNNFQAISSSISDIYNRLDELSADAQVDRLITGRLTALNAFVSQTLTRQAEVRASRQLAKDKVNECVRSQSQRFGFCGNGTHLFSLANAAPNGMIFFHTVLLPTAYETVTAWSGICASDGDRTFGLVVKDVQLTLFRNLDDKFYLTPRTMYQPRVATSSDFVQIEGCDVLFVNATVIDLPSIIPDYIDINQTVQDILENYRPNWTVPEFTLDIFNATYLNLTGEIDDLEFRSEKLHNTTVELAILIDNINNTLVNLEWLNRIETYVKWPWYVWLLIGLVVVFCIPLLLFCCFSTGCCGCIGCLGSCCHSICSRRQFENYEPIEKVHVH

SEQ ID NO: 76 - protein, 1356 aa, synthetic construct
MATQGQRVNWGDEPSKRRGRSNSRGRKNNTIPLSFFNPIQLEPGSKFWSVCPRDFVPKGIGNKDQQIGYWNRQERYRIVKGQRKELPERWFFYFLGTGPQADAKFKDKIDGVFWVAKDGAMNKPTTLGTRGTNNESKPLKFDGKIPPQFQLEVNRSRNNSRSGSQSRSVSRNRSQSRGRQQSNNQNNVEDTIVAVLQKLGVTEKQRSRSKSRDRGDSKPRDTTPNNANKHTWKKTAGKGDVTNFYGARSASANFGDSDLVANGNAAKSYPQIAECVPSVSSMLFGSQWSAEDDGDQVKVTLTHTYYLPKDDAKTSQFLEQIDAYKRPSQVAKDQRQRKSRSKSAEKKPEELSVTLVEAYTDVFDDTQVEMIDEVTNGSGATNFSLLKQAGDVEENPGPMSIYNYTSERTRDTAIDSNDVDCEPVITYSNIGVCKNGALVFINVTHSDGDVQPISTGNVTIPTNFTISVQVEYMQVYTTPVSIDCARYVCNGNPRCNKLLTQYVSACQTIEQALAMGARLENMEVDSMLFVSENALKLASVEAFNSTENLDSIYKEWPSIGGSWLGGLKDILPSHNSKRKYGSAIEDLLFDKVVTSGLGTVDEDYKRCTGGYDIADLVCAQYYNGIMVLPGVANADKMTMYTASLAGGITLGALGGGAVAIPFAVAVQARLNYVALQTDVLNKNQQILANAFNQAIGNITQAFGKVNDAIHQTSQGLATVAKALAKVQDVVNTQGQALSHLTVQLQNNFQAISSSISDIYNRLDELSADAQVDRLITGRLTALNAFVSQTLTRQAEVRASRQLAKDKVNECVRSQSQRFGFCGNGTHLFSLANAAPNGMIFFHTVLLPTAYETVTAWSGICASDGDRTFGLVVKDVQLTLFRNLDDKFYLTPRTMYQPRVATSSDFVQIEGCDVLFVNATVIDLPSIIPDYIDINQTVQDILENYRPNWTVPEFTLDIFNATYLNLTGEIDDLEFRSEKLHNTTVELAILIDNINNTLVNLEWLNRIETYVKWPWYVWLLIGLVVVFCIPLLLFCCFSTGCCGCIGCLGSCCHSICSRRQFENYEPIEKVHVHGSGATNFSLLKQAGDVEENPGPMKYILLILACIIACVYGERYCAMQNTGSQCINGTDSSCSTCFERGGLIWHLANWNFSWSVILIVFITVLKYGRPQFSWLVYGIKMLIMWLLWPIVLALTIFNAYSEYQVSRYVMFGFSVAGAVVTFALWMMYFVRSIQLYRRTKSWWSFNPETNAILCVNALGRSYVLPLDGTPTGVTLTLLSGNLYAEGFKMAGGLTIEHLPKYVMIATPSRTIVYTLVGKQLKATTATGWAYYVKSKAGDYSTEARTDNLSEHEKLLHMV